European Patent Specification EP 3 870 202 B1, published May 14, 2025. Title: Miniaturized Dystrophins and Uses Thereof. Applicant: BRISTOL-MYERS SQUIBB COMPANY Banks, Glen. The sequence listing filed with the application follows.

SEQUENCE LISTING (166 sequences)

SEQ ID NO: 1 - protein, 3685 aa, Homo sapiens
MLWWEEVEDCYEREDVQKKTFTKWVNAQFSKFGKQHIENLFSDLQDGRRLLDLLEGLTGQKLPKEKGSTRVHALNNVNKALRVLQNNNVDLVNIGSTDIVDGNHKLTLGLIWNIILHWQVKNVMKNIMAGLQQTNSEKILLSWVRQSTRNYPQVNVINFTTSWSDGLALNALIHSHRPDLFDWNSVVCQQSATQRLEHAFNIARYQLGIEKLLDPEDVDTTYPDKKSILMYITSLFQVLPQQVSIEAIQEVEMLPRPPKVTKEEHFQLHHQMHYSQQITVSLAQGYERTSSPKPRFKSYAYTQAAYVTTSDPTRSPFPSQHLEAPEDKSFGSSLMESEVNLDRYQTALEEVLSWLLSAEDTLQAQGEISNDVEVVKDQFHTHEGYMMDLTAHQGRVGNILQLGSKLIGTGKLSEDEETEVQEQMNLLNSRWECLRVASMEKQSNLHRVLMDLQNQKLKELNDWLTKTEERTRKMEEEPLGPDLEDLKRQVQQHKVLQEDLEQEQVRVNSLTHMVVVVDESSGDHATAALEEQLKVLGDRWANICRWTEDRWVLLQDILLKWQRLTEEQCLFSAWLSEKEDAVNKIHTTGFKDQNEMLSSLQKLAVLKADLEKKKQSMGKLYSLKQDLLSTLKNKSVTQKTEAWLDNFARCWDNLVQKLEKSTAQISQAVTTTQPSLTQTTVMETVTTVTTREQILVKHAQEELPPPPPQKKRQITVDSEIRKRLDVDITELHSWITRSEAVLQSPEFAIFRKEGNFSDLKEKVNAIEREKAEKFRKLQDASRSAQALVEQMVNEGVNADSIKQASEQLNSRWIEFCQLLSERLNWLEYQNNIIAFYNQLQQLEQMTTTAENWLKIQPTTPSEPTAIKSQLKICKDEVNRLSGLQPQIERLKIQSIALKEKGQGPMFLDADFVAFTNHFKQVFSDVQAREKELQTIFDTLPPMRYQETMSAIRTWVQQSETKLSIPQLSVTDYEIMEQRLGELQALQSSLQEQQSGLYYLSTTVKEMSKKAPSEISRKYQSEFEEIEGRWKKLSSQLVEHCQKLEEQMNKLRKIQNHIQTLKKWMAEVDVFLKEEWPALGDSEILKKQLKQCRLLVSDIQTIQPSLNSVNEGGQKIKNEAEPEFASRLETELKELNTQWDHMCQQVYARKEALKGGLEKTVSLQKDLSEMHEWMTQAEEEYLERDFEYKTPDELQKAVEEMKRAKEEAQQKEAKVKLLTESVNSVIAQAPPVAQEALKKELETLTTNYQWLCTRLNGKCKTLEEVWACWHELLSYLEKANKWLNEVEFKLKTTENIPGGAEEISEVLDSLENLMRHSEDNPNQIRILAQTLTDGGVMDELINEELETFNSRWRELHEEAVRRQKLLEQSIQSAQETEKSLHLIQESLTFIDKQLAAYIADKVDAAQMPQEAQKIQSDLTSHEISLEEMKKHNQGKEAAQRVLSQIDVAQKKLQDVSMKFRLFQKPANFEQRLQESKMILDEVKMHLPALETKSVEQEVVQSQLNHCVNLYKSLSEVKSEVEMVIKTGRQIVQKKQTENPKELDERVTALKLHYNELGAKVTERKQQLEKCLKLSRKMRKEMNVLTEWLAATDMELTKRSAVEGMPSNLDSEVAWGKATQKEIEKQKVHLKSITEVGEALKTVLGKKETLVEDKLSLLNSNWIAVTSRAEEWLNLLLEYQKHMETFDQNVDHITKWIIQADTLLDESEKKKPQQKEDVLKRLKAELNDIRPKVDSTRDQAANLMANRGDHCRKLVEPQISELNHRFAAISHRIKTGKASIPLKELEQFNSDIQKLLEPLEAEIQQGVNLKEEDFNKDMNEDNEGTVKELLQRGDNLQQRITDERKREEIKIKQQLLQTKHNALKDLRSQRRKKALEISHQWYQYKRQADDLLKCLDDIEKKLASLPEPRDERKIKEIDRELQKKKEELNAVRRQAEGLSEDGAAMAVEPTQIQLSKRWREIESKFAQFRRLNFAQIHTVREETMMVMTEDMPLEISYVPSTYLTEITHVSQALLEVEQLLNAPDLCAKDFEDLFKQEESLKNIKDSLQQSSGRIDIIHSKKTAALQSATPVERVKLQEALSQLDFQWEKVNKMYKDRQGRFDRSVEKWRRFHYDIKIFNQWLTEAEQFLRKTQIPENWEHAKYKWYLKELQDGIGQRQTVVRTLNATGEEIIQQSSKTDASILQEKLGSLNLRWQEVCKQLSDRKKRLEEQKNILSEFQRDLNEFVLWLEEADNIASIPLEPGKEQQLKEKLEQVKLLVEELPLRQGILKQLNETGGPVLVSAPISPEEQDKLENKLKQTNLQWIKVSRALPEKQGEIEAQIKDLGQLEKKLEDLEEQLNHLLLWLSPIRNQLEIYNQPNQEGPFDVQETEIAVQAKQPDVEEILSKGQHLYKEKPATQPVKRKLEDLSSEWKAVNRLLQELRAKQPDLAPGLTTIGASPTQTVTLVTQPVVTKETAISKLEMPSSLMLEVPALADFNRAWTELTDWLSLLDQVIKSQRVMVGDLEDINEMIIKQKATMQDLEQRRPQLEELITAAQNLKNKTSNQEARTIITDRIERIQNQWDEVQEHLQNRRQQLNEMLKDSTQWLEAKEEAEQVLGQARAKLESWKEGPYTVDAIQKKITETKQLAKDLRQWQTNVDVANDLALKLLRDYSADDTRKVHMITENINASWRSIHKRVSEREAALEETHRLLQQFPLDLEKFLAWLTEAETTANVLQDATRKERLLEDSKGVKELMKQWQDLQGEIEAHTDVYHNLDENSQKILRSLEGSDDAVLLQRRLDNMNFKWSELRKKSLNIRSHLEASSDQWKRLHLSLQELLVWLQLKDDELSRQAPIGGDFPAVQKQNDVHRAFKRELKTKEPVIMSTLETVRIFLTEQPLEGLEKLYQEPRELPPEERAQNVTRLLRKQAEEVNTEWEKLNLHSADWQRKIDETLERLQELQEATDELDLKLRQAEVIKGSWQPVGDLLIDSLQDHLEKVKALRGEIAPLKENVSHVNDLARQLTTLGIQLSPYNLSTLEDLNTRWKLLQVAVEDRVRQLHEAHRDFGPASQHFLSTSVQGPWERAISPNKVPYYINHETQTTCWDHPKMTELYQSLADLNNVRFSAYRTAMKLRRLQKALCLDLLSLSAACDALDQHNLKQNDQPMDILQIINCLTTIYDRLEQEHNNLVNVPLCVDMCLNWLLNVYDTGRTGRIRVLSFKTGIISLCKAHLEDKYRYLFKQVASSTGFCDQRRLGLLLHDSIQIPRQLGEVASFGGSNIEPSVRSCFQFANNKPEIEAALFLDWMRLEPQSMVWLPVLHRVAAAETAKHQAKCNICKECPIIGFRYRSLKHFNYDICQSCFFSGRVAKGHKMHYPMVEYCTPTTSGEDVRDFAKVLKNKFRTKRYFAKHPRMGYLPVQTVLEGDNMETPVTLINFWPVDSAPASSPQLSHDDTHSRIEHYASRLAEMENSNGSYLNDSISPNESIDDEHLLIQHYCQSLNQDSPLSQPRSPAQILISLESEERGELERILADLEEENRNLQAEYDRLKQQHEHKGLSPLPSPPEMMPTSPQSPRDAELIAEAKLLRQHKGRLEARMQILEDHNKQLESQLHRLRQLLEQPQAEAKVNGTTVSSPSTSLQRSDSSQPMLLRVVGSQTSDSMGEEDLLSPPQDTSTGLEEVMEQLNNSFPSSRGRNTPGKPMREDTM

SEQ ID NO: 2 - DNA, 13957 bp, Homo sapiens
gggattccctcactttccccctacaggactcagatctgggaggcaattaccttcggagaaaaacgaataggaaaaactgaagtgttactttttttaaagctgctgaagtttgttggtttctcattgtttttaagcctactggagcaataaagtttgaagaacttttaccaggttttttttatcgctgccttgatatacacttttcaaaatgctttggtgggaagaagtagaggactgttatgaaagagaagatgttcaaaagaaaacattcacaaaatgggtaaatgcacaattttctaagtttgggaagcagcatattgagaacctcttcagtgacctacaggatgggaggcgcctcctagacctcctcgaaggcctgacagggcaaaaactgccaaaagaaaaaggatccacaagagttcatgccctgaacaatgtcaacaaggcactgcgggttttgcagaacaataatgttgatttagtgaatattggaagtactgacatcgtagatggaaatcataaactgactcttggtttgatttggaatataatcctccactggcaggtcaaaaatgtaatgaaaaatatcatggctggattgcaacaaaccaacagtgaaaagattctcctgagctgggtccgacaatcaactcgtaattatccacaggttaatgtaatcaacttcaccaccagctggtctgatggcctggctttgaatgctctcatccatagtcataggccagacctatttgactggaatagtgtggtttgccagcagtcagccacacaacgactggaacatgcattcaacatcgccagatatcaattaggcatagagaaactactcgatcctgaagatgttgataccacctatccagataagaagtccatcttaatgtacatcacatcactcttccaagttttgcctcaacaagtgagcattgaagccatccaggaagtggaaatgttgccaaggccacctaaagtgactaaagaagaacattttcagttacatcatcaaatgcactattctcaacagatcacggtcagtctagcacagggatatgagagaacttcttcccctaagcctcgattcaagagctatgcctacacacaggctgcttatgtcaccacctctgaccctacacggagcccatttccttcacagcatttggaagctcctgaagacaagtcatttggcagttcattgatggagagtgaagtaaacctggaccgttatcaaacagctttagaagaagtattatcgtggcttctttctgctgaggacacattgcaagcacaaggagagatttctaatgatgtggaagtggtgaaagaccagtttcatactcatgaggggtacatgatggatttgacagcccatcagggccgggttggtaatattctacaattgggaagtaagctgattggaacaggaaaattatcagaagatgaagaaactgaagtacaagagcagatgaatctcctaaattcaagatgggaatgcctcagggtagctagcatggaaaaacaaagcaatttacatagagttttaatggatctccagaatcagaaactgaaagagttgaatgactggctaacaaaaacagaagaaagaacaaggaaaatggaggaagagcctcttggacctgatcttgaagacctaaaacgccaagtacaacaacataaggtgcttcaagaagatctagaacaagaacaagtcagggtcaattctctcactcacatggtggtggtagttgatgaatctagtggagatcacgcaactgctgctttggaagaacaacttaaggtattgggagatcgatgggcaaacatctgtagatggacagaagaccgctgggttcttttacaagacatccttctcaaatggcaacgtcttactgaagaacagtgcctttttagtgcatggctttcagaaaaagaagatgcagtgaacaagattcacacaactggctttaaagatcaaaatgaaatgttatcaagtcttcaaaaactggccgttttaaaagcggatctagaaaagaaaaagcaatccatgggcaaactgtattcactcaaacaagatcttctttcaacactgaagaataagtcagtgacccagaagacggaagcatggctggataactttgcccggtgttgggataatttagtccaaaaacttgaaaagagtacagcacagatttcacaggctgtcaccaccactcagccatcactaacacagacaactgtaatggaaacagtaactacggtgaccacaagggaacagatcctggtaaagcatgctcaagaggaacttccaccaccacctccccaaaagaagaggcagattactgtggattctgaaattaggaaaaggttggatgttgatataactgaacttcacagctggattactcgctcagaagctgtgttgcagagtcctgaatttgcaatctttcggaaggaaggcaacttctcagacttaaaagaaaaagtcaatgccatagagcgagaaaaagctgagaagttcagaaaactgcaagatgccagcagatcagctcaggccctggtggaacagatggtgaatgagggtgttaatgcagatagcatcaaacaagcctcagaacaactgaacagccggtggatcgaattctgccagttgctaagtgagagacttaactggctggagtatcagaacaacatcatcgctttctataatcagctacaacaattggagcagatgacaactactgctgaaaactggttgaaaatccaacccaccaccccatcagagccaacagcaattaaaagtcagttaaaaatttgtaaggatgaagtcaaccggctatcaggtcttcaacctcaaattgaacgattaaaaattcaaagcatagccctgaaagagaaaggacaaggacccatgttcctggatgcagactttgtggcctttacaaatcattttaagcaagtcttttctgatgtgcaggccagagagaaagagctacagacaatttttgacactttgccaccaatgcgctatcaggagaccatgagtgccatcaggacatgggtccagcagtcagaaaccaaactctccatacctcaacttagtgtcaccgactatgaaatcatggagcagagactcggggaattgcaggctttacaaagttctctgcaagagcaacaaagtggcctatactatctcagcaccactgtgaaagagatgtcgaagaaagcgccctctgaaattagccggaaatatcaatcagaatttgaagaaattgagggacgctggaagaagctctcctcccagctggttgagcattgtcaaaagctagaggagcaaatgaataaactccgaaaaattcagaatcacatacaaaccctgaagaaatggatggctgaagttgatgtttttctgaaggaggaatggcctgcccttggggattcagaaattctaaaaaagcagctgaaacagtgcagacttttagtcagtgatattcagacaattcagcccagtctaaacagtgtcaatgaaggtgggcagaagataaagaatgaagcagagccagagtttgcttcgagacttgagacagaactcaaagaacttaacactcagtgggatcacatgtgccaacaggtctatgccagaaaggaggccttgaagggaggtttggagaaaactgtaagcctccagaaagatctatcagagatgcacgaatggatgacacaagctgaagaagagtatcttgagagagattttgaatataaaactccagatgaattacagaaagcagttgaagagatgaagagagctaaagaagaggcccaacaaaaagaagcgaaagtgaaactccttactgagtctgtaaatagtgtcatagctcaagctccacctgtagcacaagaggccttaaaaaaggaacttgaaactctaaccaccaactaccagtggctctgcactaggctgaatgggaaatgcaagactttggaagaagtttgggcatgttggcatgagttattgtcatacttggagaaagcaaacaagtggctaaatgaagtagaatttaaacttaaaaccactgaaaacattcctggcggagctgaggaaatctctgaggtgctagattcacttgaaaatttgatgcgacattcagaggataacccaaatcagattcgcatattggcacagaccctaacagatggcggagtcatggatgagctaatcaatgaggaacttgagacatttaattctcgttggagggaactacatgaagaggctgtaaggaggcaaaagttgcttgaacagagcatccagtctgcccaggagactgaaaaatccttacacttaatccaggagtccctcacattcattgacaagcagttggcagcttatattgcagacaaggtggacgcagctcaaatgcctcaggaagcccagaaaatccaatctgatttgacaagtcatgagatcagtttagaagaaatgaagaaacataatcaggggaaggaggctgcccaaagagtcctgtctcagattgatgttgcacagaaaaaattacaagatgtctccatgaagtttcgattattccagaaaccagccaattttgagctgcgtctacaagaaagtaagatgattttagatgaagtgaagatgcacttgcctgcattggaaacaaagagtgtggaacaggaagtagtacagtcacagctaaatcattgtgtgaacttgtataaaagtctgagtgaagtgaagtctgaagtggaaatggtgataaagactggacgtcagattgtacagaaaaagcagacggaaaatcccaaagaacttgatgaaagagtaacagctttgaaattgcattataatgagctgggagcaaaggtaacagaaagaaagcaacagttggagaaatgcttgaaattgtcccgtaagatgcgaaaggaaatgaatgtcttgacagaatggctggcagctacagatatggaattgacaaagagatcagcagttgaaggaatgcctagtaatttggattctgaagttgcctggggaaaggctactcaaaaagagattgagaaacagaaggtgcacctgaagagtatcacagaggtaggagaggccttgaaaacagttttgggcaagaaggagacgttggtggaagataaactcagtcttctgaatagtaactggatagctgtcacctcccgagcagaagagtggttaaatcttttgttggaataccagaaacacatggaaacttttgaccagaatgtggaccacatcacaaagtggatcattcaggctgacacacttttggatgaatcagagaaaaagaaaccccagcaaaaagaagacgtgcttaagcgtttaaaggcagaactgaatgacatacgcccaaaggtggactctacacgtgaccaagcagcaaacttgatggcaaaccgcggtgaccactgcaggaaattagtagagccccaaatctcagagctcaaccatcgatttgcagccatttcacacagaattaagactggaaaggcctccattcctttgaaggaattggagcagtttaactcagatatacaaaaattgcttgaaccactggaggctgaaattcagcagggggtgaatctgaaagaggaagacttcaataaagatatgaatgaagacaatgagggtactgtaaaagaattgttgcaaagaggagacaacttacaacaaagaatcacagatgagagaaagagagaggaaataaagataaaacagcagctgttacagacaaaacataatgctctcaaggatttgaggtctcaaagaagaaaaaaggctctagaaatttctcatcagtggtatcagtacaagaggcaggctgatgatctcctgaaatgcttggatgacattgaaaaaaaattagccagcctacctgagcccagagatgaaaggaaaataaaggaaattgatcgggaattgcagaagaagaaagaggagctgaatgcagtgcgtaggcaagctgagggcttgtctgaggatggggccgcaatggcagtggagccaactcagatccagctcagcaagcgctggcgggaaattgagagcaaatttgctcagtttcgaagactcaactttgcacaaattcacactgtccgtgaagaaacgatgatggtgatgactgaagacatgcctttggaaatttcttatgtgccttctacttatttgactgaaatcactcatgtctcacaagccctattagaagtggaacaacttctcaatgctcctgacctctgtgctaaggactttgaagatctctttaagcaagaggagtctctgaagaatataaaagatagtctacaacaaagctcaggtcggattgacattattcatagcaagaagacagcagcattgcaaagtgcaacgcctgtggaaagggtgaagctacaggaagctctctcccagcttgatttccaatgggaaaaagttaacaaaatgtacaaggaccgacaagggcgatttgacagatctgttgagaaatggcggcgttttcattatgatataaagatatttaatcagtggctaacagaagctgaacagtttctcagaaagacacaaattcctgagaattgggaacatgctaaatacaaatggtatcttaaggaactccaggatggcattgggcagcggcaaactgttgtcagaacattgaatgcaactggggaagaaataattcagcaatcctcaaaaacagatgccagtattctacaggaaaaattgggaagcctgaatctgcggtggcaggaggtctgcaaacagctgtcagacagaaaaaagaggctagaagaacaaaagaatatcttgtcagaatttcaaagagatttaaatgaatttgttttatggttggaggaagcagataacattgctagtatcccacttgaacctggaaaagagcagcaactaaaagaaaagcttgagcaagtcaagttactggtggaagagttgcccctgcgccagggaattctcaaacaattaaatgaaactggaggacccgtgcttgtaagtgctcccataagcccagaagagcaagataaacttgaaaataagctcaagcagacaaatctccagtggataaaggtttccagagctttacctgagaaacaaggagaaattgaagctcaaataaaagaccttgggcagcttgaaaaaaagcttgaagaccttgaagagcagttaaatcatctgctgctgtggttatctcctattaggaatcagttggaaatttataaccaaccaaaccaagaaggaccatttgacgttcaggaaactgaaatagcagttcaagctaaacaaccggatgtggaagagattttgtctaaagggcagcatttgtacaaggaaaaaccagccactcagccagtgaagaggaagttagaagatctgagctctgagtggaaggcggtaaaccgtttacttcaagagctgagggcaaagcagcctgacctagctcctggactgaccactattggagcctctcctactcagactgttactctggtgacacaacctgtggttactaaggaaactgccatctccaaactagaaatgccatcttccttgatgttggaggtacctgctctggcagatttcaaccgggcttggacagaacttaccgactggctttctctgcttgatcaagttataaaatcacagagggtgatggtgggtgaccttgaggatatcaacgagatgatcatcaagcagaaggcaacaatgcaggatttggaacagaggcgtccccagttggaagaactcattaccgctgcccaaaatttgaaaaacaagaccagcaatcaagaggctagaacaatcattacggatcgaattgaaagaattcagaatcagtgggatgaagtacaagaacaccttcagaaccggaggcaacagttgaatgaaatgttaaaggattcaacacaatggctggaagctaaggaagaagctgagcaggtcttaggacaggccagagccaagcttgagtcatggaaggagggtccctatacagtagatgcaatccaaaagaaaatcacagaaaccaagcagttggccaaagacctccgccagtggcagacaaatgtagatgtggcaaatgacttggccctgaaacttctccgggattattctgcagatgataccagaaaagtccacatgataacagagaatatcaatgcctcttggagaagcattcataaaagggtgagtgagcgagaggctgctttggaagaaactcatagattactgcaacagttccccctggacctggaaaagtttcttgcctggcttacagaagctgaaacaactgccaatgtcctacaggatgctacccgtaaggaaaggctcctagaagactccaagggagtaaaagagctgatgaaacaatggcaagacctccaaggtgaaattgaagctcacacagatgtttatcacaacctggatgaaaacagccaaaaaatcctgagatccctggaaggttccgatgatgcagtcctgttacaaagacgtttggataacatgaacttcaagtggagtgaacttcggaaaaagtctctcaacattaggtcccatttggaagccagttctgaccagtggaagcgtctgcacctttctctgcaggaacttctggtgtggctacagctgaaagatgatgaattaagccggcaggcacctattggaggcgactttccagcagttcagaagcagaacgatgtacatagggccttcaagagggaattgaaaactaaagaacctgtaatcatgagtactcttgagactgtacgaatatttctgacagagcagcctttggaaggactagagaaactctaccaggagcccagagagctgcctcctgaggagagagcccagaatgtcactcggcttctacgaaagcaggctgaggaggtcaatactgagtgggaaaaattgaacctgcactccgctgactggcagagaaaaatagatgagacccttgaaagactccaggaacttcaagaggccacggatgagctggacctcaagctgcgccaagctgaggtgatcaagggatcctggcagcccgtgggcgatctcctcattgactctctccaagatcacctcgagaaagtcaaggcacttcgaggagaaattgcgcctctgaaagagaacgtgagccacgtcaatgaccttgctcgccagcttaccactttgggcattcagctctcaccgtataacctcagcactctggaagacctgaacaccagatggaagcttctgcaggtggccgtcgaggaccgagtcaggcagctgcatgaagcccacagggactttggtccagcatctcagcactttctttccacgtctgtccagggtccctgggagagagccatctcgccaaacaaagtgccctactatatcaaccacgagactcaaacaacttgctgggaccatcccaaaatgacagagctctaccagtctttagctgacctgaataatgtcagattctcagcttataggactgccatgaaactccgaagactgcagaaggccctttgcttggatctcttgagcctgtcagctgcatgtgatgccttggaccagcacaacctcaagcaaaatgaccagcccatggatatcctgcagattattaattgtttgaccactatttatgaccgcctggagcaagagcacaacaatttggtcaacgtccctctctgcgtggatatgtgtctgaactggctgctgaatgtttatgatacgggacgaacagggaggatccgtgtcctgtcttttaaaactggcatcatttccctgtgtaaagcacatttggaagacaagtacagataccttttcaagcaagtggcaagttcaacaggattttgtgaccagcgcaggctgggcctccttctgcatgattctatccaaattccaagacagttgggtgaagttgcatcctttgggggcagtaacattgagccaagtgtccggagctgcttccaatttgctaataataagccagagatcgaagcggccctcttcctagactggatgagactggaaccccagtccatggtgtggctgcccgtcctgcacagagtggctgctgcagaaactgccaagcatcaggccaaatgtaacatctgcaaagagtgtccaatcattggattcaggtacaggagtctaaagcactttaattatgacatctgccaaagctgctttttttctggtcgagttgcaaaaggccataaaatgcactatcccatggtggaatattgcactccgactacatcaggagaagatgttcgagactttgccaaggtactaaaaaacaaatttcgaaccaaaaggtattttgcgaagcatccccgaatgggctacctgccagtgcagactgtcttagagggggacaacatggaaactcccgttactctgatcaacttctggccagtagattctgcgcctgcctcgtcccctcagctttcacacgatgatactcattcacgcattgaacattatgctagcaggctagcagaaatggaaaacagcaatggatcttatctaaatgatagcatctctcctaatgagagcatagatgatgaacatttgttaatccagcattactgccaaagtttgaaccaggactcccccctgagccagcctcgtagtcctgcccagatcttgatttccttagagagtgaggaaagaggggagctagagagaatcctagcagatcttgaggaagaaaacaggaatctgcaagcagaatatgaccgtctaaagcagcagcacgaacataaaggcctgtccccactgccgtcccctcctgaaatgatgcccacctctccccagagtccccgggatgctgagctcattgctgaggccaagctactgcgtcaacacaaaggccgcctggaagccaggatgcaaatcctggaagaccacaataaacagctggagtcacagttacacaggctaaggcagctgctggagcaaccccaggcagaggccaaagtgaatggcacaacggtgtcctctccttctacctctctacagaggtccgacagcagtcagcctatgctgctccgagtggttggcagtcaaacttcggactccatgggtgaggaagatcttctcagtcctccccaggacacaagcacagggttagaggaggtgatggagcaactcaacaactccttccctagttcaagaggaagaaatacccctggaaagccaatgagagaggacacaatgtaggaagtcttttccacatggcagatgatttgggcagagcgatggagtccttagtatcagtcatgacagatgaagaaggagcagaataaatgttttacaactcctgattcccgcatggtttttataatattcatacaacaaagaggattagacagtaagagtttacaagaaataaatctatatttttgtgaagggtagtggtattatactgtagatttcagtagtttctaagtctgttattgttttgttaacaatggcaggttttacacgtctatgcaattgtacaaaaaagttataagaaaactacatgtaaaatcttgatagctaaataacttgccatttctttatatggaacgcattttgggttgtttaaaaatttataacagttataaagaaagattgtaaactaaagtgtgctttataaaaaaaagttgtttataaaaacccctaaaaacaaaacaaacacacacacacacacatacacacacacacacaaaactttgaggcagcgcattgttttgcatccttttggcgtgatatccatatgaaattcatggctttttctttttttgcatattaaagataagacttcctctaccaccacaccaaatgactactacacactgctcatttgagaactgtcagctgagtggggcaggcttgagttttcatttcatatatctatatgtctataagtatataaatactatagttatatagataaagagatacgaatttctatagactgactttttccattttttaaatgttcatgtcacatcctaatagaaagaaattacttctagtcagtcatccaggcttacctgcttggtctagaatggatttttcccggagccggaagccaggaggaaactacaccacactaaaacattgtctacagctccagatgtttctcattttaaacaactttccactgacaacgaaagtaaagtaaagtattggatttttttaaagggaacatgtgaatgaatacacaggacttattatatcagagtgagtaatcggttggttggttgattgattgattgattgatacattcagcttcctgctgctagcaatgccacgatttagatttaatgatgcttcagtggaaatcaatcagaaggtattctgaccttgtgaacatcagaaggtattttttaactcccaagcagtagcaggacgatgatagggctggagggctatggattcccagcccatccctgtgaaggagtaggccactctttaagtgaaggattggatgattgttcataatacataaagttctctgtaattacaactaaattattatgccctcttctcacagtcaaaaggaactgggtggtttggtttttgttgcttttttagatttattgtcccatgtgggatgagtttttaaatgccacaagacataatttaaaataaataaactttgggaaaaggtgtaagacagtagccccatcacatttgtgatactgacaggtatcaacccagaagcccatgaactgtgtttccatcctttgcatttctctgcgagtagttccacacaggtttgtaagtaagtaagaaagaaggcaaattgattcaaatgttacaaaaaaacccttcttggtggattagacaggttaaatatataaacaaacaaacaaaaattgctcaaaaaagaggagaaaagctcaagaggaaaagctaaggactggtaggaaaaagctttactctttcatgccattttatttctttttgatttttaaatcattcattcaatagataccaccgtgtgacctataattttgcaaatctgttacctctgacatcaagtgtaattagcttttggagagtgggctgacatcaagtgtaattagcttttggagagtgggttttgtccattattaataattaattaattaacatcaaacacggcttctcatgctatttctacctcactttggttttggggtgttcctgataattgtgcacacctgagttcacagcttcaccacttgtccattgcgttattttctttttcctttataattctttctttttccttcataattttcaaaagaaaacccaaagctctaaggtaacaaattaccaaattacatgaagatttggtttttgtcttgcatttttttcctttatgtgacgctggaccttttctttacccaaggatttttaaaactcagatttaaaacaaggggttactttacatcctactaagaagtttaagtaagtaagtttcattctaaaatcagaggtaaatagagtgcataaataattttgttttaatctttttgtttttcttttagacacattagctctggagtgagtctgtcataatatttgaacaaaaattgagagctttattgctgcattttaagcataattaatttggacattatttcgtgttgtgttctttataaccaccgagtattaaactgtaaatcataatgtaactgaagcataaacatcacatggcatgttttgtcattgttttcaggtactgagttcttacttgagtatcataatatattgtgttttaacaccaacactgtaacatttacgaattatttttttaaacttcagttttactgcattttcacaacatatcagacttcaccaaatatatgccttactattgtattatagtactgctttactgtgtatctcaataaagcacgcagttatgttac

SEQ ID NO: 3 - protein, 252 aa, Homo sapiens
MLWWEEVEDCYEREDVQKKTFTKWVNAQFSKFGKQHIENLFSDLQDGRRLLDLLEGLTGQKLPKEKGSTRVHALNNVNKALRVLQNNNVDLVNIGSTDIVDGNHKLTLGLIWNIILHWQVKNVMKNIMAGLQQTNSEKILLSWVRQSTRNYPQVNVINFTTSWSDGLALNALIHSHRPDLFDWNSVVCQQSATQRLEHAFNIARYQLGIEKLLDPEDVDTTYPDKKSILMYITSLFQVLPQQVSIEAIQEVE

SEQ ID NO: 4 - protein, 85 aa, Homo sapiens
MLPRPPKVTKEEHFQLHHQMHYSQQITVSLAQGYERTSSPKPRFKSYAYTQAAYVTTSDPTRSPFPSQHLEAPEDKSFGSSLMES

SEQ ID NO: 5 - protein, 109 aa, Homo sapiens
EVNLDRYQTALEEVLSWLLSAEDTLQAQGEISNDVEVVKDQFHTHEGYMMDLTAHQGRVGNILQLGSKLIGTGKLSEDEETEVQEQMNLLNSRWECLRVASMEKQSNLH

SEQ ID NO: 6 - protein, 111 aa, Homo sapiens
RVLMDLQNQKLKELNDWLTKTEERTRKMEEEPLGPDLEDLKRQVQQHKVLQEDLEQEQVRVNSLTHMVVVVDESSGDHATAALEEQLKVLGDRWANICRWTEDRWVLLQDI

SEQ ID NO: 7 - protein, 111 aa, Homo sapiens
LLKWQRLTEEQCLFSAWLSEKEDAVNKIHTTGFKDQNEMLSSLQKLAVLKADLEKKKQSMGKLYSLKQDLLSTLKNKSVTQKTEAWLDNFARCWDNLVQKLEKSTAQISQA

SEQ ID NO: 8 - protein, 49 aa, Homo sapiens
VTTTQPSLTQTTVMETVTTVTTREQILVKHAQEELPPPPPQKKRQITVD

SEQ ID NO: 9 - protein, 111 aa, Homo sapiens
SEIRKRLDVDITELHSWITRSEAVLQSPEFAIFRKEGNFSDLKEKVNAIEREKAEKFRKLQDASRSAQALVEQMVNEGVNADSIKQASEQLNSRWIEFCQLLSERLNWLEY

SEQ ID NO: 10 - protein, 109 aa, Homo sapiens
QNNIIAFYNQLQQLEQMTTTAENWLKIQPTTPSEPTAIKSQLKICKDEVNRLSGLQPQIERLKIQSIALKEKGQGPMFLDADFVAFTNHFKQVFSDVQAREKELQTIFD

SEQ ID NO: 11 - protein, 109 aa, Homo sapiens
TLPPMRYQETMSAIRTWVQQSETKLSIPQLSVTDYEIMEQRLGELQALQSSLQEQQSGLYYLSTTVKEMSKKAPSEISRKYQSEFEEIEGRWKKLSSQLVEHCQKLEEQ

SEQ ID NO: 12 - protein, 109 aa, Homo sapiens
MNKLRKIQNHIQTLKKWMAEVDVFLKEEWPALGDSEILKKQLKQCRLLVSDIQTIQPSLNSVNEGGQKIKNEAEPEFASRLETELKELNTQWDHMCQQVYARKEALKGG

SEQ ID NO: 13 - protein, 109 aa, Homo sapiens
LEKTVSLQKDLSEMHEWMTQAEEEYLERDFEYKTPDELQKAVEEMKRAKEEAQQKEAKVKLLTESVNSVIAQAPPVAQEALKKELETLTTNYQWLCTRLNGKCKTLEEV

SEQ ID NO: 14 - protein, 104 aa, Homo sapiens
WACWHELLSYLEKANKWLNEVEFKLKTTENIPGGAEEISEVLDSLENLMRHSEDNPNQIRILAQTLTDGGVMDELINEELETFNSRWRELHEEAVRRQKLLEQS

SEQ ID NO: 15 - protein, 92 aa, Homo sapiens
IQSAQETEKSLHLIQESLTFIDKQLAAYIADKVDAAQMPQEAQKIQSDLTSHEISLEEMKKHNQGKEAAQRVLSQIDVAQKKLQDVSMKFRL

SEQ ID NO: 16 - protein, 109 aa, Homo sapiens
FQKPANFEQRLQESKMILDEVKMHLPALETKSVEQEVVQSQLNHCVNLYKSLSEVKSEVEMVIKTGRQIVQKKQTENPKELDERVTALKLHYNELGAKVTERKQQLEKC

SEQ ID NO: 17 - protein, 108 aa, Homo sapiens
LKLSRKMRKEMNVLTEWLAATDMELTKRSAVEGMPSNLDSEVAWGKATQKEIEKQKVHLKSITEVGEALKTVLGKKETLVEDKLSLLNSNWIAVTSRAEEWLNLLLEY

SEQ ID NO: 18 - protein, 104 aa, Homo sapiens
QKHMETFDQNVDHITKWIIQADTLLDESEKKKPQQKEDVLKRLKAELNDIRPKVDSTRDQAANLMANRGDHCRKLVEPQISELNHRFAAISHRIKTGKASIPLK

SEQ ID NO: 19 - protein, 94 aa, Homo sapiens
ELEQFNSDIQKLLEPLEAEIQQGVNLKEEDFNKDMNEDNEGTVKELLQRGDNLQQRITDERKREEIKIKQQLLQTKHNALKDLRSQRRKKALEI

SEQ ID NO: 20 - protein, 98 aa, Homo sapiens
SHQWYQYKRQADDLLKCLDDIEKKLASLPEPRDERKIKEIDRELQKKKEELNAVRRQAEGLSEDGAAMAVEPTQIQLSKRWREIESKFAQFRRLNFAQ

SEQ ID NO: 21 - protein, 20 aa, Homo sapiens
IHTVREETMMVMTEDMPLEI

SEQ ID NO: 22 - protein, 109 aa, Homo sapiens
SYVPSTYLTEITHVSQALLEVEQLLNAPDLCAKDFEDLFKQEESLKNIKDSLQQSSGRIDIIHSKKTAALQSATPVERVKLQEALSQLDFQWEKVNKMYKDRQGRFDRS

SEQ ID NO: 23 - protein, 107 aa, Homo sapiens
VEKWRRFHYDIKIFNQWLTEAEQFLRKTQIPENWEHAKYKWYLKELQDGIGQRQTVVRTLNATGEEIIQQSSKTDASILQEKLGSLNLRWQEVCKQLSDRKKRLEEQ

SEQ ID NO: 24 - protein, 117 aa, Homo sapiens
KNILSEFQRDLNEFVLWLEEADNIASIPLEPGKEQQLKEKLEQVKLLVEELPLRQGILKQLNETGGPVLVSAPISPEEQDKLENKLKQTNLQWIKVSRALPEKQGEIEAQIKDLGQL

SEQ ID NO: 25 - protein, 101 aa, Homo sapiens
EKKLEDLEEQLNHLLLWLSPIRNQLEIYNQPNQEGPFDVQETEIAVQAKQPDVEEILSKGQHLYKEKPATQPVKRKLEDLSSEWKAVNRLLQELRAKQPDL

SEQ ID NO: 26 - protein, 41 aa, Homo sapiens
APGLTTIGASPTQTVTLVTQPVVTKETAISKLEMPSSLMLE

SEQ ID NO: 27 - protein, 110 aa, Homo sapiens
VPALADFNRAWTELTDWLSLLDQVIKSQRVMVGDLEDINEMIIKQKATMQDLEQRRPQLEELITAAQNLKNKTSNQEARTIITDRIERIQNQWDEVQEHLQNRRQQLNEM

SEQ ID NO: 28 - protein, 109 aa, Homo sapiens
LKDSTQWLEAKEEAEQVLGQARAKLESWKEGPYTVDAIQKKITETKQLAKDLRQWQTNVDVANDLALKLLRDYSADDTRKVHMITENINASWRSIHKRVSEREAALEET

SEQ ID NO: 29 - protein, 116 aa, Homo sapiens
HRLLQQFPLDLEKFLAWLTEAETTANVLQDATRKERLLEDSKGVKELMKQWQDLQGEIEAHTDVYHNLDENSQKILRSLEGSDDAVLLQRRLDNMNFKWSELRKKSLNIRSHLEAS

SEQ ID NO: 30 - protein, 129 aa, Homo sapiens
SDQWKRLHLSLQELLVWLQLKDDELSRQAPIGGDFPAVQKQNDVHRAFKRELKTKEPVIMSTLETVRIFLTEQPLEGLEKLYQEPRELPPEERAQNVTRLLRKQAEEVNTEWEKLNLHSADWQRKIDET

SEQ ID NO: 31 - protein, 108 aa, Homo sapiens
LERLQELQEATDELDLKLRQAEVIKGSWQPVGDLLIDSLQDHLEKVKALRGEIAPLKENVSHVNDLARQLTTLGIQLSPYNLSTLEDLNTRWKLLQVAVEDRVRQLHE

SEQ ID NO: 32 - protein, 72 aa, Homo sapiens
AHRDFGPASQHFLSTSVQGPWERAISPNKVPYYINHETQTTCWDHPKMTELYQSLADLNNVRFSAYRTAMKL

SEQ ID NO: 33 - protein, 296 aa, Homo sapiens
RRLQKALCLDLLSLSAACDALDQHNLKQNDQPMDILQIINCLTTIYDRLEQEHNNLVNVPLCVDMCLNWLLNVYDTGRTGRIRVLSFKTGIISLCKAHLEDKYRYLFKQVASSTGFCDQRRLGLLLHDSIQIPRQLGEVASFGGSNIEPSVRSCFQFANNKPEIEAALFLDWMRLEPQSMVWLPVLHRVAAAETAKHQAKCNICKECPIIGFRYRSLKHFNYDICQSCFFSGRVAKGHKMHYPMVEYCTPTTSGEDVRDFAKVLKNKFRTKRYFAKHPRMGYLPVQTVLEGDNMET

SEQ ID NO: 34 - protein, 277 aa, Homo sapiens
PVTLINFWPVDSAPASSPQLSHDDTHSRIEHYASRLAEMENSNGSYLNDSISPNESIDDEHLLIQHYCQSLNQDSPLSQPRSPAQILISLESEERGELERILADLEEENRNLQAEYDRLKQQHEHKGLSPLPSPPEMMPTSPQSPRDAELIAEAKLLRQHKGRLEARMQILEDHNKQLESQLHRLRQLLEQPQAEAKVNGTTVSSPSTSLQRSDSSQPMLLRVVGSQTSDSMGEEDLLSPPQDTSTGLEEVMEQLNNSFPSSRGRNTPGKPMREDTM

SEQ ID NO: 35 - DNA, 208 bp, Homo sapiens
gggattccctcactttccccctacaggactcagatctgggaggcaattaccttcggagaaaaacgaataggaaaaactgaagtgttactttttttaaagctgctgaagtttgttggtttctcattgtttttaagcctactggagcaataaagtttgaagaacttttaccaggttttttttatcgctgccttgatatacacttttcaaa

SEQ ID NO: 36 - DNA, 756 bp, Homo sapiens
atgctttggtgggaagaagtagaggactgttatgaaagagaagatgttcaaaagaaaacattcacaaaatgggtaaatgcacaattttctaagtttgggaagcagcatattgagaacctcttcagtgacctacaggatgggaggcgcctcctagacctcctcgaaggcctgacagggcaaaaactgccaaaagaaaaaggatccacaagagttcatgccctgaacaatgtcaacaaggcactgcgggttttgcagaacaataatgttgatttagtgaatattggaagtactgacatcgtagatggaaatcataaactgactcttggtttgatttggaatataatcctccactggcaggtcaaaaatgtaatgaaaaatatcatggctggattgcaacaaaccaacagtgaaaagattctcctgagctgggtccgacaatcaactcgtaattatccacaggttaatgtaatcaacttcaccaccagctggtctgatggcctggctttgaatgctctcatccatagtcataggccagacctatttgactggaatagtgtggtttgccagcagtcagccacacaacgactggaacatgcattcaacatcgccagatatcaattaggcatagagaaactactcgatcctgaagatgttgataccacctatccagataagaagtccatcttaatgtacatcacatcactcttccaagttttgcctcaacaagtgagcattgaagccatccaggaagtggaa

SEQ ID NO: 37 - DNA, 255 bp, Homo sapiens
atgttgccaaggccacctaaagtgactaaagaagaacattttcagttacatcatcaaatgcactattctcaacagatcacggtcagtctagcacagggatatgagagaacttcttcccctaagcctcgattcaagagctatgcctacacacaggctgcttatgtcaccacctctgaccctacacggagcccatttccttcacagcatttggaagctcctgaagacaagtcatttggcagttcattgatggagagt

SEQ ID NO: 38 - DNA, 327 bp, Homo sapiens
gaagtaaacctggaccgttatcaaacagctttagaagaagtattatcgtggcttctttctgctgaggacacattgcaagcacaaggagagatttctaatgatgtggaagtggtgaaagaccagtttcatactcatgaggggtacatgatggatttgacagcccatcagggccgggttggtaatattctacaattgggaagtaagctgattggaacaggaaaattatcagaagatgaagaaactgaagtacaagagcagatgaatctcctaaattcaagatgggaatgcctcagggtagctagcatggaaaaacaaagcaatttacat

SEQ ID NO: 39 - DNA, 333 bp, Homo sapiens
agagttttaatggatctccagaatcagaaactgaaagagttgaatgactggctaacaaaaacagaagaaagaacaaggaaaatggaggaagagcctcttggacctgatcttgaagacctaaaacgccaagtacaacaacataaggtgcttcaagaagatctagaacaagaacaagtcagggtcaattctctcactcacatggtggtggtagttgatgaatctagtggagatcacgcaactgctgctttggaagaacaacttaaggtattgggagatcgatgggcaaacatctgtagatggacagaagaccgctgggttcttttacaagacatc

SEQ ID NO: 40 - DNA, 333 bp, Homo sapiens
cttctcaaatggcaacgtcttactgaagaacagtgcctttttagtgcatggctttcagaaaaagaagatgcagtgaacaagattcacacaactggctttaaagatcaaaatgaaatgttatcaagtcttcaaaaactggccgttttaaaagcggatctagaaaagaaaaagcaatccatgggcaaactgtattcactcaaacaagatcttctttcaacactgaagaataagtcagtgacccagaagacggaagcatggctggataactttgcccggtgttgggataatttagtccaaaaacttgaaaagagtacagcacagatttcacaggct

SEQ ID NO: 41 - DNA, 147 bp, Homo sapiens
gtcaccaccactcagccatcactaacacagacaactgtaatggaaacagtaactacggtgaccacaagggaacagatcctggtaaagcatgctcaagaggaacttccaccaccacctccccaaaagaagaggcagattactgtggat

SEQ ID NO: 42 - DNA, 333 bp, Homo sapiens
tctgaaattaggaaaaggttggatgttgatataactgaacttcacagctggattactcgctcagaagctgtgttgcagagtcctgaatttgcaatctttcggaaggaaggcaacttctcagacttaaaagaaaaagtcaatgccatagagcgagaaaaagctgagaagttcagaaaactgcaagatgccagcagatcagctcaggccctggtggaacagatggtgaatgagggtgttaatgcagatagcatcaaacaagcctcagaacaactgaacagccggtggatcgaattctgccagttgctaagtgagagacttaactggctggagtat

SEQ ID NO: 43 - DNA, 327 bp, Homo sapiens
cagaacaacatcatcgctttctataatcagctacaacaattggagcagatgacaactactgctgaaaactggttgaaaatccaacccaccaccccatcagagccaacagcaattaaaagtcagttaaaaatttgtaaggatgaagtcaaccggctatcaggtcttcaacctcaaattgaacgattaaaaattcaaagcatagccctgaaagagaaaggacaaggacccatgttcctggatgcagactttgtggcctttacaaatcattttaagcaagtcttttctgatgtgcaggccagagagaaagagctacagacaatttttgac

SEQ ID NO: 44 - DNA, 327 bp, Homo sapiens
actttgccaccaatgcgctatcaggagaccatgagtgccatcaggacatgggtccagcagtcagaaaccaaactctccatacctcaacttagtgtcaccgactatgaaatcatggagcagagactcggggaattgcaggctttacaaagttctctgcaagagcaacaaagtggcctatactatctcagcaccactgtgaaagagatgtcgaagaaagcgccctctgaaattagccggaaatatcaatcagaatttgaagaaattgagggacgctggaagaagctctcctcccagctggttgagcattgtcaaaagctagaggagcaa

SEQ ID NO: 45 - DNA, 327 bp, Homo sapiens
atgaataaactccgaaaaattcagaatcacatacaaaccctgaagaaatggatggctgaagttgatgtttttctgaaggaggaatggcctgcccttggggattcagaaattctaaaaaagcagctgaaacagtgcagacttttagtcagtgatattcagacaattcagcccagtctaaacagtgtcaatgaaggtgggcagaagataaagaatgaagcagagccagagtttgcttcgagacttgagacagaactcaaagaacttaacactcagtgggatcacatgtgccaacaggtctatgccagaaaggaggccttgaagggaggt

SEQ ID NO: 46 - DNA, 327 bp, Homo sapiens
ttggagaaaactgtaagcctccagaaagatctatcagagatgcacgaatggatgacacaagctgaagaagagtatcttgagagagattttgaatataaaactccagatgaattacagaaagcagttgaagagatgaagagagctaaagaagaggcccaacaaaaagaagcgaaagtgaaactccttactgagtctgtaaatagtgtcatagctcaagctccacctgtagcacaagaggccttaaaaaaggaacttgaaactctaaccaccaactaccagtggctctgcactaggctgaatgggaaatgcaagactttggaagaagtt

SEQ ID NO: 47 - DNA, 312 bp, Homo sapiens
tgggcatgttggcatgagttattgtcatacttggagaaagcaaacaagtggctaaatgaagtagaatttaaacttaaaaccactgaaaacattcctggcggagctgaggaaatctctgaggtgctagattcacttgaaaatttgatgcgacattcagaggataacccaaatcagattcgcatattggcacagaccctaacagatggcggagtcatggatgagctaatcaatgaggaacttgagacatttaattctcgttggagggaactacatgaagaggctgtaaggaggcaaaagttgcttgaacagagc

SEQ ID NO: 48 - DNA, 276 bp, Homo sapiens
atccagtctgcccaggagactgaaaaatccttacacttaatccaggagtccctcacattcattgacaagcagttggcagcttatattgcagacaaggtggacgcagctcaaatgcctcaggaagcccagaaaatccaatctgatttgacaagtcatgagatcagtttagaagaaatgaagaaacataatcaggggaaggaggctgcccaaagagtcctgtctcagattgatgttgcacagaaaaaattacaagatgtctccatgaagtttcgatta

SEQ ID NO: 49 - DNA, 327 bp, Homo sapiens
ttccagaaaccagccaattttgagctgcgtctacaagaaagtaagatgattttagatgaagtgaagatgcacttgcctgcattggaaacaaagagtgtggaacaggaagtagtacagtcacagctaaatcattgtgtgaacttgtataaaagtctgagtgaagtgaagtctgaagtggaaatggtgataaagactggacgtcagattgtacagaaaaagcagacggaaaatcccaaagaacttgatgaaagagtaacagctttgaaattgcattataatgagctgggagcaaaggtaacagaaagaaagcaacagttggagaaatgc

SEQ ID NO: 50 - DNA, 324 bp, Homo sapiens
ttgaaattgtcccgtaagatgcgaaaggaaatgaatgtcttgacagaatggctggcagctacagatatggaattgacaaagagatcagcagttgaaggaatgcctagtaatttggattctgaagttgcctggggaaaggctactcaaaaagagattgagaaacagaaggtgcacctgaagagtatcacagaggtaggagaggccttgaaaacagttttgggcaagaaggagacgttggtggaagataaactcagtcttctgaatagtaactggatagctgtcacctcccgagcagaagagtggttaaatcttttgttggaatac

SEQ ID NO: 51 - DNA, 312 bp, Homo sapiens
cagaaacacatggaaacttttgaccagaatgtggaccacatcacaaagtggatcattcaggctgacacacttttggatgaatcagagaaaaagaaaccccagcaaaaagaagacgtgcttaagcgtttaaaggcagaactgaatgacatacgcccaaaggtggactctacacgtgaccaagcagcaaacttgatggcaaaccgcggtgaccactgcaggaaattagtagagccccaaatctcagagctcaaccatcgatttgcagccatttcacacagaattaagactggaaaggcctccattcctttgaag

SEQ ID NO: 52 - DNA, 282 bp, Homo sapiens
gaattggagcagtttaactcagatatacaaaaattgcttgaaccactggaggctgaaattcagcagggggtgaatctgaaagaggaagacttcaataaagatatgaatgaagacaatgagggtactgtaaaagaattgttgcaaagaggagacaacttacaacaaagaatcacagatgagagaaagagagaggaaataaagataaaacagcagctgttacagacaaaacataatgctctcaaggatttgaggtctcaaagaagaaaaaaggctctagaaatt

SEQ ID NO: 53 - DNA, 294 bp, Homo sapiens
tctcatcagtggtatcagtacaagaggcaggctgatgatctcctgaaatgcttggatgacattgaaaaaaaattagccagcctacctgagcccagagatgaaaggaaaataaaggaaattgatcgggaattgcagaagaagaaagaggagctgaatgcagtgcgtaggcaagctgagggcttgtctgaggatggggccgcaatggcagtggagccaactcagatccagctcagcaagcgctggcgggaaattgagagcaaatttgctcagtttcgaagactcaactttgcacaa

SEQ ID NO: 54 - DNA, 60 bp, Homo sapiens
attcacactgtccgtgaagaaacgatgatggtgatgactgaagacatgcctttggaaatt

SEQ ID NO: 55 - DNA, 327 bp, Homo sapiens
tcttatgtgccttctacttatttgactgaaatcactcatgtctcacaagccctattagaagtggaacaacttctcaatgctcctgacctctgtgctaaggactttgaagatctctttaagcaagaggagtctctgaagaatataaaagatagtctacaacaaagctcaggtcggattgacattattcatagcaagaagacagcagcattgcaaagtgcaacgcctgtggaaagggtgaagctacaggaagctctctcccagcttgatttccaatgggaaaaagttaacaaaatgtacaaggaccgacaagggcgatttgacagatct

SEQ ID NO: 56 - DNA, 321 bp, Homo sapiens
gttgagaaatggcggcgttttcattatgatataaagatatttaatcagtggctaacagaagctgaacagtttctcagaaagacacaaattcctgagaattgggaacatgctaaatacaaatggtatcttaaggaactccaggatggcattgggcagcggcaaactgttgtcagaacattgaatgcaactggggaagaaataattcagcaatcctcaaaaacagatgccagtattctacaggaaaaattgggaagcctgaatctgcggtggcaggaggtctgcaaacagctgtcagacagaaaaaagaggctagaagaacaa

SEQ ID NO: 57 - DNA, 351 bp, Homo sapiens
aagaatatcttgtcagaatttcaaagagatttaaatgaatttgttttatggttggaggaagcagataacattgctagtatcccacttgaacctggaaaagagcagcaactaaaagaaaagcttgagcaagtcaagttactggtggaagagttgcccctgcgccagggaattctcaaacaattaaatgaaactggaggacccgtgcttgtaagtgctcccataagcccagaagagcaagataaacttgaaaataagctcaagcagacaaatctccagtggataaaggtttccagagctttacctgagaaacaaggagaaattgaagctcaaataaaagaccttgggcagctt

SEQ ID NO: 58 - DNA, 303 bp, Homo sapiens
gaaaaaaagcttgaagaccttgaagagcagttaaatcatctgctgctgtggttatctcctattaggaatcagttggaaatttataaccaaccaaaccaagaaggaccatttgacgttcaggaaactgaaatagcagttcaagctaaacaaccggatgtggaagagattttgtctaaagggcagcatttgtacaaggaaaaaccagccactcagccagtgaagaggaagttagaagatctgagctctgagtggaaggcggtaaaccgtttacttcaagagctgagggcaaagcagcctgaccta

SEQ ID NO: 59 - DNA, 123 bp, Homo sapiens
gctcctggactgaccactattggagcctctcctactcagactgttactctggtgacacaacctgtggttactaaggaaactgccatctccaaactagaaatgccatcttccttgatgttggag

SEQ ID NO: 60 - DNA, 330 bp, Homo sapiens
gtacctgctctggcagatttcaaccgggcttggacagaacttaccgactggctttctctgcttgatcaagttataaaatcacagagggtgatggtgggtgaccttgaggatatcaacgagatgatcatcaagcagaaggcaacaatgcaggatttggaacagaggcgtccccagttggaagaactcattaccgctgcccaaaatttgaaaaacaagaccagcaatcaagaggctagaacaatcattacggatcgaattgaaagaattcagaatcagtgggatgaagtacaagaacaccttcagaaccggaggcaacagttgaatgaaatg

SEQ ID NO: 61 - DNA, 327 bp, Homo sapiens
ttaaaggattcaacacaatggctggaagctaaggaagaagctgagcaggtcttaggacaggccagagccaagcttgagtcatggaaggagggtccctatacagtagatgcaatccaaaagaaaatcacagaaaccaagcagttggccaaagacctccgccagtggcagacaaatgtagatgtggcaaatgacttggccctgaaacttctccgggattattctgcagatgataccagaaaagtccacatgataacagagaatatcaatgcctcttggagaagcattcataaaagggtgagtgagcgagaggctgctttggaagaaact

SEQ ID NO: 62 - DNA, 348 bp, Homo sapiens
catagattactgcaacagttccccctggacctggaaaagtttcttgcctggcttacagaagctgaaacaactgccaatgtcctacaggatgctacccgtaaggaaaggctcctagaagactccaagggagtaaaagagctgatgaaacaatggcaagacctccaaggtgaaattgaagctcacacagatgtttatcacaacctggatgaaaacagccaaaaaatcctgagatccctggaaggttccgatgatgcagtcctgttacaaagacgtttggataacatgaacttcaagtggagtgaacttcggaaaaagtctctcaacattaggtcccatttggaagccagt

SEQ ID NO: 63 - DNA, 387 bp, Homo sapiens
tctgaccagtggaagcgtctgcacctttctctgcaggaacttctggtgtggctacagctgaaagatgatgaattaagccggcaggcacctattggaggcgactttccagcagttcagaagcagaacgatgtacatagggccttcaagagggaattgaaaactaaagaacctgtaatcatgagtactcttgagactgtacgaatatttctgacagagcagcctttggaaggactagagaaactctaccaggagcccagagagctgcctcctgaggagagagcccagaatgtcactcggcttctacgaaagcaggctgaggaggtcaatactgagtgggaaaaattgaacctgcactccgctgactggcagagaaaaatagatgagacc

SEQ ID NO: 64 - DNA, 324 bp, Homo sapiens
cttgaaagactccaggaacttcaagaggccacggatgagctggacctcaagctgcgccaagctgaggtgatcaagggatcctggcagcccgtgggcgatctcctcattgactctctccaagatcacctcgagaaagtcaaggcacttcgaggagaaattgcgcctctgaaagagaacgtgagccacgtcaatgaccttgctcgccagcttaccactttgggcattcagctctcaccgtataacctcagcactctggaagacctgaacaccagatggaagcttctgcaggtggccgtcgaggaccgagtcaggcagctgcatgaa

SEQ ID NO: 65 - DNA, 216 bp, Homo sapiens
gcccacagggactttggtccagcatctcagcactttctttccacgtctgtccagggtccctgggagagagccatctcgccaaacaaagtgccctactatatcaaccacgagactcaaacaacttgctgggaccatcccaaaatgacagagctctaccagtctttagctgacctgaataatgtcagattctcagcttataggactgccatgaaactc

SEQ ID NO: 66 - DNA, 888 bp, Homo sapiens
cgaagactgcagaaggccctttgcttggatctcttgagcctgtcagctgcatgtgatgccttggaccagcacaacctcaagcaaaatgaccagcccatggatatcctgcagattattaattgtttgaccactatttatgaccgcctggagcaagagcacaacaatttggtcaacgtccctctctgcgtggatatgtgtctgaactggctgctgaatgtttatgatacgggacgaacagggaggatccgtgtcctgtcttttaaaactggcatcatttccctgtgtaaagcacatttggaagacaagtacagataccttttcaagcaagtggcaagttcaacaggattttgtgaccagcgcaggctgggcctccttctgcatgattctatccaaattccaagacagttgggtgaagttgcatcctttgggggcagtaacattgagccaagtgtccggagctgcttccaatttgctaataataagccagagatcgaagcggccctcttcctagactggatgagactggaaccccagtccatggtgtggctgcccgtcctgcacagagtggctgctgcagaaactgccaagcatcaggccaaatgtaacatctgcaaagagtgtccaatcattggattcaggtacaggagtctaaagcactttaattatgacatctgccaaagctgctttttttctggtcgagttgcaaaaggccataaaatgcactatcccatggtggaatattgcactccgactacatcaggagaagatgttcgagactttgccaaggtactaaaaaacaaatttcgaaccaaaaggtattttgcgaagcatccccgaatgggctacctgccagtgcagactgtcttagagggggacaacatggaaact

SEQ ID NO: 67 - DNA, 834 bp, Homo sapiens
cccgttactctgatcaacttctggccagtagattctgcgcctgcctcgtcccctcagctttcacacgatgatactcattcacgcattgaacattatgctagcaggctagcagaaatggaaaacagcaatggatcttatctaaatgatagcatctctcctaatgagagcatagatgatgaacatttgttaatccagcattactgccaaagtttgaaccaggactcccccctgagccagcctcgtagtcctgcccagatcttgatttccttagagagtgaggaaagaggggagctagagagaatcctagcagatcttgaggaagaaaacaggaatctgcaagcagaatatgaccgtctaaagcagcagcacgaacataaaggcctgtccccactgccgtcccctcctgaaatgatgcccacctctccccagagtccccgggatgctgagctcattgctgaggccaagctactgcgtcaacacaaaggccgcctggaagccaggatgcaaatcctggaagaccacaataaacagctggagtcacagttacacaggctaaggcagctgctggagcaaccccaggcagaggccaaagtgaatggcacaacggtgtcctctccttctacctctctacagaggtccgacagcagtcagcctatgctgctccgagtggttggcagtcaaacttcggactccatgggtgaggaagatcttctcagtcctccccaggacacaagcacagggttagaggaggtgatggagcaactcaacaactccttccctagttcaagaggaagaaatacccctggaaagccaatgagagaggacacaatgtag

SEQ ID NO: 68 - protein, 252 aa, Homo sapiens; identical to SEQ ID NO: 3

SEQ ID NO: 69 - protein, 85 aa, Homo sapiens; identical to SEQ ID NO: 4

SEQ ID NO: 70 - protein, 109 aa, Homo sapiens; identical to SEQ ID NO: 5

SEQ ID NO: 71 - protein, 2 aa, Homo sapiens
  MISC_FEATURE: RV-Linker
RV

SEQ ID NO: 72 - protein, 111 aa, Homo sapiens; identical to SEQ ID NO: 7

SEQ ID NO: 73 - protein, 49 aa, Homo sapiens; identical to SEQ ID NO: 8

SEQ ID NO: 74 - protein, 4 aa, Homo sapiens
  MISC_FEATURE: SEAQ linker
SEAQ

SEQ ID NO: 75 - protein, 20 aa, Homo sapiens
IHTVREETMMVMTEDMPLEI

SEQ ID NO: 76 - protein, 109 aa, Homo sapiens; identical to SEQ ID NO: 22

SEQ ID NO: 77 - protein, 107 aa, Homo sapiens; identical to SEQ ID NO: 23

SEQ ID NO: 78 - protein, 108 aa, Homo sapiens; identical to SEQ ID NO: 31

SEQ ID NO: 79 - protein, 72 aa, Homo sapiens; identical to SEQ ID NO: 32

SEQ ID NO: 80 - protein, 299 aa, Homo sapiens
RRLQKALCLDLLSLSAACDALDQHNLKQNDQPMDILQIINCLTTIYDRLEQEHNNLVNVPLCVDMCLNWLLNVYDTGRTGRIRVLSFKTGIISLCKAHLEDKYRYLFKQVASSTGFCDQRRLGLLLHDSIQIPRQLGEVASFGGSNIEPSVRSCFQFANNKPEIEAALFLDWMRLEPQSMVWLPVLHRVAAAETAKHQAKCNICKECPIIGFRYRSLKHFNYDICQSCFFSGRVAKGHKMHYPMVEYCTPTTSGEDVRDFAKVLKNKFRTKRYFAKHPRMGYLPVQTVLEGDNMETDTM

SEQ ID NO: 81 - protein, 252 aa, Homo sapiens; identical to SEQ ID NO: 3

SEQ ID NO: 82 - protein, 85 aa, Homo sapiens; identical to SEQ ID NO: 4

SEQ ID NO: 83 - protein, 109 aa, Homo sapiens; identical to SEQ ID NO: 5

SEQ ID NO: 84 - protein, 20 aa, Homo sapiens
IHTVREETMMVMTEDMPLEI

SEQ ID NO: 85 - protein, 109 aa, Homo sapiens; identical to SEQ ID NO: 22

SEQ ID NO: 86 - protein, 107 aa, Homo sapiens; identical to SEQ ID NO: 23

SEQ ID NO: 87 - protein, 41 aa, Homo sapiens; identical to SEQ ID NO: 26

SEQ ID NO: 88 - protein, 129 aa, Homo sapiens; identical to SEQ ID NO: 30

SEQ ID NO: 89 - protein, 108 aa, Homo sapiens; identical to SEQ ID NO: 31

SEQ ID NO: 90 - protein, 72 aa, Homo sapiens; identical to SEQ ID NO: 32

SEQ ID NO: 91 - protein, 352 aa, Homo sapiens
RRLQKALCLDLLSLSAACDALDQHNLKQNDQPMDILQIINCLTTIYDRLEQEHNNLVNVPLCVDMCLNWLLNVYDTGRTGRIRVLSFKTGIISLCKAHLEDKYRYLFKQVASSTGFCDQRRLGLLLHDSIQIPRQLGEVASFGGSNIEPSVRSCFQFANNKPEIEAALFLDWMRLEPQSMVWLPVLHRVAAAETAKHQAKCNICKECPIIGFRYRSLKHFNYDICQSCFFSGRVAKGHKMHYPMVEYCTPTTSGEDVRDFAKVLKNKFRTKRYFAKHPRMGYLPVQTVLEGDNMETPAQILISLESEERGELERILADLEEENRNLQAEYDRLKQQHEHKGLSPLPSPPDTM

SEQ ID NO: 92 - DNA, 322 bp, Homo sapiens
ccgccttcggcaccattcctcacgacacccaaatatggcacgggtgaggaatggtggggagttattttagagcggtgaggaaggtgggcaggcagcaggtgttggcgctctaaaaataactcccgggagttattttagagcggaggaatggtggacacccaaataggcgacggttcctcacccgtcgccatatttgggtgtccgccctcggccggggccgcattcctggggccgggcggtgctcccgcccgcctcgataaaaggctccggggccggcggcggcccacgagctacccggaggagcgggaggctctagaccacc

SEQ ID NO: 93 - DNA, 756 bp, Homo sapiens
atgctgtggtgggaggaagtggaagattgctacgagcgcgaggacgtgcagaagaaaaccttcaccaaatgggtgaacgcccagttcagcaagttcggcaagcagcacatcgagaacctgttcagcgacctgcaggacggcagacggctgctggacctgctggaaggcctgaccggccagaagctgcccaaagagaagggcagcaccagagtgcacgccctgaacaacgtgaacaaggccctgcgggtgctgcagaacaacaacgtggacctggtgaacatcggcagcaccgacatcgtggacggcaaccacaagctgaccctgggcctgatctggaacatcatcctgcactggcaggtcaaaaacgtgatgaagaacatcatggccggcctgcagcagaccaacagcgagaagatcctgctgagctgggtgcgccagagcacccggaactacccccaggtcaacgtgatcaacttcaccacctcttggagcgacggcctggccctgaacgccctgatccacagccaccggcccgacctgttcgactggaacagcgtggtctgccagcagagcgccacccagcggctggaacacgccttcaatatcgccagataccagctgggcatcgagaagctgctggatcccgaggacgtggacaccacctaccccgacaagaaatccatcctgatgtatatcaccagcctgttccaggtgctgccccagcaggtgtccatcgaggccatccaggaagtggaa

SEQ ID NO: 94 - DNA, 255 bp, Homo sapiens
atgctgcccagaccccccaaagtgaccaaagaggaacacttccagctgcaccaccagatgcactacagccagcagatcaccgtgtccctggcccagggctacgagagaaccagcagccccaagccccggttcaagagctacgcctatacccaggccgcctacgtgaccaccagcgaccctaccagaagcccattccccagccagcatctggaagcccccgaggacaagagcttcggcagcagcctgatggaaagc

SEQ ID NO: 95 - DNA, 327 bp, Homo sapiens
gaagtgaacctggacagataccagaccgccctggaagaggtgctgagctggctgctgagcgccgaggatacactgcaggctcagggcgagatcagcaacgacgtggaagtcgtgaaggaccagttccacacccacgagggctacatgatggacctgacagcccaccagggcagagtgggcaacatcctgcagctgggctccaagctgatcggcaccggcaagctgagcgaggacgaagagacagaggtgcaggaacagatgaacctgctgaacagcagatgggagtgcctgcgggtggccagcatggaaaagcagagcaacctgcat

SEQ ID NO: 96 - DNA, 6 bp, Homo sapiens
agggtc

SEQ ID NO: 97 - DNA, 333 bp, Homo sapiens
ctgctgaagtggcagcggctgaccgaggaacagtgcctgtttagcgcctggctgtccgagaaagaggacgccgtgaacaagatccacaccaccggcttcaaggaccagaacgagatgctgagcagcctgcagaaactggccgtgctgaaggccgacctggaaaagaaaaagcagtccatgggcaagctgtactccctgaagcaggacctgctgtccaccctgaagaacaagagcgtgacccagaaaaccgaggcctggctggacaacttcgcccggtgctgggacaacctggtgcagaagctggaaaagtccaccgcccagatctcccaggcc

SEQ ID NO: 98 - DNA, 147 bp, Homo sapiens
gtgaccacaacacagcccagcctgacccagaccaccgtgatggaaaccgtgacaacagtgaccacccgggaacagatcctcgtgaagcacgcccaggaagaactgccccctccacccccccagaagaaacggcagatcacagtggac

SEQ ID NO: 99 - DNA, 12 bp, Homo sapiens
agtgaagctcag

SEQ ID NO: 100 - DNA, 60 bp, Homo sapiens
atccacaccgtgcgggaagagacaatgatggtcatgacagaggacatgcccctggaaatc

SEQ ID NO: 101 - DNA, 327 bp, Homo sapiens
agctacgtgcccagcacctacctgaccgagatcacccatgtgtcccaggccctgctggaagtggaacagctgctgaacgcccccgacctgtgcgccaaggatttcgaggacctgttcaagcaggaagagagcctgaagaatatcaaggatagcctgcagcagagcagcggccggatcgacatcatccacagcaagaaaacagccgccctgcagagcgccacccccgtggaaagagtgaaactgcaggaagccctgtcccagctggacttccagtgggagaaagtgaacaaaatgtacaaggaccggcagggcagattcgaccgcagc

SEQ ID NO: 102 - DNA, 321 bp, Homo sapiens
gtggaaaagtggcggcggttccactacgacatcaagatcttcaaccagtggctgacagaggccgagcagttcctgagaaagacccagatccccgagaactgggagcacgccaagtacaagtggtatctgaaagagctgcaggacggcatcggccagagacagacagtcgtgcggaccctgaatgccaccggcgaggaaatcatccagcagtccagcaagaccgacgccagcattctgcaggaaaagctgggcagcctgaacctgcggtggcaggaagtgtgcaagcagctgtccgaccggaagaagcggctggaagaacag

SEQ ID NO: 103 - DNA, 324 bp, Homo sapiens
ctggaacggctgcaggaactgcaggaggccaccgacgagctggacctgaaactgagacaggccgaagtgatcaagggcagctggcagccagtgggcgacctgctgatcgactccctgcaggaccatctggaaaaagtgaaggccctgagaggcgagatcgcccccctgaaagaaaacgtgtcccacgtgaacgacctggcccggcagctgacaacactgggcattcagctgagcccctacaacctgagcacactggaagatctgaacacccggtggaagctgctgcaggtggccgtggaagatagagtgcggcagctgcacgag

SEQ ID NO: 104 - DNA, 215 bp, Homo sapiens
gcccacagagattttggccctgcctcccagcacttcctgagcaccagtgtgcagggcccttgggagagagccatctcccctaacaaggtgccctactacatcaaccacgagacacagaccacctgttgggaccaccccaagatgaccgagctgtaccagagcctggctgacctgaacaacgtgcggttcaggcctaccggaccgccatgaagctg

SEQ ID NO: 105 - DNA, 1068 bp, Homo sapiens
cggagactgcagaaagctctgtgcctggatctgctgtccctgtccgccgcctgtgatgccctggaccagcacaatctgaagcagaacgaccagcccatggatatcctgcagatcatcaactgcctgaccaccatctacgaccggctggaacaggaacacaacaatctcgtgaacgtgcccctgtgcgtggacatgtgcctgaattggctgctgaatgtgtacgacaccggccggacaggccggatcagagtgctgtccttcaagaccggcatcatcagcctgtgcaaagcccacctggaagataagtaccggtatctgttcaaacaggtggcctctagcaccggcttttgcgaccagagaaggctgggcctgctgctgcacgacagcatccagatccctagacagctgggcgaagtggccagctttggcggcagcaacatcgagcctagcgtgcggagctgcttccagttcgccaacaacaagcccgagatcgaggccgccctgttcctggactggatgagactggaaccccagagcatggtgtggctgcccgtgctgcatagagtggccgctgccgagacagccaagcaccaggccaagtgcaacatctgcaaagagtgccccatcatcggcttccggtacagaagcctgaagcacttcaactacgatatctgccagagctgtttcttcagcggcagggtggccaagggccacaaaatgcactaccccatggtggaatactgcacccccaccacaagcggcgaggatgtgcgggatttcgccaaggtgctgaaaaacaagttccggaccaagcggtacttcgccaaacacccccggatgggctacctgcctgtgcagacagtgctggaaggcgacaacatggaaaccgacaccatgtgatgatgatttgggcagagcgatggagtccttagtatcagtcatgacagatgaagaaggagcagaataaatgttttacaactcctgattcccgcatgcggccagcttatcgataccgtcgaaataaaagatccttattttcattggatctgtgtgttggttttttgtgtg

SEQ ID NO: 106 - DNA, 334 bp, Homo sapiens
cctgcggccgccttcggcaccattcctcacgacacccaaatatggcgacgggtgaggaatggtggggagttatttttagagcggtgaggaaggtgggcaggcagcaggtgttggcgctctaaaaataactcccgggagttatttttagagcggaggaatggtggacacccaaatatggcgacggttcctcacccgtcgccatatttgggtgtccgccctcggccggggccgcattcctgggggccgggcggtgctcccgcccgcctcgataaaaggctccggggccggcggcggcccacgagctacccggaggagcgggaggctctagaccacc

SEQ ID NO: 107 - DNA, 756 bp, Homo sapiens; identical to SEQ ID NO: 93

SEQ ID NO: 108 - DNA, 255 bp, Homo sapiens
atgctgcccagaccccccaaagtgaccaaagaggaacacttccagctgcaccaccagatgcactacagccagcagatcaccgtgtccctggctcagggctacgagcggaccagcagccccaagccccggttcaagagctacgcctacacccaggccgcctacgtgaccaccagcgaccccaccagaagcccattccccagccagcatctggaagcccccgaggacaagagcttcggcagcagcctgatggaaagc

SEQ ID NO: 109 - DNA, 327 bp, Homo sapiens
gaagtgaacctggacagataccagaccgccctggaagaggtgctgtcctggctgctgagcgccgaggatacactgcaggcccagggcgagatcagcaacgacgtggaagtggtgaaagaccagttccacacccacgagggctacatgatggacctgaccgcccaccagggcagagtgggcaacatcctgcagctgggcagcaagctgatcggcaccggcaagctgagcgaggacgaagagacagaggtgcaggaacagatgaacctgctgaacagcagatgggagtgcctgcgggtggccagcatggaaaagcagagcaacctgcac

SEQ ID NO: 110 - DNA, 60 bp, Homo sapiens
atccacaccgtgcgggaagagacaatgatggtgatgaccgaggacatgcccctggaaatc

SEQ ID NO: 111 - DNA, 327 bp, Homo sapiens
agctacgtgcccagcacctacctgaccgagatcacccacgtgtcccaggctctgctggaagtggaacagctgctgaacgcccccgacctgtgcgccaaggacttcgaggatctgttcaagcaggaagagagcctgaagaatatcaaggactccctgcagcagtccagcggccggatcgacatcatccacagcaagaaaacagccgccctgcagtccgccacccccgtggaaagagtgaagctgcaggaagccctgagccagctggacttccagtgggagaaagtgaacaagatgtacaaggaccggcagggcagattcgaccgcagc

SEQ ID NO: 112 - DNA, 321 bp, Homo sapiens
gtggaaaagtggcggcggttccactacgacatcaagatcttcaaccagtggctgaccgaggccgagcagttcctgagaaagacccagatccccgagaactgggagcacgccaagtacaagtggtatctgaaagaactgcaggatggcatcggccagcggcagaccgtggtgcgcacactgaatgccaccggcgaggaaatcatccagcagagcagcaagaccgacgccagcatcctgcaggaaaagctgggctccctgaacctgcggtggcaggaagtgtgcaagcagctgagcgaccggaagaagaggctggaagaacag

SEQ ID NO: 113 - DNA, 123 bp, Homo sapiens
gcccctggcctgaccaccatcggcgccagccctacccagaccgtgaccctggtgacacagcccgtggtgacaaaagagacagccatctccaagctggaaatgcccagctccctgatgctggaa

SEQ ID NO: 114 - DNA, 387 bp, Homo sapiens; identical to SEQ ID NO: 63

SEQ ID NO: 115 - DNA, 324 bp, Homo sapiens
ctggaaaggctgcaggaactgcaggaggccaccgacgagctggacctgaagctgcggcaggccgaagtgatcaagggcagctggcagcccgtgggcgacctgctgatcgacagcctgcaggaccacctggaaaaagtgaaggccctgagaggcgagatcgcccccctgaaagaaaacgtgtcccacgtgaacgacctggcccggcagctgaccaccctgggcatccagctgagcccctacaacctgagcaccctggaagatctgaacacccggtggaagctgctgcaggtggccgtggaagatagagtgcggcagctgcacgag

SEQ ID NO: 116 - DNA, 216 bp, Homo sapiens
gcccacagagactttggccctgccagccagcacttcctgagcacctctgtgcagggaccctgggagagagccatcagccccaacaaggtgccctactacatcaaccacgagacacagaccacctgttgggaccaccccaagatgaccgagctgtaccagagcctggccgacctgaacaatgtgcggttcagcgcctaccggaccgccatgaagctg

SEQ ID NO: 117 - DNA, 1059 bp, Homo sapiens
aggcggctgcagaaagctctgtgcctggatctgctgagcctgagcgccgcctgcgacgccctggaccagcacaacctgaagcagaacgaccagcccatggatatcctgcagatcatcaactgcctgaccacaatctacgacaggctggaacaggaacacaacaatctggtcaacgtgcccctgtgcgtggacatgtgcctgaattggctgctgaatgtgtacgacaccggccggaccggcagaatccgggtgctgagcttcaagaccggcatcatcagcctgtgcaaggcccacctggaagataagtaccgctacctgttcaaacaggtggccagctccaccggcttttgcgaccagcggagactgggcctgctgctgcacgacagcatccagatccccagacagctgggcgaggtggcctccttcggcggcagcaacattgagcccagcgtgcggagctgcttccagttcgccaacaacaagcccgagatcgaggccgccctgttcctggactggatgagactggaaccccagagcatggtgtggctgcccgtgctgcatcgggtggccgctgccgagacagccaagcaccaggccaagtgcaacatctgcaaagagtgccccatcatcggcttccggtacagaagcctgaagcacttcaactacgatatctgccagagctgcttcttcagcggcagagtggccaagggccacaaaatgcactaccccatggtggaatactgcacccccaccaccagcggcgaggatgtgcgggacttcgccaaggtgctgaaaaacaagttccggaccaagcggtactttgccaagcacccccggatgggctacctgcccgtgcagacagtgctggaaggcgacaacatggaaacccctgcccagatcctgatcagcctggaaagcgaggaacggggcgagctggaacggatcctggccgatctggaagaggaaaaccggaacctgcaggccgagtacgaccggctgaagcagcagcacgagcacaagggcctgagccccctgcctagcccccctgacaccatgtga

SEQ ID NO: 118 - protein, 1327 aa, Homo sapiens
MLWWEEVEDCYEREDVQKKTFTKWVNAQFSKFGKQHIENLFSDLQDGRRLLDLLEGLTGQKLPKEKGSTRVHALNNVNKALRVLQNNNVDLVNIGSTDIVDGNHKLTLGLIWNIILHWQVKNVMKNIMAGLQQTNSEKILLSWVRQSTRNYPQVNVINFTTSWSDGLALNALIHSHRPDLFDWNSVVCQQSATQRLEHAFNIARYQLGIEKLLDPEDVDTTYPDKKSILMYITSLFQVLPQQVSIEAIQEVEMLPRPPKVTKEEHFQLHHQMHYSQQITVSLAQGYERTSSPKPRFKSYAYTQAAYVTTSDPTRSPFPSQHLEAPEDKSFGSSLMESEVNLDRYQTALEEVLSWLLSAEDTLQAQGEISNDVEVVKDQFHTHEGYMMDLTAHQGRVGNILQLGSKLIGTGKLSEDEETEVQEQMNLLNSRWECLRVASMEKQSNLHRVLLKWQRLTEEQCLFSAWLSEKEDAVNKIHTTGFKDQNEMLSSLQKLAVLKADLEKKKQSMGKLYSLKQDLLSTLKNKSVTQKTEAWLDNFARCWDNLVQKLEKSTAQISQAVTTTQPSLTQTTVMETVTTVTTREQILVKHAQEELPPPPPQKKRQITVDSEAQIHTVREETMMVMTEDMPLEISYVPSTYLTEITHVSQALLEVEQLLNAPDLCAKDFEDLFKQEESLKNIKDSLQQSSGRIDIIHSKKTAALQSATPVERVKLQEALSQLDFQWEKVNKMYKDRQGRFDRSVEKWRRFHYDIKIFNQWLTEAEQFLRKTQIPENWEHAKYKWYLKELQDGIGQRQTVVRTLNATGEEIIQQSSKTDASILQEKLGSLNLRWQEVCKQLSDRKKRLEEQLERLQELQEATDELDLKLRQAEVIKGSWQPVGDLLIDSLQDHLEKVKALRGEIAPLKENVSHVNDLARQLTTLGIQLSPYNLSTLEDLNTRWKLLQVAVEDRVRQLHEAHRDFGPASQHFLSTSVQGPWERAISPNKVPYYINHETQTTCWDHPKMTELYQSLADLNNVRFSAYRTAMKLRRLQKALCLDLLSLSAACDALDQHNLKQNDQPMDILQIINCLTTIYDRLEQEHNNLVNVPLCVDMCLNWLLNVYDTGRTGRIRVLSFKTGIISLCKAHLEDKYRYLFKQVASSTGFCDQRRLGLLLHDSIQIPRQLGEVASFGGSNIEPSVRSCFQFANNKPEIEAALFLDWMRLEPQSMVWLPVLHRVAAAETAKHQAKCNICKECPIIGFRYRSLKHFNYDICQSCFFSGRVAKGHKMHYPMVEYCTPTTSGEDVRDFAKVLKNKFRTKRYFAKHPRMGYLPVQTVLEGDNMETDTM

SEQ ID NO: 119 - protein, 1321 aa, Homo sapiens
MLWWEEVEDCYEREDVQKKTFTKWVNAQFSKFGKQHIENLFSDLQDGRRLLDLLEGLTGQKLPKEKGSTRVHALNNVNKALRVLQNNNVDLVNIGSTDIVDGNHKLTLGLIWNIILHWQVKNVMKNIMAGLQQTNSEKILLSWVRQSTRNYPQVNVINFTTSWSDGLALNALIHSHRPDLFDWNSVVCQQSATQRLEHAFNIARYQLGIEKLLDPEDVDTTYPDKKSILMYITSLFQVLPQQVSIEAIQEVEMLPRPPKVTKEEHFQLHHQMHYSQQITVSLAQGYERTSSPKPRFKSYAYTQAAYVTTSDPTRSPFPSQHLEAPEDKSFGSSLMESEVNLDRYQTALEEVLSWLLSAEDTLQAQGEISNDVEVVKDQFHTHEGYMMDLTAHQGRVGNILQLGSKLIGTGKLSEDEETEVQEQMNLLNSRWECLRVASMEKQSNLHLLKWQRLTEEQCLFSAWLSEKEDAVNKIHTTGFKDQNEMLSSLQKLAVLKADLEKKKQSMGKLYSLKQDLLSTLKNKSVTQKTEAWLDNFARCWDNLVQKLEKSTAQISQAVTTTQPSLTQTTVMETVTTVTTREQILVKHAQEELPPPPPQKKRQITVDIHTVREETMMVMTEDMPLEISYVPSTYLTEITHVSQALLEVEQLLNAPDLCAKDFEDLFKQEESLKNIKDSLQQSSGRIDIIHSKKTAALQSATPVERVKLQEALSQLDFQWEKVNKMYKDRQGRFDRSVEKWRRFHYDIKIFNQWLTEAEQFLRKTQIPENWEHAKYKWYLKELQDGIGQRQTVVRTLNATGEEIIQQSSKTDASILQEKLGSLNLRWQEVCKQLSDRKKRLEEQLERLQELQEATDELDLKLRQAEVIKGSWQPVGDLLIDSLQDHLEKVKALRGEIAPLKENVSHVNDLARQLTTLGIQLSPYNLSTLEDLNTRWKLLQVAVEDRVRQLHEAHRDFGPASQHFLSTSVQGPWERAISPNKVPYYINHETQTTCWDHPKMTELYQSLADLNNVRFSAYRTAMKLRRLQKALCLDLLSLSAACDALDQHNLKQNDQPMDILQIINCLTTIYDRLEQEHNNLVNVPLCVDMCLNWLLNVYDTGRTGRIRVLSFKTGIISLCKAHLEDKYRYLFKQVASSTGFCDQRRLGLLLHDSIQIPRQLGEVASFGGSNIEPSVRSCFQFANNKPEIEAALFLDWMRLEPQSMVWLPVLHRVAAAETAKHQAKCNICKECPIIGFRYRSLKHFNYDICQSCFFSGRVAKGHKMHYPMVEYCTPTTSGEDVRDFAKVLKNKFRTKRYFAKHPRMGYLPVQTVLEGDNMETDTM

SEQ ID NO: 120 - protein, 1347 aa, Homo sapiens
MLWWEEVEDCYEREDVQKKTFTKWVNAQFSKFGKQHIENLFSDLQDGRRLLDLLEGLTGQKLPKEKGSTRVHALNNVNKALRVLQNNNVDLVNIGSTDIVDGNHKLTLGLIWNIILHWQVKNVMKNIMAGLQQTNSEKILLSWVRQSTRNYPQVNVINFTTSWSDGLALNALIHSHRPDLFDWNSVVCQQSATQRLEHAFNIARYQLGIEKLLDPEDVDTTYPDKKSILMYITSLFQVLPQQVSIEAIQEVEMLPRPPKVTKEEHFQLHHQMHYSQQITVSLAQGYERTSSPKPRFKSYAYTQAAYVTTSDPTRSPFPSQHLEAPEDKSFGSSLMESEVNLDRYQTALEEVLSWLLSAEDTLQAQGEISNDVEVVKDQFHTHEGYMMDLTAHQGRVGNILQLGSKLIGTGKLSEDEETEVQEQMNLLNSRWECLRVASMEKQSNLHLLKWQRLTEEQCLFSAWLSEKEDAVNKIHTTGFKDQNEMLSSLQKLAVLKADLEKKKQSMGKLYSLKQDLLSTLKNKSVTQKTEAWLDNFARCWDNLVQKLEKSTAQISQAVTTTQPSLTQTTVMETVTTVTTREQILVKHAQEELPPPPPQKKRQITVDSEAQIHTVREETMMVMTEDMPLEISYVPSTYLTEITHVSQALLEVEQLLNAPDLCAKDFEDLFKQEESLKNIKDSLQQSSGRIDIIHSKKTAALQSATPVERVKLQEALSQLDFQWEKVNKMYKDRQGRFDRSVEKWRRFHYDIKIFNQWLTEAEQFLRKTQIPENWEHAKYKWYLKELQDGIGQRQTVVRTLNATGEEIIQQSSKTDASILQEKLGSLNLRWQEVCKQLSDRKKRLEEQKNILQELQEATDELDLKLRQAEVIKGSWQPVGDLLIDSLQDHLEKVKALRGEIAPLKENVSHVNDLARQLTTLGIQLSPYNLSTLEDLNTRWKLLQVAVEDRVRQLHEAHRDFGPASQHFLSTSVQGPWERAISPNKVPYYINHETQTTCWDHPKMTELYQSLADLNNVRFSAYRTAMKLRRLQKALCLDLLSLSAACDALDQHNLKQNDQPMDILQIINCLTTIYDRLEQEHNNLVNVPLCVDMCLNWLLNVYDTGRTGRIRVLSFKTGIISLCKAHLEDKYRYLFKQVASSTGFCDQRRLGLLLHDSIQIPRQLGEVASFGGSNIEPSVRSCFQFANNKPEIEAALFLDWMRLEPQSMVWLPVLHRVAAAETAKHQAKCNICKECPIIGFRYRSLKHFNYDICQSCFFSGRVAKGHKMHYPMVEYCTPTTSGEDVRDFAKVLKNKFRTKRYFAKHPRMGYLPVQTVLEGDNMETTPCDDDLGRAMESLVSVMTDEEGAE

SEQ ID NO: 121 - protein, 1326 aa, Homo sapiens
MLWWEEVEDCYEREDVQKKTFTKWVNAQFSKFGKQHIENLFSDLQDGRRLLDLLEGLTGQKLPKEKGSTRVHALNNVNKALRVLQNNNVDLVNIGSTDIVDGNHKLTLGLIWNIILHWQVKNVMKNIMAGLQQTNSEKILLSWVRQSTRNYPQVNVINFTTSWSDGLALNALIHSHRPDLFDWNSVVCQQSATQRLEHAFNIARYQLGIEKLLDPEDVDTTYPDKKSILMYITSLFQVLPQQVSIEAIQEVEMLPRPPKVTKEEHFQLHHQMHYSQQITVSLAQGYERTSSPKPRFKSYAYTQAAYVTTSDPTRSPFPSQHLEAPEDKSFGSSLMESEVNLDRYQTALEEVLSWLLSAEDTLQAQGEISNDVEVVKDQFHTHEGYMMDLTAHQGRVGNILQLGSKLIGTGKLSEDEETEVQEQMNLLNSRWECLRVASMEKQSNLHLLKWQRLTEEQCLFSAWLSEKEDAVNKIHTTGFKDQNEMLSSLQKLAVLKADLEKKKQSMGKLYSLKQDLLSTLKNKSVTQKTEAWLDNFARCWDNLVQKLEKSTAQISQAVTTTQPSLTQTTVMETVTTVTTREQILVKHAQEELPPPPPQKKRQITVDSEAQIHTVREETMMVMTEDMPLEISYVPSTYLTEITHVSQALLEVEQLLNAPDLCAKDFEDLFKQEESLKNIKDSLQQSSGRIDIIHSKKTAALQSATPVERVKLQEALSQLDFQWEKVNKMYKDRQGRFDRSVEKWRRFHYDIKIFNQWLTEAEQFLRKTQIPENWEHAKYKWYLKELQDGIGQRQTVVRTLNATGEEIIQQSSKTDASILQEKLGSLNLRWQEVCKQLSDRKKRLEEQKLERLQELQEATDELDLKLRQAEVIKGSWQPVGDLLIDSLQDHLEKVKALRGEIAPLKENVSHVNDLARQLTTLGIQLSPYNLSTLEDLNTRWKLLQVAVEDRVRQLHEAHRDFGPASQHFLSTSVQGPWERAISPNKVPYYINHETQTTCWDHPKMTELYQSLADLNNVRFSAYRTAMKLRRLQKALCLDLLSLSAACDALDQHNLKQNDQPMDILQIINCLTTIYDRLEQEHNNLVNVPLCVDMCLNWLLNVYDTGRTGRIRVLSFKTGIISLCKAHLEDKYRYLFKQVASSTGFCDQRRLGLLLHDSIQIPRQLGEVASFGGSNIEPSVRSCFQFANNKPEIEAALFLDWMRLEPQSMVWLPVLHRVAAAETAKHQAKCNICKECPIIGFRYRSLKHFNYDICQSCFFSGRVAKGHKMHYPMVEYCTPTTSGEDVRDFAKVLKNKFRTKRYFAKHPRMGYLPVQTVLEGDNMETDTM

SEQ ID NO: 122 - protein, 1328 aa, Homo sapiens
MLWWEEVEDCYEREDVQKKTFTKWVNAQFSKFGKQHIENLFSDLQDGRRLLDLLEGLTGQKLPKEKGSTRVHALNNVNKALRVLQNNNVDLVNIGSTDIVDGNHKLTLGLIWNIILHWQVKNVMKNIMAGLQQTNSEKILLSWVRQSTRNYPQVNVINFTTSWSDGLALNALIHSHRPDLFDWNSVVCQQSATQRLEHAFNIARYQLGIEKLLDPEDVDTTYPDKKSILMYITSLFQVLPQQVSIEAIQEVEMLPRPPKVTKEEHFQLHHQMHYSQQITVSLAQGYERTSSPKPRFKSYAYTQAAYVTTSDPTRSPFPSQHLEAPEDKSFGSSLMESEVNLDRYQTALEEVLSWLLSAEDTLQAQGEISNDVEVVKDQFHTHEGYMMDLTAHQGRVGNILQLGSKLIGTGKLSEDEETEVQEQMNLLNSRWECLRVASMEKQSNLHLLKWQRLTEEQCLFSAWLSEKEDAVNKIHTTGFKDQNEMLSSLQKLAVLKADLEKKKQSMGKLYSLKQDLLSTLKNKSVTQKTEAWLDNFARCWDNLVQKLEKSTAQISQAVTTTQPSLTQTTVMETVTTVTTREQILVKHAQEELPPPPPQKKRQITVDSEAQIHTVREETMMVMTEDMPLEISYVPSTYLTEITHVSQALLEVEQLLNAPDLCAKDFEDLFKQEESLKNIKDSLQQSSGRIDIIHSKKTAALQSATPVERVKLQEALSQLDFQWEKVNKMYKDRQGRFDRSVEKWRRFHYDIKIFNQWLTEAEQFLRKTQIPENWEHAKYKWYLKELQDGIGQRQTVVRTLNATGEEIIQQSSKTDASILQEKLGSLNLRWQEVCKQLSDRKKRLEEQKNILERLQELQEATDELDLKLRQAEVIKGSWQPVGDLLIDSLQDHLEKVKALRGEIAPLKENVSHVNDLARQLTTLGIQLSPYNLSTLEDLNTRWKLLQVAVEDRVRQLHEAHRDFGPASQHFLSTSVQGPWERAISPNKVPYYINHETQTTCWDHPKMTELYQSLADLNNVRFSAYRTAMKLRRLQKALCLDLLSLSAACDALDQHNLKQNDQPMDILQIINCLTTIYDRLEQEHNNLVNVPLCVDMCLNWLLNVYDTGRTGRIRVLSFKTGIISLCKAHLEDKYRYLFKQVASSTGFCDQRRLGLLLHDSIQIPRQLGEVASFGGSNIEPSVRSCFQFANNKPEIEAALFLDWMRLEPQSMVWLPVLHRVAAAETAKHQAKCNICKECPIIGFRYRSLKHFNYDICQSCFFSGRVAKGHKMHYPMVEYCTPTTSGEDVRDFAKVLKNKFRTKRYFAKHPRMGYLPVQTVLEGDNMETDTM

SEQ ID NO: 123 - protein, 1327 aa, Homo sapiens; identical to SEQ ID NO: 118

SEQ ID NO: 124 - protein, 1332 aa, Homo sapiens
MLWWEEVEDCYEREDVQKKTFTKWVNAQFSKFGKQHIENLFSDLQDGRRLLDLLEGLTGQKLPKEKGSTRVHALNNVNKALRVLQNNNVDLVNIGSTDIVDGNHKLTLGLIWNIILHWQVKNVMKNIMAGLQQTNSEKILLSWVRQSTRNYPQVNVINFTTSWSDGLALNALIHSHRPDLFDWNSVVCQQSATQRLEHAFNIARYQLGIEKLLDPEDVDTTYPDKKSILMYITSLFQVLPQQVSIEAIQEVEMLPRPPKVTKEEHFQLHHQMHYSQQITVSLAQGYERTSSPKPRFKSYAYTQAAYVTTSDPTRSPFPSQHLEAPEDKSFGSSLMESEVNLDRYQTALEEVLSWLLSAEDTLQAQGEISNDVEVVKDQFHTHEGYMMDLTAHQGRVGNILQLGSKLIGTGKLSEDEETEVQEQMNLLNSRWECLRVASMEKQSNLHRVLLQDILLKWQRLTEEQCLFSAWLSEKEDAVNKIHTTGFKDQNEMLSSLQKLAVLKADLEKKKQSMGKLYSLKQDLLSTLKNKSVTQKTEAWLDNFARCWDNLVQKLEKSTAQISQAVTTTQPSLTQTTVMETVTTVTTREQILVKHAQEELPPPPPQKKRQITVDSEAQIHTVREETMMVMTEDMPLEISYVPSTYLTEITHVSQALLEVEQLLNAPDLCAKDFEDLFKQEESLKNIKDSLQQSSGRIDIIHSKKTAALQSATPVERVKLQEALSQLDFQWEKVNKMYKDRQGRFDRSVEKWRRFHYDIKIFNQWLTEAEQFLRKTQIPENWEHAKYKWYLKELQDGIGQRQTVVRTLNATGEEIIQQSSKTDASILQEKLGSLNLRWQEVCKQLSDRKKRLEEQLERLQELQEATDELDLKLRQAEVIKGSWQPVGDLLIDSLQDHLEKVKALRGEIAPLKENVSHVNDLARQLTTLGIQLSPYNLSTLEDLNTRWKLLQVAVEDRVRQLHEAHRDFGPASQHFLSTSVQGPWERAISPNKVPYYINHETQTTCWDHPKMTELYQSLADLNNVRFSAYRTAMKLRRLQKALCLDLLSLSAACDALDQHNLKQNDQPMDILQIINCLTTIYDRLEQEHNNLVNVPLCVDMCLNWLLNVYDTGRTGRIRVLSFKTGIISLCKAHLEDKYRYLFKQVASSTGFCDQRRLGLLLHDSIQIPRQLGEVASFGGSNIEPSVRSCFQFANNKPEIEAALFLDWMRLEPQSMVWLPVLHRVAAAETAKHQAKCNICKECPIIGFRYRSLKHFNYDICQSCFFSGRVAKGHKMHYPMVEYCTPTTSGEDVRDFAKVLKNKFRTKRYFAKHPRMGYLPVQTVLEGDNMETDTM

SEQ ID NO: 125 - protein, 1325 aa, Homo sapiens
MLWWEEVEDCYEREDVQKKTFTKWVNAQFSKFGKQHIENLFSDLQDGRRLLDLLEGLTGQKLPKEKGSTRVHALNNVNKALRVLQNNNVDLVNIGSTDIVDGNHKLTLGLIWNIILHWQVKNVMKNIMAGLQQTNSEKILLSWVRQSTRNYPQVNVINFTTSWSDGLALNALIHSHRPDLFDWNSVVCQQSATQRLEHAFNIARYQLGIEKLLDPEDVDTTYPDKKSILMYITSLFQVLPQQVSIEAIQEVEMLPRPPKVTKEEHFQLHHQMHYSQQITVSLAQGYERTSSPKPRFKSYAYTQAAYVTTSDPTRSPFPSQHLEAPEDKSFGSSLMESEVNLDRYQTALEEVLSWLLSAEDTLQAQGEISNDVEVVKDQFHTHEGYMMDLTAHQGRVGNILQLGSKLIGTGKLSEDEETEVQEQMNLLNSRWECLRVASMEKQSNLHLLKWQRLTEEQCLFSAWLSEKEDAVNKIHTTGFKDQNEMLSSLQKLAVLKADLEKKKQSMGKLYSLKQDLLSTLKNKSVTQKTEAWLDNFARCWDNLVQKLEKSTAQISQAVTTTQPSLTQTTVMETVTTVTTREQILVKHAQEELPPPPPQKKRQITVDSEAQIHTVREETMMVMTEDMPLEISYVPSTYLTEITHVSQALLEVEQLLNAPDLCAKDFEDLFKQEESLKNIKDSLQQSSGRIDIIHSKKTAALQSATPVERVKLQEALSQLDFQWEKVNKMYKDRQGRFDRSVEKWRRFHYDIKIFNQWLTEAEQFLRKTQIPENWEHAKYKWYLKELQDGIGQRQTVVRTLNATGEEIIQQSSKTDASILQEKLGSLNLRWQEVCKQLSDRKKRLEEQLERLQELQEATDELDLKLRQAEVIKGSWQPVGDLLIDSLQDHLEKVKALRGEIAPLKENVSHVNDLARQLTTLGIQLSPYNLSTLEDLNTRWKLLQVAVEDRVRQLHEAHRDFGPASQHFLSTSVQGPWERAISPNKVPYYINHETQTTCWDHPKMTELYQSLADLNNVRFSAYRTAMKLRRLQKALCLDLLSLSAACDALDQHNLKQNDQPMDILQIINCLTTIYDRLEQEHNNLVNVPLCVDMCLNWLLNVYDTGRTGRIRVLSFKTGIISLCKAHLEDKYRYLFKQVASSTGFCDQRRLGLLLHDSIQIPRQLGEVASFGGSNIEPSVRSCFQFANNKPEIEAALFLDWMRLEPQSMVWLPVLHRVAAAETAKHQAKCNICKECPIIGFRYRSLKHFNYDICQSCFFSGRVAKGHKMHYPMVEYCTPTTSGEDVRDFAKVLKNKFRTKRYFAKHPRMGYLPVQTVLEGDNMETDTM

SEQ ID NO: 126 - protein, 1255 aa, Homo sapiens
MLWWEEVEDCYEREDVQKKTFTKWVNAQFSKFGKQHIENLFSDLQDGRRLLDLLEGLTGQKLPKEKGSTRVHALNNVNKALRVLQNNNVDLVNIGSTDIVDGNHKLTLGLIWNIILHWQVKNVMKNIMAGLQQTNSEKILLSWVRQSTRNYPQVNVINFTTSWSDGLALNALIHSHRPDLFDWNSVVCQQSATQRLEHAFNIARYQLGIEKLLDPEDVDTTYPDKKSILMYITSLFQVLPQQVSIEAIQEVEMLPRPPKVTKEEHFQLHHQMHYSQQITVSLAQGYERTSSPKPRFKSYAYTQAAYVTTSDPTRSPFPSQHLEAPEDKSFGSSLMESEVNLDRYQTALEEVLSWLLSAEDTLQAQGEISNDVEVVKDQFHTHEGYMMDLTAHQGRVGNILQLGSKLIGTGKLSEDEETEVQEQMNLLNSRWECLRVASMEKQSNLHIHTVREETMMVMTEDMPLEISYVPSTYLTEITHVSQALLEVEQLLNAPDLCAKDFEDLFKQEESLKNIKDSLQQSSGRIDIIHSKKTAALQSATPVERVKLQEALSQLDFQWEKVNKMYKDRQGRFDRSVEKWRRFHYDIKIFNQWLTEAEQFLRKTQIPENWEHAKYKWYLKELQDGIGQRQTVVRTLNATGEEIIQQSSKTDASILQEKLGSLNLRWQEVCKQLSDRKKRLEEQAPGLTTIGASPTQTVTLVTQPVVTKETAISKLEMPSSLMLELERLQELQEATDELDLKLRQAEVIKGSWQPVGDLLIDSLQDHLEKVKALRGEIAPLKENVSHVNDLARQLTTLGIQLSPYNLSTLEDLNTRWKLLQVAVEDRVRQLHEAHRDFGPASQHFLSTSVQGPWERAISPNKVPYYINHETQTTCWDHPKMTELYQSLADLNNVRFSAYRTAMKLRRLQKALCLDLLSLSAACDALDQHNLKQNDQPMDILQIINCLTTIYDRLEQEHNNLVNVPLCVDMCLNWLLNVYDTGRTGRIRVLSFKTGIISLCKAHLEDKYRYLFKQVASSTGFCDQRRLGLLLHDSIQIPRQLGEVASFGGSNIEPSVRSCFQFANNKPEIEAALFLDWMRLEPQSMVWLPVLHRVAAAETAKHQAKCNICKECPIIGFRYRSLKHFNYDICQSCFFSGRVAKGHKMHYPMVEYCTPTTSGEDVRDFAKVLKNKFRTKRYFAKHPRMGYLPVQTVLEGDNMETPAQILISLESEERGELERILADLEEENRNLQAEYDRLKQQHEHKGLSPLPSPPDTM

SEQ ID NO: 127 - protein, 1262 aa, Homo sapiens
MLWWEEVEDCYEREDVQKKTFTKWVNAQFSKFGKQHIENLFSDLQDGRRLLDLLEGLTGQKLPKEKGSTRVHALNNVNKALRVLQNNNVDLVNIGSTDIVDGNHKLTLGLIWNIILHWQVKNVMKNIMAGLQQTNSEKILLSWVRQSTRNYPQVNVINFTTSWSDGLALNALIHSHRPDLFDWNSVVCQQSATQRLEHAFNIARYQLGIEKLLDPEDVDTTYPDKKSILMYITSLFQVLPQQVSIEAIQEVEMLPRPPKVTKEEHFQLHHQMHYSQQITVSLAQGYERTSSPKPRFKSYAYTQAAYVTTSDPTRSPFPSQHLEAPEDKSFGSSLMESEVNLDRYQTALEEVLSWLLSAEDTLQAQGEISNDVEVVKDQFHTHEGYMMDLTAHQGRVGNILQLGSKLIGTGKLSEDEETEVQEQMNLLNSRWECLRVASMEKQSNLHRVLIHTVREETMMVMTEDMPLEISYVPSTYLTEITHVSQALLEVEQLLNAPDLCAKDFEDLFKQEESLKNIKDSLQQSSGRIDIIHSKKTAALQSATPVERVKLQEALSQLDFQWEKVNKMYKDRQGRFDRSVEKWRRFHYDIKIFNQWLTEAEQFLRKTQIPENWEHAKYKWYLKELQDGIGQRQTVVRTLNATGEEIIQQSSKTDASILQEKLGSLNLRWQEVCKQLSDRKKRLEEQKNDLAPGLTTIGASPTQTVTLVTQPVVTKETAISKLEMPSSLMLEVERLQELQEATDELDLKLRQAEVIKGSWQPVGDLLIDSLQDHLEKVKALRGEIAPLKENVSHVNDLARQLTTLGIQLSPYNLSTLEDLNTRWKLLQVAVEDRVRQLHEAHRDFGPASQHFLSTSVQGPWERAISPNKVPYYINHETQTTCWDHPKMTELYQSLADLNNVRFSAYRTAMKLRRLQKALCLDLLSLSAACDALDQHNLKQNDQPMDILQIINCLTTIYDRLEQEHNNLVNVPLCVDMCLNWLLNVYDTGRTGRIRVLSFKTGIISLCKAHLEDKYRYLFKQVASSTGFCDQRRLGLLLHDSIQIPRQLGEVASFGGSNIEPSVRSCFQFANNKPEIEAALFLDWMRLEPQSMVWLPVLHRVAAAETAKHQAKCNICKECPIIGFRYRSLKHFNYDICQSCFFSGRVAKGHKMHYPMVEYCTPTTSGEDVRDFAKVLKNKFRTKRYFAKHPRMGYLPVQTVLEGDNMETPAQILISLESEERGELERILADLEEENRNLQAEYDRLKQQHEHKGLSPLPSPPDTM

SEQ ID NO: 128 - protein, 1249 aa, Homo sapiens
MLWWEEVEDCYEREDVQKKTFTKWVNAQFSKFGKQHIENLFSDLQDGRRLLDLLEGLTGQKLPKEKGSTRVHALNNVNKALRVLQNNNVDLVNIGSTDIVDGNHKLTLGLIWNIILHWQVKNVMKNIMAGLQQTNSEKILLSWVRQSTRNYPQVNVINFTTSWSDGLALNALIHSHRPDLFDWNSVVCQQSATQRLEHAFNIARYQLGIEKLLDPEDVDTTYPDKKSILMYITSLFQVLPQQVSIEAIQEVEMLPRPPKVTKEEHFQLHHQMHYSQQITVSLAQGYERTSSPKPRFKSYAYTQAAYVTTSDPTRSPFPSQHLEAPEDKSFGSSLMESEVNLDRYQTALEEVLSWLLSAEDTLQAQGEISNDVEVVKDQFHTHEGYMMDLTAHQGRVGNILQLGSKLIGTGKLSEDEETEVQEQMNLLNSRWECLRVASMEKQSNLHSYVPSTYLTEITHVSQALLEVEQLLNAPDLCAKDFEDLFKQEESLKNIKDSLQQSSGRIDIIHSKKTAALQSATPVERVKLQEALSQLDFQWEKVNKMYKDRQGRFDRSVEKWRRFHYDIKIFNQWLTEAEQFLRKTQIPENWEHAKYKWYLKELQDGIGQRQTVVRTLNATGEEIIQQSSKTDASILQEKLGSLNLRWQEVCKQLSDRKKRLEEQLEGLEKLYQEPRELPPEERAQNVTRLLRKQAEEVNTEWEKLNLHSADWQRKIDETLERLQELQEATDELDLKLRQAEVIKGSWQPVGDLLIDSLQDHLEKVKALRGEIAPLKENVSHVNDLARQLTTLGIQLSPYNLSTLEDLNTRWKLLQVAVEDRVRQLHEAHRDFGPASQHFLSTSVQGPWERAISPNKVPYYINHETQTTCWDHPKMTELYQSLADLNNVRFSAYRTAMKLRRLQKALCLDLLSLSAACDALDQHNLKQNDQPMDILQIINCLTTIYDRLEQEHNNLVNVPLCVDMCLNWLLNVYDTGRTGRIRVLSFKTGIISLCKAHLEDKYRYLFKQVASSTGFCDQRRLGLLLHDSIQIPRQLGEVASFGGSNIEPSVRSCFQFANNKPEIEAALFLDWMRLEPQSMVWLPVLHRVAAAETAKHQAKCNICKECPIIGFRYRSLKHFNYDICQSCFFSGRVAKGHKMHYPMVEYCTPTTSGEDVRDFAKVLKNKFRTKRYFAKHPRMGYLPVQTVLEGDNMETPAQILISLESEERGELERILADLEEENRNLQAEYDRLKQQHEHKGLSPLPSPPDTM

SEQ ID NO: 129 - protein, 1374 aa, Homo sapiens
MLWWEEVEDCYEREDVQKKTFTKWVNAQFSKFGKQHIENLFSDLQDGRRLLDLLEGLTGQKLPKEKGSTRVHALNNVNKALRVLQNNNVDLVNIGSTDIVDGNHKLTLGLIWNIILHWQVKNVMKNIMAGLQQTNSEKILLSWVRQSTRNYPQVNVINFTTSWSDGLALNALIHSHRPDLFDWNSVVCQQSATQRLEHAFNIARYQLGIEKLLDPEDVDTTYPDKKSILMYITSLFQVLPQQVSIEAIQEVEMLPRPPKVTKEEHFQLHHQMHYSQQITVSLAQGYERTSSPKPRFKSYAYTQAAYVTTSDPTRSPFPSQHLEAPEDKSFGSSLMESEVNLDRYQTALEEVLSWLLSAEDTLQAQGEISNDVEVVKDQFHTHEGYMMDLTAHQGRVGNILQLGSKLIGTGKLSEDEETEVQEQMNLLNSRWECLRVASMEKQSNLHLLKWQRLTEEQCLFSAWLSEKEDAVNKIHTTGFKDQNEMLSSLQKLAVLKADLEKKKQSMGKLYSLKQDLLSTLKNKSVTQKTEAWLDNFARCWDNLVQKLEKSTAQISQAVTTTQPSLTQTTVMETVTTVTTREQILVKHAQEELPPPPPQKKRQITVDIHTVREETMMVMTEDMPLEISYVPSTYLTEITHVSQALLEVEQLLNAPDLCAKDFEDLFKQEESLKNIKDSLQQSSGRIDIIHSKKTAALQSATPVERVKLQEALSQLDFQWEKVNKMYKDRQGRFDRSVEKWRRFHYDIKIFNQWLTEAEQFLRKTQIPENWEHAKYKWYLKELQDGIGQRQTVVRTLNATGEEIIQQSSKTDASILQEKLGSLNLRWQEVCKQLSDRKKRLEEQLERLQELQEATDELDLKLRQAEVIKGSWQPVGDLLIDSLQDHLEKVKALRGEIAPLKENVSHVNDLARQLTTLGIQLSPYNLSTLEDLNTRWKLLQVAVEDRVRQLHEAHRDFGPASQHFLSTSVQGPWERAISPNKVPYYINHETQTTCWDHPKMTELYQSLADLNNVRFSAYRTAMKLRRLQKALCLDLLSLSAACDALDQHNLKQNDQPMDILQIINCLTTIYDRLEQEHNNLVNVPLCVDMCLNWLLNVYDTGRTGRIRVLSFKTGIISLCKAHLEDKYRYLFKQVASSTGFCDQRRLGLLLHDSIQIPRQLGEVASFGGSNIEPSVRSCFQFANNKPEIEAALFLDWMRLEPQSMVWLPVLHRVAAAETAKHQAKCNICKECPIIGFRYRSLKHFNYDICQSCFFSGRVAKGHKMHYPMVEYCTPTTSGEDVRDFAKVLKNKFRTKRYFAKHPRMGYLPVQTVLEGDNMETPAQILISLESEERGELERILADLEEENRNLQAEYDRLKQQHEHKGLSPLPSPPDTM

SEQ ID NO: 130 - protein, 1365 aa, Homo sapiens
MLWWEEVEDCYEREDVQKKTFTKWVNAQFSKFGKQHIENLFSDLQDGRRLLDLLEGLTGQKLPKEKGSTRVHALNNVNKALRVLQNNNVDLVNIGSTDIVDGNHKLTLGLIWNIILHWQVKNVMKNIMAGLQQTNSEKILLSWVRQSTRNYPQVNVINFTTSWSDGLALNALIHSHRPDLFDWNSVVCQQSATQRLEHAFNIARYQLGIEKLLDPEDVDTTYPDKKSILMYITSLFQVLPQQVSIEAIQEVEMLPRPPKVTKEEHFQLHHQMHYSQQITVSLAQGYERTSSPKPRFKSYAYTQAAYVTTSDPTRSPFPSQHLEAPEDKSFGSSLMESEVNLDRYQTALEEVLSWLLSAEDTLQAQGEISNDVEVVKDQFHTHEGYMMDLTAHQGRVGNILQLGSKLIGTGKLSEDEETEVQEQMNLLNSRWECLRVASMEKQSNLHIHTVREETMMVMTEDMPLEISYVPSTYLTEITHVSQALLEVEQLLNAPDLCAKDFEDLFKQEESLKNIKDSLQQSSGRIDIIHSKKTAALQSATPVERVKLQEALSQLDFQWEKVNKMYKDRQGRFDRSVEKWRRFHYDIKIFNQWLTEAEQFLRKTQIPENWEHAKYKWYLKELQDGIGQRQTVVRTLNATGEEIIQQSSKTDASILQEKLGSLNLRWQEVCKQLSDRKKRLEEQAPGLTTIGASPTQTVTLVTQPVVTKETAISKLEMPSSLMLEVPALADFNRAWTELTDWLSLLDQVIKSQRVMVGDLEDINEMIIKQKATMQDLEQRRPQLEELITAAQNLKNKTSNQEARTIITDRIERIQNQWDEVQEHLQNRRQQLNEMLERLQELQEATDELDLKLRQAEVIKGSWQPVGDLLIDSLQDHLEKVKALRGEIAPLKENVSHVNDLARQLTTLGIQLSPYNLSTLEDLNTRWKLLQVAVEDRVRQLHEAHRDFGPASQHFLSTSVQGPWERAISPNKVPYYINHETQTTCWDHPKMTELYQSLADLNNVRFSAYRTAMKLRRLQKALCLDLLSLSAACDALDQHNLKQNDQPMDILQIINCLTTIYDRLEQEHNNLVNVPLCVDMCLNWLLNVYDTGRTGRIRVLSFKTGIISLCKAHLEDKYRYLFKQVASSTGFCDQRRLGLLLHDSIQIPRQLGEVASFGGSNIEPSVRSCFQFANNKPEIEAALFLDWMRLEPQSMVWLPVLHRVAAAETAKHQAKCNICKECPIIGFRYRSLKHFNYDICQSCFFSGRVAKGHKMHYPMVEYCTPTTSGEDVRDFAKVLKNKFRTKRYFAKHPRMGYLPVQTVLEGDNMETPAQILISLESEERGELERILADLEEENRNLQAEYDRLKQQHEHKGLSPLPSPPDTM

SEQ ID NO: 131 - protein, 1383 aa, Homo sapiens
MLWWEEVEDCYEREDVQKKTFTKWVNAQFSKFGKQHIENLFSDLQDGRRLLDLLEGLTGQKLPKEKGSTRVHALNNVNKALRVLQNNNVDLVNIGSTDIVDGNHKLTLGLIWNIILHWQVKNVMKNIMAGLQQTNSEKILLSWVRQSTRNYPQVNVINFTTSWSDGLALNALIHSHRPDLFDWNSVVCQQSATQRLEHAFNIARYQLGIEKLLDPEDVDTTYPDKKSILMYITSLFQVLPQQVSIEAIQEVEMLPRPPKVTKEEHFQLHHQMHYSQQITVSLAQGYERTSSPKPRFKSYAYTQAAYVTTSDPTRSPFPSQHLEAPEDKSFGSSLMESEVNLDRYQTALEEVLSWLLSAEDTLQAQGEISNDVEVVKDQFHTHEGYMMDLTAHQGRVGNILQLGSKLIGTGKLSEDEETEVQEQMNLLNSRWECLRVASMEKQSNLHRVLMDLQNQKLKELNDWLTKTEERTRKMEEEPLGPDLEDLKRQVQQHKVLQEDLEQEQVRVNSLTHMVVVVDESSGDHATAALEEQLKVLGDRWANICRWTEDRWVLLQDILLKWQRLTEEQCLFSAWLSEKEDAVNKIHTTGFKDQNEMLSSLQKLAVLKADLEKKKQSMGKLYSLKQDLLSTLKNKSVTQKTEAWLDNFARCWDNLVQKLEKSTAQISQAIHTVREETMMVMTEDMPLEISYVPSTYLTEITHVSQALLEVEQLLNAPDLCAKDFEDLFKQEESLKNIKDSLQQSSGRIDIIHSKKTAALQSATPVERVKLQEALSQLDFQWEKVNKMYKDRQGRFDRSVEKWRRFHYDIKIFNQWLTEAEQFLRKTQIPENWEHAKYKWYLKELQDGIGQRQTVVRTLNATGEEIIQQSSKTDASILQEKLGSLNLRWQEVCKQLSDRKKRLEEQLERLQELQEATDELDLKLRQAEVIKGSWQPVGDLLIDSLQDHLEKVKALRGEIAPLKENVSHVNDLARQLTTLGIQLSPYNLSTLEDLNTRWKLLQVAVEDRVRQLHEAHRDFGPASQHFLSTSVQGPWERAISPNKVPYYINHETQTTCWDHPKMTELYQSLADLNNVRFSAYRTAMKLRRLQKALCLDLLSLSAACDALDQHNLKQNDQPMDILQIINCLTTIYDRLEQEHNNLVNVPLCVDMCLNWLLNVYDTGRTGRIRVLSFKTGIISLCKAHLEDKYRYLFKQVASSTGFCDQRRLGLLLHDSIQIPRQLGEVASFGGSNIEPSVRSCFQFANNKPEIEAALFLDWMRLEPQSMVWLPVLHRVAAAETAKHQAKCNICKECPIIGFRYRSLKHFNYDICQSCFFSGRVAKGHKMHYPMVEYCTPTTSGEDVRDFAKVLKNKFRTKRYFAKHPRMGYLPVQTVLEGDNMETDTM

SEQ ID NO: 132 - protein, 1384 aa, Homo sapiens
MLWWEEVEDCYEREDVQKKTFTKWVNAQFSKFGKQHIENLFSDLQDGRRLLDLLEGLTGQKLPKEKGSTRVHALNNVNKALRVLQNNNVDLVNIGSTDIVDGNHKLTLGLIWNIILHWQVKNVMKNIMAGLQQTNSEKILLSWVRQSTRNYPQVNVINFTTSWSDGLALNALIHSHRPDLFDWNSVVCQQSATQRLEHAFNIARYQLGIEKLLDPEDVDTTYPDKKSILMYITSLFQVLPQQVSIEAIQEVEMLPRPPKVTKEEHFQLHHQMHYSQQITVSLAQGYERTSSPKPRFKSYAYTQAAYVTTSDPTRSPFPSQHLEAPEDKSFGSSLMESEVNLDRYQTALEEVLSWLLSAEDTLQAQGEISNDVEVVKDQFHTHEGYMMDLTAHQGRVGNILQLGSKLIGTGKLSEDEETEVQEQMNLLNSRWECLRVASMEKQSNLHIHTVREETMMVMTEDMPLEISYVPSTYLTEITHVSQALLEVEQLLNAPDLCAKDFEDLFKQEESLKNIKDSLQQSSGRIDIIHSKKTAALQSATPVERVKLQEALSQLDFQWEKVNKMYKDRQGRFDRSVEKWRRFHYDIKIFNQWLTEAEQFLRKTQIPENWEHAKYKWYLKELQDGIGQRQTVVRTLNATGEEIIQQSSKTDASILQEKLGSLNLRWQEVCKQLSDRKKRLEEQAPGLTTIGASPTQTVTLVTQPVVTKETAISKLEMPSSLMLESDQWKRLHLSLQELLVWLQLKDDELSRQAPIGGDFPAVQKQNDVHRAFKRELKTKEPVIMSTLETVRIFLTEQPLEGLEKLYQEPRELPPEERAQNVTRLLRKQAEEVNTEWEKLNLHSADWQRKIDETLERLQELQEATDELDLKLRQAEVIKGSWQPVGDLLIDSLQDHLEKVKALRGEIAPLKENVSHVNDLARQLTTLGIQLSPYNLSTLEDLNTRWKLLQVAVEDRVRQLHEAHRDFGPASQHFLSTSVQGPWERAISPNKVPYYINHETQTTCWDHPKMTELYQSLADLNNVRFSAYRTAMKLRRLQKALCLDLLSLSAACDALDQHNLKQNDQPMDILQIINCLTTIYDRLEQEHNNLVNVPLCVDMCLNWLLNVYDTGRTGRIRVLSFKTGIISLCKAHLEDKYRYLFKQVASSTGFCDQRRLGLLLHDSIQIPRQLGEVASFGGSNIEPSVRSCFQFANNKPEIEAALFLDWMRLEPQSMVWLPVLHRVAAAETAKHQAKCNICKECPIIGFRYRSLKHFNYDICQSCFFSGRVAKGHKMHYPMVEYCTPTTSGEDVRDFAKVLKNKFRTKRYFAKHPRMGYLPVQTVLEGDNMETPAQILISLESEERGELERILADLEEENRNLQAEYDRLKQQHEHKGLSPLPSPPDTM

SEQ ID NO: 133 - DNA, 4152 bp, Homo sapiens
atgctgtggtgggaggaagtggaagattgctacgagcgcgaggacgtgcagaagaaaaccttcaccaaatgggtgaacgcccagttcagcaagttcggcaagcagcacatcgagaacctgttcagcgacctgcaggacggcagacggctgctggacctgctggaaggcctgaccggccagaagctgcccaaagagaagggcagcaccagagtgcacgccctgaacaacgtgaacaaggccctgcgggtgctgcagaacaacaacgtggacctggtgaacatcggcagcaccgacatcgtggacggcaaccacaagctgaccctgggcctgatctggaacatcatcctgcactggcaggtcaaaaacgtgatgaagaacatcatggccggcctgcagcagaccaacagcgagaagatcctgctgagctgggtgcgccagagcacccggaactacccccaggtcaacgtgatcaacttcaccacctcttggagcgacggcctggccctgaacgccctgatccacagccaccggcccgacctgttcgactggaacagcgtggtctgccagcagagcgccacccagcggctggaacacgccttcaatatcgccagataccagctgggcatcgagaagctgctggatcccgaggacgtggacaccacctaccccgacaagaaatccatcctgatgtatatcaccagcctgttccaggtgctgccccagcaggtgtccatcgaggccatccaggaagtggaaatgctgcccagaccccccaaagtgaccaaagaggaacacttccagctgcaccaccagatgcactacagccagcagatcaccgtgtccctggcccagggctacgagagaaccagcagccccaagccccggttcaagagctacgcctatacccaggccgcctacgtgaccaccagcgaccctaccagaagcccattccccagccagcatctggaagcccccgaggacaagagcttcggcagcagcctgatggaaagcgaagtgaacctggacagataccagaccgccctggaagaggtgctgagctggctgctgagcgccgaggatacactgcaggctcagggcgagatcagcaacgacgtggaagtcgtgaaggaccagttccacacccacgagggctacatgatggacctgacagcccaccagggcagagtgggcaacatcctgcagctgggctccaagctgatcggcaccggcaagctgagcgaggacgaagagacagaggtgcaggaacagatgaacctgctgaacagcagatgggagtgcctgcgggtggccagcatggaaaagcagagcaacctgcatagggtcctgctgaagtggcagcggctgaccgaggaacagtgcctgtttagcgcctggctgtccgagaaagaggacgccgtgaacaagatccacaccaccggcttcaaggaccagaacgagatgctgagcagcctgcagaaactggccgtgctgaaggccgacctggaaaagaaaaagcagtccatgggcaagctgtactccctgaagcaggacctgctgtccaccctgaagaacaagagcgtgacccagaaaaccgaggcctggctggacaacttcgcccggtgctgggacaacctggtgcagaagctggaaaagtccaccgcccagatctcccaggccgtgaccacaacacagcccagcctgacccagaccaccgtgatggaaaccgtgacaacagtgaccacccgggaacagatcctcgtgaagcacgcccaggaagaactgccccctccacccccccagaagaaacggcagatcacagtggacagtgaagctcagatccacaccgtgcgggaagagacaatgatggtcatgacagaggacatgcccctggaaatcagctacgtgcccagcacctacctgaccgagatcacccatgtgtcccaggccctgctggaagtggaacagctgctgaacgcccccgacctgtgcgccaaggatttcgaggacctgttcaagcaggaagagagcctgaagaatatcaaggatagcctgcagcagagcagcggccggatcgacatcatccacagcaagaaaacagccgccctgcagagcgccacccccgtggaaagagtgaaactgcaggaagccctgtcccagctggacttccagtgggagaaagtgaacaaaatgtacaaggaccggcagggcagattcgaccgcagcgtggaaaagtggcggcggttccactacgacatcaagatcttcaaccagtggctgacagaggccgagcagttcctgagaaagacccagatccccgagaactgggagcacgccaagtacaagtggtatctgaaagagctgcaggacggcatcggccagagacagacagtcgtgcggaccctgaatgccaccggcgaggaaatcatccagcagtccagcaagaccgacgccagcattctgcaggaaaagctgggcagcctgaacctgcggtggcaggaagtgtgcaagcagctgtccgaccggaagaagcggctggaagaacagctggaacggctgcaggaactgcaggaggccaccgacgagctggacctgaaactgagacaggccgaagtgatcaagggcagctggcagccagtgggcgacctgctgatcgactccctgcaggaccatctggaaaaagtgaaggccctgagaggcgagatcgcccccctgaaagaaaacgtgtcccacgtgaacgacctggcccggcagctgacaacactgggcattcagctgagcccctacaacctgagcacactggaagatctgaacacccggtggaagctgctgcaggtggccgtggaagatagagtgcggcagctgcacgaggcccacagagattttggccctgcctcccagcacttcctgagcaccagtgtgcagggcccttgggagagagccatctcccctaacaaggtgccctactacatcaaccacgagacacagaccacctgttgggaccaccccaagatgaccgagctgtaccagagcctggctgacctgaacaacgtgcggttcagcgcctaccggaccgccatgaagctgcggagactgcagaaagctctgtgcctggatctgctgtccctgtccgccgcctgtgatgccctggaccagcacaatctgaagcagaacgaccagcccatggatatcctgcagatcatcaactgcctgaccaccatctacgaccggctggaacaggaacacaacaatctcgtgaacgtgcccctgtgcgtggacatgtgcctgaattggctgctgaatgtgtacgacaccggccggacaggccggatcagagtgctgtccttcaagaccggcatcatcagcctgtgcaaagcccacctggaagataagtaccggtatctgttcaaacaggtggcctctagcaccggcttttgcgaccagagaaggctgggcctgctgctgcacgacagcatccagatccctagacagctgggcgaagtggccagctttggcggcagcaacatcgagcctagcgtgcggagctgcttccagttcgccaacaacaagcccgagatcgaggccgccctgttcctggactggatgagactggaaccccagagcatggtgtggctgcccgtgctgcatagagtggccgctgccgagacagccaagcaccaggccaagtgcaacatctgcaaagagtgccccatcatcggcttccggtacagaagcctgaagcacttcaactacgatatctgccagagctgtttcttcagcggcagggtggccaagggccacaaaatgcactaccccatggtggaatactgcacccccaccacaagcggcgaggatgtgcgggatttcgccaaggtgctgaaaaacaagttccggaccaagcggtacttcgccaaacacccccggatgggctacctgcctgtgcagacagtgctggaaggcgacaacatggaaaccgacaccatgtgatgatgatttgggcagagcgatggagtccttagtatcagtcatgacagatgaagaaggagcagaataaatgttttacaactcctgattcccgcatgcggccagcttatcgataccgtcgaaataaaagatccttattttcattggatctgtgtgttggttttttgtgtg

SEQ ID NO: 134 - DNA, 4134 bp, Homo sapiens
atgctgtggtgggaggaagtggaagattgctacgagcgcgaggacgtgcagaagaaaaccttcaccaaatgggtgaacgcccagttcagcaagttcggcaagcagcacatcgagaacctgttcagcgacctgcaggacggcagacggctgctggacctgctggaaggcctgaccggccagaagctgcccaaagagaagggcagcaccagagtgcacgccctgaacaacgtgaacaaggccctgcgggtgctgcagaacaacaacgtggacctggtgaacatcggcagcaccgacatcgtggacggcaaccacaagctgaccctgggcctgatctggaacatcatcctgcactggcaggtcaaaaacgtgatgaagaacatcatggccggcctgcagcagaccaacagcgagaagatcctgctgagctgggtgcgccagagcacccggaactacccccaggtcaacgtgatcaacttcaccacctcttggagcgacggcctggccctgaacgccctgatccacagccaccggcccgacctgttcgactggaacagcgtggtctgccagcagagcgccacccagcggctggaacacgccttcaatatcgccagataccagctgggcatcgagaagctgctggatcccgaggacgtggacaccacctaccccgacaagaaatccatcctgatgtatatcaccagcctgttccaggtgctgccccagcaggtgtccatcgaggccatccaggaagtggaaatgctgcccagaccccccaaagtgaccaaagaggaacacttccagctgcaccaccagatgcactacagccagcagatcaccgtgtccctggcccagggctacgagagaaccagcagccccaagccccggttcaagagctacgcctatacccaggccgcctacgtgaccaccagcgaccctaccagaagcccattccccagccagcatctggaagcccccgaggacaagagcttcggcagcagcctgatggaaagcgaagtgaacctggacagataccagaccgccctggaagaggtgctgagctggctgctgagcgccgaggatacactgcaggctcagggcgagatcagcaacgacgtggaagtcgtgaaggaccagttccacacccacgagggctacatgatggacctgacagcccaccagggcagagtgggcaacatcctgcagctgggctccaagctgatcggcaccggcaagctgagcgaggacgaagagacagaggtgcaggaacagatgaacctgctgaacagcagatgggagtgcctgcgggtggccagcatggaaaagcagagcaacctgcatctgctgaagtggcagcggctgaccgaggaacagtgcctgtttagcgcctggctgtccgagaaagaggacgccgtgaacaagatccacaccaccggcttcaaggaccagaacgagatgctgagcagcctgcagaaactggccgtgctgaaggccgacctggaaaagaaaaagcagtccatgggcaagctgtactccctgaagcaggacctgctgtccaccctgaagaacaagagcgtgacccagaaaaccgaggcctggctggacaacttcgcccggtgctgggacaacctggtgcagaagctggaaaagtccaccgcccagatctcccaggccgtgaccacaacacagcccagcctgacccagaccaccgtgatggaaaccgtgacaacagtgaccacccgggaacagatcctcgtgaagcacgcccaggaagaactgccccctccacccccccagaagaaacggcagatcacagtggacatccacaccgtgcgggaagagacaatgatggtcatgacagaggacatgcccctggaaatcagctacgtgcccagcacctacctgaccgagatcacccatgtgtcccaggccctgctggaagtggaacagctgctgaacgcccccgacctgtgcgccaaggatttcgaggacctgttcaagcaggaagagagcctgaagaatatcaaggatagcctgcagcagagcagcggccggatcgacatcatccacagcaagaaaacagccgccctgcagagcgccacccccgtggaaagagtgaaactgcaggaagccctgtcccagctggacttccagtgggagaaagtgaacaaaatgtacaaggaccggcagggcagattcgaccgcagcgtggaaaagtggcggcggttccactacgacatcaagatcttcaaccagtggctgacagaggccgagcagttcctgagaaagacccagatccccgagaactgggagcacgccaagtacaagtggtatctgaaagagctgcaggacggcatcggccagagacagacagtcgtgcggaccctgaatgccaccggcgaggaaatcatccagcagtccagcaagaccgacgccagcattctgcaggaaaagctgggcagcctgaacctgcggtggcaggaagtgtgcaagcagctgtccgaccggaagaagcggctggaagaacagctggaacggctgcaggaactgcaggaggccaccgacgagctggacctgaaactgagacaggccgaagtgatcaagggcagctggcagccagtgggcgacctgctgatcgactccctgcaggaccatctggaaaaagtgaaggccctgagaggcgagatcgcccccctgaaagaaaacgtgtcccacgtgaacgacctggcccggcagctgacaacactgggcattcagctgagcccctacaacctgagcacactggaagatctgaacacccggtggaagctgctgcaggtggccgtggaagatagagtgcggcagctgcacgaggcccacagagattttggccctgcctcccagcacttcctgagcaccagtgtgcagggcccttgggagagagccatctcccctaacaaggtgccctactacatcaaccacgagacacagaccacctgttgggaccaccccaagatgaccgagctgtaccagagcctggctgacctgaacaacgtgcggttcagcgcctaccggaccgccatgaagctgcggagactgcagaaagctctgtgcctggatctgctgtccctgtccgccgcctgtgatgccctggaccagcacaatctgaagcagaacgaccagcccatggatatcctgcagatcatcaactgcctgaccaccatctacgaccggctggaacaggaacacaacaatctcgtgaacgtgcccctgtgcgtggacatgtgcctgaattggctgctgaatgtgtacgacaccggccggacaggccggatcagagtgctgtccttcaagaccggcatcatcagcctgtgcaaagcccacctggaagataagtaccggtatctgttcaaacaggtggcctctagcaccggcttttgcgaccagagaaggctgggcctgctgctgcacgacagcatccagatccctagacagctgggcgaagtggccagctttggcggcagcaacatcgagcctagcgtgcggagctgcttccagttcgccaacaacaagcccgagatcgaggccgccctgttcctggactggatgagactggaaccccagagcatggtgtggctgcccgtgctgcatagagtggccgctgccgagacagccaagcaccaggccaagtgcaacatctgcaaagagtgccccatcatcggcttccggtacagaagcctgaagcacttcaactacgatatctgccagagctgtttcttcagcggcagggtggccaagggccacaaaatgcactaccccatggtggaatactgcacccccaccacaagcggcgaggatgtgcgggatttcgccaaggtgctgaaaaacaagttccggaccaagcggtacttcgccaaacacccccggatgggctacctgcctgtgcagacagtgctggaaggcgacaacatggaaaccgacaccatgtgatgatgatttgggcagagcgatggagtccttagtatcagtcatgacagatgaagaaggagcagaataaatgttttacaactcctgattcccgcatgcggccagcttatcgataccgtcgaaataaaagatccttattttcattggatctgtgtgttggttttttgtgtg

SEQ ID NO: 135 - DNA, 4145 bp, Homo sapiens
atgctgtggtgggaggaagtggaagattgctacgagcgcgaggacgtgcagaagaaaaccttcaccaaatgggtgaacgcccagttcagcaagttcggcaagcagcacatcgagaacctgttcagcgacctgcaggacggcagacggctgctggacctgctggaaggcctgaccggccagaagctgcccaaagagaagggcagcaccagagtgcacgccctgaacaacgtgaacaaggccctgcgggtgctgcagaacaacaacgtggacctggtgaacatcggcagcaccgacatcgtggacggcaaccacaagctgaccctgggcctgatctggaacatcatcctgcactggcaggtcaaaaacgtgatgaagaacatcatggccggcctgcagcagaccaacagcgagaagatcctgctgagctgggtgcgccagagcacccggaactacccccaggtcaacgtgatcaacttcaccacctcttggagcgacggcctggccctgaacgccctgatccacagccaccggcccgacctgttcgactggaacagcgtggtctgccagcagagcgccacccagcggctggaacacgccttcaatatcgccagataccagctgggcatcgagaagctgctggatcccgaggacgtggacaccacctaccccgacaagaaatccatcctgatgtatatcaccagcctgttccaggtgctgccccagcaggtgtccatcgaggccatccaggaagtggaaatgctgcccagaccccccaaagtgaccaaagaggaacacttccagctgcaccaccagatgcactacagccagcagatcaccgtgtccctggcccagggctacgagagaaccagcagccccaagccccggttcaagagctacgcctatacccaggccgcctacgtgaccaccagcgaccctaccagaagcccattccccagccagcatctggaagcccccgaggacaagagcttcggcagcagcctgatggaaagcgaagtgaacctggacagataccagaccgccctggaagaggtgctgagctggctgctgagcgccgaggatacactgcaggctcagggcgagatcagcaacgacgtggaagtcgtgaaggaccagttccacacccacgagggctacatgatggacctgacagcccaccagggcagagtgggcaacatcctgcagctgggctccaagctgatcggcaccggcaagctgagcgaggacgaagagacagaggtgcaggaacagatgaacctgctgaacagcagatgggagtgcctgcgggtggccagcatggaaaagcagagcaacctgcatctgctgaagtggcagcggctgaccgaggaacagtgcctgtttagcgcctggctgtccgagaaagaggacgccgtgaacaagatccacaccaccggcttcaaggaccagaacgagatgctgagcagcctgcagaaactggccgtgctgaaggccgacctggaaaagaaaaagcagtccatgggcaagctgtactccctgaagcaggacctgctgtccaccctgaagaacaagagcgtgacccagaaaaccgaggcctggctggacaacttcgcccggtgctgggacaacctggtgcagaagctggaaaagtccaccgcccagatctcccaggccgtgaccacaacacagcccagcctgacccagaccaccgtgatggaaaccgtgacaacagtgaccacccgggaacagatcctcgtgaagcacgcccaggaagaactgccccctccacccccccagaagaaacggcagatcacagtggacagtgaagctcagatccacaccgtgcgggaagagacaatgatggtcatgacagaggacatgcccctggaaatcagctacgtgcccagcacctacctgaccgagatcacccatgtgtcccaggccctgctggaagtggaacagctgctgaacgcccccgacctgtgcgccaaggatttcgaggacctgttcaagcaggaagagagcctgaagaatatcaaggatagcctgcagcagagcagcggccggatcgacatcatccacagcaagaaaacagccgccctgcagagcgccacccccgtggaaagagtgaaactgcaggaagccctgtcccagctggacttccagtgggagaaagtgaacaaaatgtacaaggaccggcagggcagattcgaccgcagcgtggaaaagtggcggcggttccactacgacatcaagatcttcaaccagtggctgacagaggccgagcagttcctgagaaagacccagatccccgagaactgggagcacgccaagtacaagtggtatctgaaagagctgcaggacggcatcggccagagacagacagtcgtgcggaccctgaatgccaccggcgaggaaatcatccagcagtccagcaagaccgacgccagcattctgcaggaaaagctgggcagcctgaacctgcggtggcaggaagtgtgcaagcagctgtccgaccggaagaagcggctggaagaacagaagaacatcctgcaggaactgcaggaggccaccgacgagctggacctgaaactgagacaggccgaagtgatcaagggcagctggcagccagtgggcgacctgctgatcgactccctgcaggaccatctggaaaaagtgaaggccctgagaggcgagatcgcccccctgaaagaaaacgtgtcccacgtgaacgacctggcccggcagctgacaacactgggcattcagctgagcccctacaacctgagcacactggaagatctgaacacccggtggaagctgctgcaggtggccgtggaagatagagtgcggcagctgcacgaggcccacagagattttggccctgcctcccagcacttcctgagcaccagtgtgcagggcccttgggagagagccatctcccctaacaaggtgccctactacatcaaccacgagacacagaccacctgttgggaccaccccaagatgaccgagctgtaccagagcctggctgacctgaacaacgtgcggttcagcgcctaccggaccgccatgaagctgcggagactgcagaaagctctgtgcctggatctgctgtccctgtccgccgcctgtgatgccctggaccagcacaatctgaagcagaacgaccagcccatggatatcctgcagatcatcaactgcctgaccaccatctacgaccggctggaacaggaacacaacaatctcgtgaacgtgcccctgtgcgtggacatgtgcctgaattggctgctgaatgtgtacgacaccggccggacaggccggatcagagtgctgtccttcaagaccggcatcatcagcctgtgcaaagcccacctggaagataagtaccggtatctgttcaaacaggtggcctctagcaccggcttttgcgaccagagaaggctgggcctgctgctgcacgacagcatccagatccctagacagctgggcgaagtggccagctttggcggcagcaacatcgagcctagcgtgcggagctgcttccagttcgccaacaacaagcccgagatcgaggccgccctgttcctggactggatgagactggaaccccagagcatggtgtggctgcccgtgctgcatagagtggccgctgccgagacagccaagcaccaggccaagtgcaacatctgcaaagagtgccccatcatcggcttccggtacagaagcctgaagcacttcaactacgatatctgccagagctgtttcttcagcggcagggtggccaagggccacaaaatgcactaccccatggtggaatactgcacccccaccacaagcggcgaggatgtgcgggatttcgccaaggtgctgaaaaacaagttccggaccaagcggtacttcgccaaacacccccggatgggctacctgcctgtgcagacagtgctggaaggcgacaacatggaaaccacaccatgtgatgatgatttgggcagagcgatggagtccttagtatcagtcatgacagatgaagaaggagcagaataaatgttttacaactcctgattcccgcatgcggccagcttatcgataccgtcgaaataaaagatccttattttcattggatctgtgtgttggttttttgtgtg

SEQ ID NO: 136 - DNA, 4149 bp, Homo sapiens
atgctgtggtgggaggaagtggaagattgctacgagcgcgaggacgtgcagaagaaaaccttcaccaaatgggtgaacgcccagttcagcaagttcggcaagcagcacatcgagaacctgttcagcgacctgcaggacggcagacggctgctggacctgctggaaggcctgaccggccagaagctgcccaaagagaagggcagcaccagagtgcacgccctgaacaacgtgaacaaggccctgcgggtgctgcagaacaacaacgtggacctggtgaacatcggcagcaccgacatcgtggacggcaaccacaagctgaccctgggcctgatctggaacatcatcctgcactggcaggtcaaaaacgtgatgaagaacatcatggccggcctgcagcagaccaacagcgagaagatcctgctgagctgggtgcgccagagcacccggaactacccccaggtcaacgtgatcaacttcaccacctcttggagcgacggcctggccctgaacgccctgatccacagccaccggcccgacctgttcgactggaacagcgtggtctgccagcagagcgccacccagcggctggaacacgccttcaatatcgccagataccagctgggcatcgagaagctgctggatcccgaggacgtggacaccacctaccccgacaagaaatccatcctgatgtatatcaccagcctgttccaggtgctgccccagcaggtgtccatcgaggccatccaggaagtggaaatgctgcccagaccccccaaagtgaccaaagaggaacacttccagctgcaccaccagatgcactacagccagcagatcaccgtgtccctggcccagggctacgagagaaccagcagccccaagccccggttcaagagctacgcctatacccaggccgcctacgtgaccaccagcgaccctaccagaagcccattccccagccagcatctggaagcccccgaggacaagagcttcggcagcagcctgatggaaagcgaagtgaacctggacagataccagaccgccctggaagaggtgctgagctggctgctgagcgccgaggatacactgcaggctcagggcgagatcagcaacgacgtggaagtcgtgaaggaccagttccacacccacgagggctacatgatggacctgacagcccaccagggcagagtgggcaacatcctgcagctgggctccaagctgatcggcaccggcaagctgagcgaggacgaagagacagaggtgcaggaacagatgaacctgctgaacagcagatgggagtgcctgcgggtggccagcatggaaaagcagagcaacctgcatctgctgaagtggcagcggctgaccgaggaacagtgcctgtttagcgcctggctgtccgagaaagaggacgccgtgaacaagatccacaccaccggcttcaaggaccagaacgagatgctgagcagcctgcagaaactggccgtgctgaaggccgacctggaaaagaaaaagcagtccatgggcaagctgtactccctgaagcaggacctgctgtccaccctgaagaacaagagcgtgacccagaaaaccgaggcctggctggacaacttcgcccggtgctgggacaacctggtgcagaagctggaaaagtccaccgcccagatctcccaggccgtgaccacaacacagcccagcctgacccagaccaccgtgatggaaaccgtgacaacagtgaccacccgggaacagatcctcgtgaagcacgcccaggaagaactgccccctccacccccccagaagaaacggcagatcacagtggacagtgaagctcagatccacaccgtgcgggaagagacaatgatggtcatgacagaggacatgcccctggaaatcagctacgtgcccagcacctacctgaccgagatcacccatgtgtcccaggccctgctggaagtggaacagctgctgaacgcccccgacctgtgcgccaaggatttcgaggacctgttcaagcaggaagagagcctgaagaatatcaaggatagcctgcagcagagcagcggccggatcgacatcatccacagcaagaaaacagccgccctgcagagcgccacccccgtggaaagagtgaaactgcaggaagccctgtcccagctggacttccagtgggagaaagtgaacaaaatgtacaaggaccggcagggcagattcgaccgcagcgtggaaaagtggcggcggttccactacgacatcaagatcttcaaccagtggctgacagaggccgagcagttcctgagaaagacccagatccccgagaactgggagcacgccaagtacaagtggtatctgaaagagctgcaggacggcatcggccagagacagacagtcgtgcggaccctgaatgccaccggcgaggaaatcatccagcagtccagcaagaccgacgccagcattctgcaggaaaagctgggcagcctgaacctgcggtggcaggaagtgtgcaagcagctgtccgaccggaagaagcggctggaagaacagaagctggaacggctgcaggaactgcaggaggccaccgacgagctggacctgaaactgagacaggccgaagtgatcaagggcagctggcagccagtgggcgacctgctgatcgactccctgcaggaccatctggaaaaagtgaaggccctgagaggcgagatcgcccccctgaaagaaaacgtgtcccacgtgaacgacctggcccggcagctgacaacactgggcattcagctgagcccctacaacctgagcacactggaagatctgaacacccggtggaagctgctgcaggtggccgtggaagatagagtgcggcagctgcacgaggcccacagagattttggccctgcctcccagcacttcctgagcaccagtgtgcagggcccttgggagagagccatctcccctaacaaggtgccctactacatcaaccacgagacacagaccacctgttgggaccaccccaagatgaccgagctgtaccagagcctggctgacctgaacaacgtgcggttcagcgcctaccggaccgccatgaagctgcggagactgcagaaagctctgtgcctggatctgctgtccctgtccgccgcctgtgatgccctggaccagcacaatctgaagcagaacgaccagcccatggatatcctgcagatcatcaactgcctgaccaccatctacgaccggctggaacaggaacacaacaatctcgtgaacgtgcccctgtgcgtggacatgtgcctgaattggctgctgaatgtgtacgacaccggccggacaggccggatcagagtgctgtccttcaagaccggcatcatcagcctgtgcaaagcccacctggaagataagtaccggtatctgttcaaacaggtggcctctagcaccggcttttgcgaccagagaaggctgggcctgctgctgcacgacagcatccagatccctagacagctgggcgaagtggccagctttggcggcagcaacatcgagcctagcgtgcggagctgcttccagttcgccaacaacaagcccgagatcgaggccgccctgttcctggactggatgagactggaaccccagagcatggtgtggctgcccgtgctgcatagagtggccgctgccgagacagccaagcaccaggccaagtgcaacatctgcaaagagtgccccatcatcggcttccggtacagaagcctgaagcacttcaactacgatatctgccagagctgtttcttcagcggcagggtggccaagggccacaaaatgcactaccccatggtggaatactgcacccccaccacaagcggcgaggatgtgcgggatttcgccaaggtgctgaaaaacaagttccggaccaagcggtacttcgccaaacacccccggatgggctacctgcctgtgcagacagtgctggaaggcgacaacatggaaaccgacaccatgtgatgatgatttgggcagagcgatggagtccttagtatcagtcatgacagatgaagaaggagcagaataaatgttttacaactcctgattcccgcatgcggccagcttatcgataccgtcgaaataaaagatccttattttcattggatctgtgtgttggttttttgtgtg

SEQ ID NO: 137 - DNA, 4155 bp, Homo sapiens
atgctgtggtgggaggaagtggaagattgctacgagcgcgaggacgtgcagaagaaaaccttcaccaaatgggtgaacgcccagttcagcaagttcggcaagcagcacatcgagaacctgttcagcgacctgcaggacggcagacggctgctggacctgctggaaggcctgaccggccagaagctgcccaaagagaagggcagcaccagagtgcacgccctgaacaacgtgaacaaggccctgcgggtgctgcagaacaacaacgtggacctggtgaacatcggcagcaccgacatcgtggacggcaaccacaagctgaccctgggcctgatctggaacatcatcctgcactggcaggtcaaaaacgtgatgaagaacatcatggccggcctgcagcagaccaacagcgagaagatcctgctgagctgggtgcgccagagcacccggaactacccccaggtcaacgtgatcaacttcaccacctcttggagcgacggcctggccctgaacgccctgatccacagccaccggcccgacctgttcgactggaacagcgtggtctgccagcagagcgccacccagcggctggaacacgccttcaatatcgccagataccagctgggcatcgagaagctgctggatcccgaggacgtggacaccacctaccccgacaagaaatccatcctgatgtatatcaccagcctgttccaggtgctgccccagcaggtgtccatcgaggccatccaggaagtggaaatgctgcccagaccccccaaagtgaccaaagaggaacacttccagctgcaccaccagatgcactacagccagcagatcaccgtgtccctggcccagggctacgagagaaccagcagccccaagccccggttcaagagctacgcctatacccaggccgcctacgtgaccaccagcgaccctaccagaagcccattccccagccagcatctggaagcccccgaggacaagagcttcggcagcagcctgatggaaagcgaagtgaacctggacagataccagaccgccctggaagaggtgctgagctggctgctgagcgccgaggatacactgcaggctcagggcgagatcagcaacgacgtggaagtcgtgaaggaccagttccacacccacgagggctacatgatggacctgacagcccaccagggcagagtgggcaacatcctgcagctgggctccaagctgatcggcaccggcaagctgagcgaggacgaagagacagaggtgcaggaacagatgaacctgctgaacagcagatgggagtgcctgcgggtggccagcatggaaaagcagagcaacctgcatctgctgaagtggcagcggctgaccgaggaacagtgcctgtttagcgcctggctgtccgagaaagaggacgccgtgaacaagatccacaccaccggcttcaaggaccagaacgagatgctgagcagcctgcagaaactggccgtgctgaaggccgacctggaaaagaaaaagcagtccatgggcaagctgtactccctgaagcaggacctgctgtccaccctgaagaacaagagcgtgacccagaaaaccgaggcctggctggacaacttcgcccggtgctgggacaacctggtgcagaagctggaaaagtccaccgcccagatctcccaggccgtgaccacaacacagcccagcctgacccagaccaccgtgatggaaaccgtgacaacagtgaccacccgggaacagatcctcgtgaagcacgcccaggaagaactgccccctccacccccccagaagaaacggcagatcacagtggacagtgaagctcagatccacaccgtgcgggaagagacaatgatggtcatgacagaggacatgcccctggaaatcagctacgtgcccagcacctacctgaccgagatcacccatgtgtcccaggccctgctggaagtggaacagctgctgaacgcccccgacctgtgcgccaaggatttcgaggacctgttcaagcaggaagagagcctgaagaatatcaaggatagcctgcagcagagcagcggccggatcgacatcatccacagcaagaaaacagccgccctgcagagcgccacccccgtggaaagagtgaaactgcaggaagccctgtcccagctggacttccagtgggagaaagtgaacaaaatgtacaaggaccggcagggcagattcgaccgcagcgtggaaaagtggcggcggttccactacgacatcaagatcttcaaccagtggctgacagaggccgagcagttcctgagaaagacccagatccccgagaactgggagcacgccaagtacaagtggtatctgaaagagctgcaggacggcatcggccagagacagacagtcgtgcggaccctgaatgccaccggcgaggaaatcatccagcagtccagcaagaccgacgccagcattctgcaggaaaagctgggcagcctgaacctgcggtggcaggaagtgtgcaagcagctgtccgaccggaagaagcggctggaagaacagaagaacatcctggaacggctgcaggaactgcaggaggccaccgacgagctggacctgaaactgagacaggccgaagtgatcaagggcagctggcagccagtgggcgacctgctgatcgactccctgcaggaccatctggaaaaagtgaaggccctgagaggcgagatcgcccccctgaaagaaaacgtgtcccacgtgaacgacctggcccggcagctgacaacactgggcattcagctgagcccctacaacctgagcacactggaagatctgaacacccggtggaagctgctgcaggtggccgtggaagatagagtgcggcagctgcacgaggcccacagagattttggccctgcctcccagcacttcctgagcaccagtgtgcagggcccttgggagagagccatctcccctaacaaggtgccctactacatcaaccacgagacacagaccacctgttgggaccaccccaagatgaccgagctgtaccagagcctggctgacctgaacaacgtgcggttcagcgcctaccggaccgccatgaagctgcggagactgcagaaagctctgtgcctggatctgctgtccctgtccgccgcctgtgatgccctggaccagcacaatctgaagcagaacgaccagcccatggatatcctgcagatcatcaactgcctgaccaccatctacgaccggctggaacaggaacacaacaatctcgtgaacgtgcccctgtgcgtggacatgtgcctgaattggctgctgaatgtgtacgacaccggccggacaggccggatcagagtgctgtccttcaagaccggcatcatcagcctgtgcaaagcccacctggaagataagtaccggtatctgttcaaacaggtggcctctagcaccggcttttgcgaccagagaaggctgggcctgctgctgcacgacagcatccagatccctagacagctgggcgaagtggccagctttggcggcagcaacatcgagcctagcgtgcggagctgcttccagttcgccaacaacaagcccgagatcgaggccgccctgttcctggactggatgagactggaaccccagagcatggtgtggctgcccgtgctgcatagagtggccgctgccgagacagccaagcaccaggccaagtgcaacatctgcaaagagtgccccatcatcggcttccggtacagaagcctgaagcacttcaactacgatatctgccagagctgtttcttcagcggcagggtggccaagggccacaaaatgcactaccccatggtggaatactgcacccccaccacaagcggcgaggatgtgcgggatttcgccaaggtgctgaaaaacaagttccggaccaagcggtacttcgccaaacacccccggatgggctacctgcctgtgcagacagtgctggaaggcgacaacatggaaaccgacaccatgtgatgatgatttgggcagagcgatggagtccttagtatcagtcatgacagatgaagaaggagcagaataaatgttttacaactcctgattcccgcatgcggccagcttatcgataccgtcgaaataaaagatccttattttcattggatctgtgtgttggttttttgtgtg

SEQ ID NO: 138 - DNA, 4152 bp, Homo sapiens; identical to SEQ ID NO: 133

SEQ ID NO: 139 - DNA, 4167 bp, Homo sapiens
atgctgtggtgggaggaagtggaagattgctacgagcgcgaggacgtgcagaagaaaaccttcaccaaatgggtgaacgcccagttcagcaagttcggcaagcagcacatcgagaacctgttcagcgacctgcaggacggcagacggctgctggacctgctggaaggcctgaccggccagaagctgcccaaagagaagggcagcaccagagtgcacgccctgaacaacgtgaacaaggccctgcgggtgctgcagaacaacaacgtggacctggtgaacatcggcagcaccgacatcgtggacggcaaccacaagctgaccctgggcctgatctggaacatcatcctgcactggcaggtcaaaaacgtgatgaagaacatcatggccggcctgcagcagaccaacagcgagaagatcctgctgagctgggtgcgccagagcacccggaactacccccaggtcaacgtgatcaacttcaccacctcttggagcgacggcctggccctgaacgccctgatccacagccaccggcccgacctgttcgactggaacagcgtggtctgccagcagagcgccacccagcggctggaacacgccttcaatatcgccagataccagctgggcatcgagaagctgctggatcccgaggacgtggacaccacctaccccgacaagaaatccatcctgatgtatatcaccagcctgttccaggtgctgccccagcaggtgtccatcgaggccatccaggaagtggaaatgctgcccagaccccccaaagtgaccaaagaggaacacttccagctgcaccaccagatgcactacagccagcagatcaccgtgtccctggcccagggctacgagagaaccagcagccccaagccccggttcaagagctacgcctatacccaggccgcctacgtgaccaccagcgaccctaccagaagcccattccccagccagcatctggaagcccccgaggacaagagcttcggcagcagcctgatggaaagcgaagtgaacctggacagataccagaccgccctggaagaggtgctgagctggctgctgagcgccgaggatacactgcaggctcagggcgagatcagcaacgacgtggaagtcgtgaaggaccagttccacacccacgagggctacatgatggacctgacagcccaccagggcagagtgggcaacatcctgcagctgggctccaagctgatcggcaccggcaagctgagcgaggacgaagagacagaggtgcaggaacagatgaacctgctgaacagcagatgggagtgcctgcgggtggccagcatggaaaagcagagcaacctgcatagagtactgctccaagacatcctgctgaagtggcagcggctgaccgaggaacagtgcctgtttagcgcctggctgtccgagaaagaggacgccgtgaacaagatccacaccaccggcttcaaggaccagaacgagatgctgagcagcctgcagaaactggccgtgctgaaggccgacctggaaaagaaaaagcagtccatgggcaagctgtactccctgaagcaggacctgctgtccaccctgaagaacaagagcgtgacccagaaaaccgaggcctggctggacaacttcgcccggtgctgggacaacctggtgcagaagctggaaaagtccaccgcccagatctcccaggccgtgaccacaacacagcccagcctgacccagaccaccgtgatggaaaccgtgacaacagtgaccacccgggaacagatcctcgtgaagcacgcccaggaagaactgccccctccacccccccagaagaaacggcagatcacagtggacagtgaagctcagatccacaccgtgcgggaagagacaatgatggtcatgacagaggacatgcccctggaaatcagctacgtgcccagcacctacctgaccgagatcacccatgtgtcccaggccctgctggaagtggaacagctgctgaacgcccccgacctgtgcgccaaggatttcgaggacctgttcaagcaggaagagagcctgaagaatatcaaggatagcctgcagcagagcagcggccggatcgacatcatccacagcaagaaaacagccgccctgcagagcgccacccccgtggaaagagtgaaactgcaggaagccctgtcccagctggacttccagtgggagaaagtgaacaaaatgtacaaggaccggcagggcagattcgaccgcagcgtggaaaagtggcggcggttccactacgacatcaagatcttcaaccagtggctgacagaggccgagcagttcctgagaaagacccagatccccgagaactgggagcacgccaagtacaagtggtatctgaaagagctgcaggacggcatcggccagagacagacagtcgtgcggaccctgaatgccaccggcgaggaaatcatccagcagtccagcaagaccgacgccagcattctgcaggaaaagctgggcagcctgaacctgcggtggcaggaagtgtgcaagcagctgtccgaccggaagaagcggctggaagaacagctggaacggctgcaggaactgcaggaggccaccgacgagctggacctgaaactgagacaggccgaagtgatcaagggcagctggcagccagtgggcgacctgctgatcgactccctgcaggaccatctggaaaaagtgaaggccctgagaggcgagatcgcccccctgaaagaaaacgtgtcccacgtgaacgacctggcccggcagctgacaacactgggcattcagctgagcccctacaacctgagcacactggaagatctgaacacccggtggaagctgctgcaggtggccgtggaagatagagtgcggcagctgcacgaggcccacagagattttggccctgcctcccagcacttcctgagcaccagtgtgcagggcccttgggagagagccatctcccctaacaaggtgccctactacatcaaccacgagacacagaccacctgttgggaccaccccaagatgaccgagctgtaccagagcctggctgacctgaacaacgtgcggttcagcgcctaccggaccgccatgaagctgcggagactgcagaaagctctgtgcctggatctgctgtccctgtccgccgcctgtgatgccctggaccagcacaatctgaagcagaacgaccagcccatggatatcctgcagatcatcaactgcctgaccaccatctacgaccggctggaacaggaacacaacaatctcgtgaacgtgcccctgtgcgtggacatgtgcctgaattggctgctgaatgtgtacgacaccggccggacaggccggatcagagtgctgtccttcaagaccggcatcatcagcctgtgcaaagcccacctggaagataagtaccggtatctgttcaaacaggtggcctctagcaccggcttttgcgaccagagaaggctgggcctgctgctgcacgacagcatccagatccctagacagctgggcgaagtggccagctttggcggcagcaacatcgagcctagcgtgcggagctgcttccagttcgccaacaacaagcccgagatcgaggccgccctgttcctggactggatgagactggaaccccagagcatggtgtggctgcccgtgctgcatagagtggccgctgccgagacagccaagcaccaggccaagtgcaacatctgcaaagagtgccccatcatcggcttccggtacagaagcctgaagcacttcaactacgatatctgccagagctgtttcttcagcggcagggtggccaagggccacaaaatgcactaccccatggtggaatactgcacccccaccacaagcggcgaggatgtgcgggatttcgccaaggtgctgaaaaacaagttccggaccaagcggtacttcgccaaacacccccggatgggctacctgcctgtgcagacagtgctggaaggcgacaacatggaaaccgacaccatgtgatgatgatttgggcagagcgatggagtccttagtatcagtcatgacagatgaagaaggagcagaataaatgttttacaactcctgattcccgcatgcggccagcttatcgataccgtcgaaataaaagatccttattttcattggatctgtgtgttggttttttgtgtg

SEQ ID NO: 140 - DNA, 4146 bp, Homo sapiens
atgctgtggtgggaggaagtggaagattgctacgagcgcgaggacgtgcagaagaaaaccttcaccaaatgggtgaacgcccagttcagcaagttcggcaagcagcacatcgagaacctgttcagcgacctgcaggacggcagacggctgctggacctgctggaaggcctgaccggccagaagctgcccaaagagaagggcagcaccagagtgcacgccctgaacaacgtgaacaaggccctgcgggtgctgcagaacaacaacgtggacctggtgaacatcggcagcaccgacatcgtggacggcaaccacaagctgaccctgggcctgatctggaacatcatcctgcactggcaggtcaaaaacgtgatgaagaacatcatggccggcctgcagcagaccaacagcgagaagatcctgctgagctgggtgcgccagagcacccggaactacccccaggtcaacgtgatcaacttcaccacctcttggagcgacggcctggccctgaacgccctgatccacagccaccggcccgacctgttcgactggaacagcgtggtctgccagcagagcgccacccagcggctggaacacgccttcaatatcgccagataccagctgggcatcgagaagctgctggatcccgaggacgtggacaccacctaccccgacaagaaatccatcctgatgtatatcaccagcctgttccaggtgctgccccagcaggtgtccatcgaggccatccaggaagtggaaatgctgcccagaccccccaaagtgaccaaagaggaacacttccagctgcaccaccagatgcactacagccagcagatcaccgtgtccctggcccagggctacgagagaaccagcagccccaagccccggttcaagagctacgcctatacccaggccgcctacgtgaccaccagcgaccctaccagaagcccattccccagccagcatctggaagcccccgaggacaagagcttcggcagcagcctgatggaaagcgaagtgaacctggacagataccagaccgccctggaagaggtgctgagctggctgctgagcgccgaggatacactgcaggctcagggcgagatcagcaacgacgtggaagtcgtgaaggaccagttccacacccacgagggctacatgatggacctgacagcccaccagggcagagtgggcaacatcctgcagctgggctccaagctgatcggcaccggcaagctgagcgaggacgaagagacagaggtgcaggaacagatgaacctgctgaacagcagatgggagtgcctgcgggtggccagcatggaaaagcagagcaacctgcatctgctgaagtggcagcggctgaccgaggaacagtgcctgtttagcgcctggctgtccgagaaagaggacgccgtgaacaagatccacaccaccggcttcaaggaccagaacgagatgctgagcagcctgcagaaactggccgtgctgaaggccgacctggaaaagaaaaagcagtccatgggcaagctgtactccctgaagcaggacctgctgtccaccctgaagaacaagagcgtgacccagaaaaccgaggcctggctggacaacttcgcccggtgctgggacaacctggtgcagaagctggaaaagtccaccgcccagatctcccaggccgtgaccacaacacagcccagcctgacccagaccaccgtgatggaaaccgtgacaacagtgaccacccgggaacagatcctcgtgaagcacgcccaggaagaactgccccctccacccccccagaagaaacggcagatcacagtggacagtgaagctcagatccacaccgtgcgggaagagacaatgatggtcatgacagaggacatgcccctggaaatcagctacgtgcccagcacctacctgaccgagatcacccatgtgtcccaggccctgctggaagtggaacagctgctgaacgcccccgacctgtgcgccaaggatttcgaggacctgttcaagcaggaagagagcctgaagaatatcaaggatagcctgcagcagagcagcggccggatcgacatcatccacagcaagaaaacagccgccctgcagagcgccacccccgtggaaagagtgaaactgcaggaagccctgtcccagctggacttccagtgggagaaagtgaacaaaatgtacaaggaccggcagggcagattcgaccgcagcgtggaaaagtggcggcggttccactacgacatcaagatcttcaaccagtggctgacagaggccgagcagttcctgagaaagacccagatccccgagaactgggagcacgccaagtacaagtggtatctgaaagagctgcaggacggcatcggccagagacagacagtcgtgcggaccctgaatgccaccggcgaggaaatcatccagcagtccagcaagaccgacgccagcattctgcaggaaaagctgggcagcctgaacctgcggtggcaggaagtgtgcaagcagctgtccgaccggaagaagcggctggaagaacagctggaacggctgcaggaactgcaggaggccaccgacgagctggacctgaaactgagacaggccgaagtgatcaagggcagctggcagccagtgggcgacctgctgatcgactccctgcaggaccatctggaaaaagtgaaggccctgagaggcgagatcgcccccctgaaagaaaacgtgtcccacgtgaacgacctggcccggcagctgacaacactgggcattcagctgagcccctacaacctgagcacactggaagatctgaacacccggtggaagctgctgcaggtggccgtggaagatagagtgcggcagctgcacgaggcccacagagattttggccctgcctcccagcacttcctgagcaccagtgtgcagggcccttgggagagagccatctcccctaacaaggtgccctactacatcaaccacgagacacagaccacctgttgggaccaccccaagatgaccgagctgtaccagagcctggctgacctgaacaacgtgcggttcagcgcctaccggaccgccatgaagctgcggagactgcagaaagctctgtgcctggatctgctgtccctgtccgccgcctgtgatgccctggaccagcacaatctgaagcagaacgaccagcccatggatatcctgcagatcatcaactgcctgaccaccatctacgaccggctggaacaggaacacaacaatctcgtgaacgtgcccctgtgcgtggacatgtgcctgaattggctgctgaatgtgtacgacaccggccggacaggccggatcagagtgctgtccttcaagaccggcatcatcagcctgtgcaaagcccacctggaagataagtaccggtatctgttcaaacaggtggcctctagcaccggcttttgcgaccagagaaggctgggcctgctgctgcacgacagcatccagatccctagacagctgggcgaagtggccagctttggcggcagcaacatcgagcctagcgtgcggagctgcttccagttcgccaacaacaagcccgagatcgaggccgccctgttcctggactggatgagactggaaccccagagcatggtgtggctgcccgtgctgcatagagtggccgctgccgagacagccaagcaccaggccaagtgcaacatctgcaaagagtgccccatcatcggcttccggtacagaagcctgaagcacttcaactacgatatctgccagagctgtttcttcagcggcagggtggccaagggccacaaaatgcactaccccatggtggaatactgcacccccaccacaagcggcgaggatgtgcgggatttcgccaaggtgctgaaaaacaagttccggaccaagcggtacttcgccaaacacccccggatgggctacctgcctgtgcagacagtgctggaaggcgacaacatggaaaccgacaccatgtgatgatgatttgggcagagcgatggagtccttagtatcagtcatgacagatgaagaaggagcagaataaatgttttacaactcctgattcccgcatgcggccagcttatcgataccgtcgaaataaaagatccttattttcattggatctgtgtgttggttttttgtgtg

SEQ ID NO: 141 - DNA, 3936 bp, Homo sapiens
atgctgtggtgggaggaagtggaagattgctacgagcgcgaggacgtgcagaagaaaaccttcaccaaatgggtgaacgcccagttcagcaagttcggcaagcagcacatcgagaacctgttcagcgacctgcaggacggcagacggctgctggacctgctggaaggcctgaccggccagaagctgcccaaagagaagggcagcaccagagtgcacgccctgaacaacgtgaacaaggccctgcgggtgctgcagaacaacaacgtggacctggtgaacatcggcagcaccgacatcgtggacggcaaccacaagctgaccctgggcctgatctggaacatcatcctgcactggcaggtcaaaaacgtgatgaagaacatcatggccggcctgcagcagaccaacagcgagaagatcctgctgagctgggtgcgccagagcacccggaactacccccaggtcaacgtgatcaacttcaccacctcttggagcgacggcctggccctgaacgccctgatccacagccaccggcccgacctgttcgactggaacagcgtggtctgccagcagagcgccacccagcggctggaacacgccttcaatatcgccagataccagctgggcatcgagaagctgctggatcccgaggacgtggacaccacctaccccgacaagaaatccatcctgatgtatatcaccagcctgttccaggtgctgccccagcaggtgtccatcgaggccatccaggaagtggaaatgctgcccagaccccccaaagtgaccaaagaggaacacttccagctgcaccaccagatgcactacagccagcagatcaccgtgtccctggctcagggctacgagcggaccagcagccccaagccccggttcaagagctacgcctacacccaggccgcctacgtgaccaccagcgaccccaccagaagcccattccccagccagcatctggaagcccccgaggacaagagcttcggcagcagcctgatggaaagcgaagtgaacctggacagataccagaccgccctggaagaggtgctgtcctggctgctgagcgccgaggatacactgcaggcccagggcgagatcagcaacgacgtggaagtggtgaaagaccagttccacacccacgagggctacatgatggacctgaccgcccaccagggcagagtgggcaacatcctgcagctgggcagcaagctgatcggcaccggcaagctgagcgaggacgaagagacagaggtgcaggaacagatgaacctgctgaacagcagatgggagtgcctgcgggtggccagcatggaaaagcagagcaacctgcacatccacaccgtgcgggaagagacaatgatggtgatgaccgaggacatgcccctggaaatcagctacgtgcccagcacctacctgaccgagatcacccacgtgtcccaggctctgctggaagtggaacagctgctgaacgcccccgacctgtgcgccaaggacttcgaggatctgttcaagcaggaagagagcctgaagaatatcaaggactccctgcagcagtccagcggccggatcgacatcatccacagcaagaaaacagccgccctgcagtccgccacccccgtggaaagagtgaagctgcaggaagccctgagccagctggacttccagtgggagaaagtgaacaagatgtacaaggaccggcagggcagattcgaccgcagcgtggaaaagtggcggcggttccactacgacatcaagatcttcaaccagtggctgaccgaggccgagcagttcctgagaaagacccagatccccgagaactgggagcacgccaagtacaagtggtatctgaaagaactgcaggatggcatcggccagcggcagaccgtggtgcgcacactgaatgccaccggcgaggaaatcatccagcagagcagcaagaccgacgccagcatcctgcaggaaaagctgggctccctgaacctgcggtggcaggaagtgtgcaagcagctgagcgaccggaagaagaggctggaagaacaggcccctggcctgaccaccatcggcgccagccctacccagaccgtgaccctggtgacacagcccgtggtgacaaaagagacagccatctccaagctggaaatgcccagctccctgatgctggaactggaaaggctgcaggaactgcaggaggccaccgacgagctggacctgaagctgcggcaggccgaagtgatcaagggcagctggcagcccgtgggcgacctgctgatcgacagcctgcaggaccacctggaaaaagtgaaggccctgagaggcgagatcgcccccctgaaagaaaacgtgtcccacgtgaacgacctggcccggcagctgaccaccctgggcatccagctgagcccctacaacctgagcaccctggaagatctgaacacccggtggaagctgctgcaggtggccgtggaagatagagtgcggcagctgcacgaggcccacagagactttggccctgccagccagcacttcctgagcacctctgtgcagggaccctgggagagagccatcagccccaacaaggtgccctactacatcaaccacgagacacagaccacctgttgggaccaccccaagatgaccgagctgtaccagagcctggccgacctgaacaatgtgcggttcagcgcctaccggaccgccatgaagctgaggcggctgcagaaagctctgtgcctggatctgctgagcctgagcgccgcctgcgacgccctggaccagcacaacctgaagcagaacgaccagcccatggatatcctgcagatcatcaactgcctgaccacaatctacgacaggctggaacaggaacacaacaatctggtcaacgtgcccctgtgcgtggacatgtgcctgaattggctgctgaatgtgtacgacaccggccggaccggcagaatccgggtgctgagcttcaagaccggcatcatcagcctgtgcaaggcccacctggaagataagtaccgctacctgttcaaacaggtggccagctccaccggcttttgcgaccagcggagactgggcctgctgctgcacgacagcatccagatccccagacagctgggcgaggtggcctccttcggcggcagcaacattgagcccagcgtgcggagctgcttccagttcgccaacaacaagcccgagatcgaggccgccctgttcctggactggatgagactggaaccccagagcatggtgtggctgcccgtgctgcatcgggtggccgctgccgagacagccaagcaccaggccaagtgcaacatctgcaaagagtgccccatcatcggcttccggtacagaagcctgaagcacttcaactacgatatctgccagagctgcttcttcagcggcagagtggccaagggccacaaaatgcactaccccatggtggaatactgcacccccaccaccagcggcgaggatgtgcgggacttcgccaaggtgctgaaaaacaagttccggaccaagcggtactttgccaagcacccccggatgggctacctgcccgtgcagacagtgctggaaggcgacaacatggaaacccctgcccagatcctgatcagcctggaaagcgaggaacggggcgagctggaacggatcctggccgatctggaagaggaaaaccggaacctgcaggccgagtacgaccggctgaagcagcagcacgagcacaagggcctgagccccctgcctagcccccctgacaccatgtgatgatgatttgggcagagcgatggagtccttagtatcagtcatgacagatgaagaaggagcagaataaatgttttacaactcctgattcccgcatgcggccagcttatcgataccgtcgaaataaaagatccttattttcattggatctgtgtgttggttttttgtgtg

SEQ ID NO: 142 - DNA, 3957 bp, Homo sapiens
atgctgtggtgggaggaagtggaagattgctacgagcgcgaggacgtgcagaagaaaaccttcaccaaatgggtgaacgcccagttcagcaagttcggcaagcagcacatcgagaacctgttcagcgacctgcaggacggcagacggctgctggacctgctggaaggcctgaccggccagaagctgcccaaagagaagggcagcaccagagtgcacgccctgaacaacgtgaacaaggccctgcgggtgctgcagaacaacaacgtggacctggtgaacatcggcagcaccgacatcgtggacggcaaccacaagctgaccctgggcctgatctggaacatcatcctgcactggcaggtcaaaaacgtgatgaagaacatcatggccggcctgcagcagaccaacagcgagaagatcctgctgagctgggtgcgccagagcacccggaactacccccaggtcaacgtgatcaacttcaccacctcttggagcgacggcctggccctgaacgccctgatccacagccaccggcccgacctgttcgactggaacagcgtggtctgccagcagagcgccacccagcggctggaacacgccttcaatatcgccagataccagctgggcatcgagaagctgctggatcccgaggacgtggacaccacctaccccgacaagaaatccatcctgatgtatatcaccagcctgttccaggtgctgccccagcaggtgtccatcgaggccatccaggaagtggaaatgctgcccagaccccccaaagtgaccaaagaggaacacttccagctgcaccaccagatgcactacagccagcagatcaccgtgtccctggctcagggctacgagcggaccagcagccccaagccccggttcaagagctacgcctacacccaggccgcctacgtgaccaccagcgaccccaccagaagcccattccccagccagcatctggaagcccccgaggacaagagcttcggcagcagcctgatggaaagcgaagtgaacctggacagataccagaccgccctggaagaggtgctgtcctggctgctgagcgccgaggatacactgcaggcccagggcgagatcagcaacgacgtggaagtggtgaaagaccagttccacacccacgagggctacatgatggacctgaccgcccaccagggcagagtgggcaacatcctgcagctgggcagcaagctgatcggcaccggcaagctgagcgaggacgaagagacagaggtgcaggaacagatgaacctgctgaacagcagatgggagtgcctgcgggtggccagcatggaaaagcagagcaacctgcaccgggtgctgatccacaccgtgcgggaagagacaatgatggtgatgaccgaggacatgcccctggaaatcagctacgtgcccagcacctacctgaccgagatcacccacgtgtcccaggctctgctggaagtggaacagctgctgaacgcccccgacctgtgcgccaaggacttcgaggatctgttcaagcaggaagagagcctgaagaatatcaaggactccctgcagcagtccagcggccggatcgacatcatccacagcaagaaaacagccgccctgcagtccgccacccccgtggaaagagtgaagctgcaggaagccctgagccagctggacttccagtgggagaaagtgaacaagatgtacaaggaccggcagggcagattcgaccgcagcgtggaaaagtggcggcggttccactacgacatcaagatcttcaaccagtggctgaccgaggccgagcagttcctgagaaagacccagatccccgagaactgggagcacgccaagtacaagtggtatctgaaagaactgcaggatggcatcggccagcggcagaccgtggtgcgcacactgaatgccaccggcgaggaaatcatccagcagagcagcaagaccgacgccagcatcctgcaggaaaagctgggctccctgaacctgcggtggcaggaagtgtgcaagcagctgagcgaccggaagaagaggctggaagaacagaagaacgacctggcccctggcctgaccaccatcggcgccagccctacccagaccgtgaccctggtgacacagcccgtggtgacaaaagagacagccatctccaagctggaaatgcccagctccctgatgctggaagtggaaaggctgcaggaactgcaggaggccaccgacgagctggacctgaagctgcggcaggccgaagtgatcaagggcagctggcagcccgtgggcgacctgctgatcgacagcctgcaggaccacctggaaaaagtgaaggccctgagaggcgagatcgcccccctgaaagaaaacgtgtcccacgtgaacgacctggcccggcagctgaccaccctgggcatccagctgagcccctacaacctgagcaccctggaagatctgaacacccggtggaagctgctgcaggtggccgtggaagatagagtgcggcagctgcacgaggcccacagagactttggccctgccagccagcacttcctgagcacctctgtgcagggaccctgggagagagccatcagccccaacaaggtgccctactacatcaaccacgagacacagaccacctgttgggaccaccccaagatgaccgagctgtaccagagcctggccgacctgaacaatgtgcggttcagcgcctaccggaccgccatgaagctgaggcggctgcagaaagctctgtgcctggatctgctgagcctgagcgccgcctgcgacgccctggaccagcacaacctgaagcagaacgaccagcccatggatatcctgcagatcatcaactgcctgaccacaatctacgacaggctggaacaggaacacaacaatctggtcaacgtgcccctgtgcgtggacatgtgcctgaattggctgctgaatgtgtacgacaccggccggaccggcagaatccgggtgctgagcttcaagaccggcatcatcagcctgtgcaaggcccacctggaagataagtaccgctacctgttcaaacaggtggccagctccaccggcttttgcgaccagcggagactgggcctgctgctgcacgacagcatccagatccccagacagctgggcgaggtggcctccttcggcggcagcaacattgagcccagcgtgcggagctgcttccagttcgccaacaacaagcccgagatcgaggccgccctgttcctggactggatgagactggaaccccagagcatggtgtggctgcccgtgctgcatcgggtggccgctgccgagacagccaagcaccaggccaagtgcaacatctgcaaagagtgccccatcatcggcttccggtacagaagcctgaagcacttcaactacgatatctgccagagctgcttcttcagcggcagagtggccaagggccacaaaatgcactaccccatggtggaatactgcacccccaccaccagcggcgaggatgtgcgggacttcgccaaggtgctgaaaaacaagttccggaccaagcggtactttgccaagcacccccggatgggctacctgcccgtgcagacagtgctggaaggcgacaacatggaaacccctgcccagatcctgatcagcctggaaagcgaggaacggggcgagctggaacggatcctggccgatctggaagaggaaaaccggaacctgcaggccgagtacgaccggctgaagcagcagcacgagcacaagggcctgagccccctgcctagcccccctgacaccatgtgatgatgatttgggcagagcgatggagtccttagtatcagtcatgacagatgaagaaggagcagaataaatgttttacaactcctgattcccgcatgcggccagcttatcgataccgtcgaaataaaagatccttattttcattggatctgtgtgttggttttttgtgtg

SEQ ID NO: 143 - DNA, 3918 bp, Homo sapiens
atgctgtggtgggaggaagtggaagattgctacgagcgcgaggacgtgcagaagaaaaccttcaccaaatgggtgaacgcccagttcagcaagttcggcaagcagcacatcgagaacctgttcagcgacctgcaggacggcagacggctgctggacctgctggaaggcctgaccggccagaagctgcccaaagagaagggcagcaccagagtgcacgccctgaacaacgtgaacaaggccctgcgggtgctgcagaacaacaacgtggacctggtgaacatcggcagcaccgacatcgtggacggcaaccacaagctgaccctgggcctgatctggaacatcatcctgcactggcaggtcaaaaacgtgatgaagaacatcatggccggcctgcagcagaccaacagcgagaagatcctgctgagctgggtgcgccagagcacccggaactacccccaggtcaacgtgatcaacttcaccacctcttggagcgacggcctggccctgaacgccctgatccacagccaccggcccgacctgttcgactggaacagcgtggtctgccagcagagcgccacccagcggctggaacacgccttcaatatcgccagataccagctgggcatcgagaagctgctggatcccgaggacgtggacaccacctaccccgacaagaaatccatcctgatgtatatcaccagcctgttccaggtgctgccccagcaggtgtccatcgaggccatccaggaagtggaaatgctgcccagaccccccaaagtgaccaaagaggaacacttccagctgcaccaccagatgcactacagccagcagatcaccgtgtccctggctcagggctacgagcggaccagcagccccaagccccggttcaagagctacgcctacacccaggccgcctacgtgaccaccagcgaccccaccagaagcccattccccagccagcatctggaagcccccgaggacaagagcttcggcagcagcctgatggaaagcgaagtgaacctggacagataccagaccgccctggaagaggtgctgtcctggctgctgagcgccgaggatacactgcaggcccagggcgagatcagcaacgacgtggaagtggtgaaagaccagttccacacccacgagggctacatgatggacctgaccgcccaccagggcagagtgggcaacatcctgcagctgggcagcaagctgatcggcaccggcaagctgagcgaggacgaagagacagaggtgcaggaacagatgaacctgctgaacagcagatgggagtgcctgcgggtggccagcatggaaaagcagagcaacctgcacagctacgtgcccagcacctacctgaccgagatcacccacgtgtcccaggctctgctggaagtggaacagctgctgaacgcccccgacctgtgcgccaaggacttcgaggatctgttcaagcaggaagagagcctgaagaatatcaaggactccctgcagcagtccagcggccggatcgacatcatccacagcaagaaaacagccgccctgcagtccgccacccccgtggaaagagtgaagctgcaggaagccctgagccagctggacttccagtgggagaaagtgaacaagatgtacaaggaccggcagggcagattcgaccgcagcgtggaaaagtggcggcggttccactacgacatcaagatcttcaaccagtggctgaccgaggccgagcagttcctgagaaagacccagatccccgagaactgggagcacgccaagtacaagtggtatctgaaagaactgcaggatggcatcggccagcggcagaccgtggtgcgcacactgaatgccaccggcgaggaaatcatccagcagagcagcaagaccgacgccagcatcctgcaggaaaagctgggctccctgaacctgcggtggcaggaagtgtgcaagcagctgagcgaccggaagaagaggctggaagaacagctggaaggactggaaaagctgtaccaggaacccagagagctgccccccgaggaacgggcccagaacgtgacccggctgctgcggaaacaggccgaagaggtgaacaccgagtgggagaagctgaacctgcactccgccgactggcagcggaagatcgacgagacactggaaaggctgcaggaactgcaggaggccaccgacgagctggacctgaagctgcggcaggccgaagtgatcaagggcagctggcagcccgtgggcgacctgctgatcgacagcctgcaggaccacctggaaaaagtgaaggccctgagaggcgagatcgcccccctgaaagaaaacgtgtcccacgtgaacgacctggcccggcagctgaccaccctgggcatccagctgagcccctacaacctgagcaccctggaagatctgaacacccggtggaagctgctgcaggtggccgtggaagatagagtgcggcagctgcacgaggcccacagagactttggccctgccagccagcacttcctgagcacctctgtgcagggaccctgggagagagccatcagccccaacaaggtgccctactacatcaaccacgagacacagaccacctgttgggaccaccccaagatgaccgagctgtaccagagcctggccgacctgaacaatgtgcggttcagcgcctaccggaccgccatgaagctgaggcggctgcagaaagctctgtgcctggatctgctgagcctgagcgccgcctgcgacgccctggaccagcacaacctgaagcagaacgaccagcccatggatatcctgcagatcatcaactgcctgaccacaatctacgacaggctggaacaggaacacaacaatctggtcaacgtgcccctgtgcgtggacatgtgcctgaattggctgctgaatgtgtacgacaccggccggaccggcagaatccgggtgctgagcttcaagaccggcatcatcagcctgtgcaaggcccacctggaagataagtaccgctacctgttcaaacaggtggccagctccaccggcttttgcgaccagcggagactgggcctgctgctgcacgacagcatccagatccccagacagctgggcgaggtggcctccttcggcggcagcaacattgagcccagcgtgcggagctgcttccagttcgccaacaacaagcccgagatcgaggccgccctgttcctggactggatgagactggaaccccagagcatggtgtggctgcccgtgctgcatcgggtggccgctgccgagacagccaagcaccaggccaagtgcaacatctgcaaagagtgccccatcatcggcttccggtacagaagcctgaagcacttcaactacgatatctgccagagctgcttcttcagcggcagagtggccaagggccacaaaatgcactaccccatggtggaatactgcacccccaccaccagcggcgaggatgtgcgggacttcgccaaggtgctgaaaaacaagttccggaccaagcggtactttgccaagcacccccggatgggctacctgcccgtgcagacagtgctggaaggcgacaacatggaaacccctgcccagatcctgatcagcctggaaagcgaggaacggggcgagctggaacggatcctggccgatctggaagaggaaaaccggaacctgcaggccgagtacgaccggctgaagcagcagcacgagcacaagggcctgagccccctgcctagcccccctgacaccatgtgatgatgatttgggcagagcgatggagtccttagtatcagtcatgacagatgaagaaggagcagaataaatgttttacaactcctgattcccgcatgcggccagcttatcgataccgtcgaaataaaagatccttattttcattggatctgtgtgttggttttttgtgtg

SEQ ID NO: 144 - DNA, 4244 bp, Homo sapiens
atgctgtggtgggaggaagtggaagattgctacgagcgcgaggacgtgcagaagaaaaccttcaccaaatgggtgaacgcccagttcagcaagttcggcaagcagcacatcgagaacctgttcagcgacctgcaggacggcagacggctgctggacctgctggaaggcctgaccggccagaagctgcccaaagagaagggcagcaccagagtgcacgccctgaacaacgtgaacaaggccctgcgggtgctgcagaacaacaacgtggacctggtgaacatcggcagcaccgacatcgtggacggcaaccacaagctgaccctgggcctgatctggaacatcatcctgcactggcaggtcaaaaacgtgatgaagaacatcatggccggcctgcagcagaccaacagcgagaagatcctgctgagctgggtgcgccagagcacccggaactacccccaggtcaacgtgatcaacttcaccacctcttggagcgacggcctggccctgaacgccctgatccacagccaccggcccgacctgttcgactggaacagcgtggtctgccagcagagcgccacccagcggctggaacacgccttcaatatcgccagataccagctgggcatcgagaagctgctggatcccgaggacgtggacaccacctaccccgacaagaaatccatcctgatgtatatcaccagcctgttccaggtgctgccccagcaggtgtccatcgaggccatccaggaagtggaaatgctgcccagaccccccaaagtgaccaaagaggaacacttccagctgcaccaccagatgcactacagccagcagatcaccgtgtccctggcccagggctacgagagaaccagcagccccaagccccggttcaagagctacgcctatacccaggccgcctacgtgaccaccagcgaccctaccagaagcccattccccagccagcatctggaagcccccgaggacaagagcttcggcagcagcctgatggaaagcgaagtgaacctggacagataccagaccgccctggaagaggtgctgagctggctgctgagcgccgaggatacactgcaggctcagggcgagatcagcaacgacgtggaagtcgtgaaggaccagttccacacccacgagggctacatgatggacctgacagcccaccagggcagagtgggcaacatcctgcagctgggctccaagctgatcggcaccggcaagctgagcgaggacgaagagacagaggtgcaggaacagatgaacctgctgaacagcagatgggagtgcctgcgggtggccagcatggaaaagcagagcaacctgcatctgctgaagtggcagcggctgaccgaggaacagtgcctgtttagcgcctggctgtccgagaaagaggacgccgtgaacaagatccacaccaccggcttcaaggaccagaacgagatgctgagcagcctgcagaaactggccgtgctgaaggccgacctggaaaagaaaaagcagtccatgggcaagctgtactccctgaagcaggacctgctgtccaccctgaagaacaagagcgtgacccagaaaaccgaggcctggctggacaacttcgcccggtgctgggacaacctggtgcagaagctggaaaagtccaccgcccagatctcccaggccgtgaccacaacacagcccagcctgacccagaccaccgtgatggaaaccgtgacaacagtgaccacccgggaacagatcctcgtgaagcacgcccaggaagaactgccccctccacccccccagaagaaacggcagatcacagtggacatccacaccgtgcgggaagagacaatgatggtcatgacagaggacatgcccctggaaatcagctacgtgcccagcacctacctgaccgagatcacccatgtgtcccaggccctgctggaagtggaacagctgctgaacgcccccgacctgtgcgccaaggatttcgaggacctgttcaagcaggaagagagcctgaagaatatcaaggatagcctgcagcagagcagcggccggatcgacatcatccacagcaagaaaacagccgccctgcagagcgccacccccgtggaaagagtgaaactgcaggaagccctgtcccagctggacttccagtgggagaaagtgaacaaaatgtacaaggaccggcagggcagattcgaccgcagcgtggaaaagtggcggcggttccactacgacatcaagatcttcaaccagtggctgacagaggccgagcagttcctgagaaagacccagatccccgagaactgggagcacgccaagtacaagtggtatctgaaagagctgcaggacggcatcggccagagacagacagtcgtgcggaccctgaatgccaccggcgaggaaatcatccagcagtccagcaagaccgacgccagcattctgcaggaaaagctgggcagcctgaacctgcggtggcaggaagtgtgcaagcagctgtccgaccggaagaagcggctggaagaacagctggaacggctgcaggaactgcaggaggccaccgacgagctggacctgaaactgagacaggccgaagtgatcaagggcagctggcagccagtgggcgacctgctgatcgactccctgcaggaccatctggaaaaagtgaaggccctgagaggcgagatcgcccccctgaaagaaaacgtgtcccacgtgaacgacctggcccggcagctgacaacactgggcattcagctgagcccctacaacctgagcacactggaagatctgaacacccggtggaagctgctgcaggtggccgtggaagatagagtgcggcagctgcacgaggcccacagagattttggccctgcctcccagcacttcctgagcaccagtgtgcagggcccttgggagagagccatctcccctaacaaggtgccctactacatcaaccacgagacacagaccacctgttgggaccaccccaagatgaccgagctgtaccagagcctggctgacctgaacaacgtgcggttcagcgcctaccggaccgccatgaagctgcggagactgcagaaagctctgtgcctggatctgctgtccctgtccgccgcctgtgatgccctggaccagcacaatctgaagcagaacgaccagcccatggatatcctgcagatcatcaactgcctgaccaccatctacgaccggctggaacaggaacacaacaatctcgtgaacgtgcccctgtgcgtggacatgtgcctgaattggctgctgaatgtgtacgacaccggccggacaggccggatcagagtgctgtccttcaagaccggcatcatcagcctgtgcaaagcccacctggaagataagtaccggtatctgttcaaacaggtggcctctagcaccggcttttgcgaccagagaaggctgggcctgctgctgcacgacagcatccagatccctagacagctgggcgaagtggccagctttggcggcagcaacatcgagcctagcgtgcggagctgcttccagttcgccaacaacaagcccgagatcgaggccgccctgttcctggactggatgagactggaaccccagagcatggtgtggctgcccgtgctgcatagagtggccgctgccgagacagccaagcaccaggccaagtgcaacatctgcaaagagtgccccatcatcggcttccggtacagaagcctgaagcacttcaactacgatatctgccagagctgtttcttcagcggcagggtggccaagggccacaaaatgcactaccccatggtggaatactgcacccccaccacaagcggcgaggatgtgcgggatttcgccaaggtgctgaaaaacaagttccggaccaagcggtacttcgccaaacacccccggatgggctacctgcctgtgcagacagtgctggaaggcgacaacatggaaacccctgcccagatcctgatcagcctggaatccgaggaacggggcgagctggaacggatcctggccgatctggaagaggaaaaccggaacctgcaggccgagtacgaccggctgaagcagcagcacgagcacaagggcctgagccccctgcctagcccccctgacaccatgtgatgatgatttgggcagagcgatggagtccttagtatcagtcatgacagatgaagaaggagcagaataaatgttttacaactcctgattcccgcatgcggccagcttatcgataccgtcga

SEQ ID NO: 145 - DNA, 4266 bp, Homo sapiens
atgctgtggtgggaggaagtggaagattgctacgagcgcgaggacgtgcagaagaaaaccttcaccaaatgggtgaacgcccagttcagcaagttcggcaagcagcacatcgagaacctgttcagcgacctgcaggacggcagacggctgctggacctgctggaaggcctgaccggccagaagctgcccaaagagaagggcagcaccagagtgcacgccctgaacaacgtgaacaaggccctgcgggtgctgcagaacaacaacgtggacctggtgaacatcggcagcaccgacatcgtggacggcaaccacaagctgaccctgggcctgatctggaacatcatcctgcactggcaggtcaaaaacgtgatgaagaacatcatggccggcctgcagcagaccaacagcgagaagatcctgctgagctgggtgcgccagagcacccggaactacccccaggtcaacgtgatcaacttcaccacctcttggagcgacggcctggccctgaacgccctgatccacagccaccggcccgacctgttcgactggaacagcgtggtctgccagcagagcgccacccagcggctggaacacgccttcaatatcgccagataccagctgggcatcgagaagctgctggatcccgaggacgtggacaccacctaccccgacaagaaatccatcctgatgtatatcaccagcctgttccaggtgctgccccagcaggtgtccatcgaggccatccaggaagtggaaatgctgcccagaccccccaaagtgaccaaagaggaacacttccagctgcaccaccagatgcactacagccagcagatcaccgtgtccctggctcagggctacgagcggaccagcagccccaagccccggttcaagagctacgcctacacccaggccgcctacgtgaccaccagcgaccccaccagaagcccattccccagccagcatctggaagcccccgaggacaagagcttcggcagcagcctgatggaaagcgaagtgaacctggacagataccagaccgccctggaagaggtgctgtcctggctgctgagcgccgaggatacactgcaggcccagggcgagatcagcaacgacgtggaagtggtgaaagaccagttccacacccacgagggctacatgatggacctgaccgcccaccagggcagagtgggcaacatcctgcagctgggcagcaagctgatcggcaccggcaagctgagcgaggacgaagagacagaggtgcaggaacagatgaacctgctgaacagcagatgggagtgcctgcgggtggccagcatggaaaagcagagcaacctgcacatccacaccgtgcgggaagagacaatgatggtgatgaccgaggacatgcccctggaaatcagctacgtgcccagcacctacctgaccgagatcacccacgtgtcccaggctctgctggaagtggaacagctgctgaacgcccccgacctgtgcgccaaggacttcgaggatctgttcaagcaggaagagagcctgaagaatatcaaggactccctgcagcagtccagcggccggatcgacatcatccacagcaagaaaacagccgccctgcagtccgccacccccgtggaaagagtgaagctgcaggaagccctgagccagctggacttccagtgggagaaagtgaacaagatgtacaaggaccggcagggcagattcgaccgcagcgtggaaaagtggcggcggttccactacgacatcaagatcttcaaccagtggctgaccgaggccgagcagttcctgagaaagacccagatccccgagaactgggagcacgccaagtacaagtggtatctgaaagaactgcaggatggcatcggccagcggcagaccgtggtgcgcacactgaatgccaccggcgaggaaatcatccagcagagcagcaagaccgacgccagcatcctgcaggaaaagctgggctccctgaacctgcggtggcaggaagtgtgcaagcagctgagcgaccggaagaagaggctggaagaacaggcccctggcctgaccaccatcggcgccagccctacccagaccgtgaccctggtgacacagcccgtggtgacaaaagagacagccatctccaagctggaaatgcccagctccctgatgctggaagtacctgctctggcagatttcaaccgggcttggacagaacttaccgactggctttctctgcttgatcaagttataaaatcacagagggtgatggtgggtgaccttgaggatatcaacgagatgatcatcaagcagaaggcaacaatgcaggatttggaacagaggcgtccccagttggaagaactcattaccgctgcccaaaatttgaaaaacaagaccagcaatcaagaggctagaacaatcattacggatcgaattgaaagaattcagaatcagtgggatgaagtacaagaacaccttcagaaccggaggcaacagttgaatgaaatgctggaaaggctgcaggaactgcaggaggccaccgacgagctggacctgaagctgcggcaggccgaagtgatcaagggcagctggcagcccgtgggcgacctgctgatcgacagcctgcaggaccacctggaaaaagtgaaggccctgagaggcgagatcgcccccctgaaagaaaacgtgtcccacgtgaacgacctggcccggcagctgaccaccctgggcatccagctgagcccctacaacctgagcaccctggaagatctgaacacccggtggaagctgctgcaggtggccgtggaagatagagtgcggcagctgcacgaggcccacagagactttggccctgccagccagcacttcctgagcacctctgtgcagggaccctgggagagagccatcagccccaacaaggtgccctactacatcaaccacgagacacagaccacctgttgggaccaccccaagatgaccgagctgtaccagagcctggccgacctgaacaatgtgcggttcagcgcctaccggaccgccatgaagctgaggcggctgcagaaagctctgtgcctggatctgctgagcctgagcgccgcctgcgacgccctggaccagcacaacctgaagcagaacgaccagcccatggatatcctgcagatcatcaactgcctgaccacaatctacgacaggctggaacaggaacacaacaatctggtcaacgtgcccctgtgcgtggacatgtgcctgaattggctgctgaatgtgtacgacaccggccggaccggcagaatccgggtgctgagcttcaagaccggcatcatcagcctgtgcaaggcccacctggaagataagtaccgctacctgttcaaacaggtggccagctccaccggcttttgcgaccagcggagactgggcctgctgctgcacgacagcatccagatccccagacagctgggcgaggtggcctccttcggcggcagcaacattgagcccagcgtgcggagctgcttccagttcgccaacaacaagcccgagatcgaggccgccctgttcctggactggatgagactggaaccccagagcatggtgtggctgcccgtgctgcatcgggtggccgctgccgagacagccaagcaccaggccaagtgcaacatctgcaaagagtgccccatcatcggcttccggtacagaagcctgaagcacttcaactacgatatctgccagagctgcttcttcagcggcagagtggccaagggccacaaaatgcactaccccatggtggaatactgcacccccaccaccagcggcgaggatgtgcgggacttcgccaaggtgctgaaaaacaagttccggaccaagcggtactttgccaagcacccccggatgggctacctgcccgtgcagacagtgctggaaggcgacaacatggaaacccctgcccagatcctgatcagcctggaaagcgaggaacggggcgagctggaacggatcctggccgatctggaagaggaaaaccggaacctgcaggccgagtacgaccggctgaagcagcagcacgagcacaagggcctgagccccctgcctagcccccctgacaccatgtgatgatgatttgggcagagcgatggagtccttagtatcagtcatgacagatgaagaaggagcagaataaatgttttacaactcctgattcccgcatgcggccagcttatcgataccgtcgaaataaaagatccttattttcattggatctgtgtgttggttttttgtgtg

SEQ ID NO: 146 - DNA, 4320 bp, Homo sapiens
atgctgtggtgggaggaagtggaagattgctacgagcgcgaggacgtgcagaagaaaaccttcaccaaatgggtcaacgcccagttcagcaagttcggcaagcagcacatcgagaacctgttcagcgacctgcaggacggcagacggctgctggatctgctggaaggcctgaccggacagaagctgcccaaagagaagggcagcaccagagtgcacgccctgaacaacgtgaacaaggccctgcgggtgctgcagaacaacaacgtggacctcgtgaacatcggcagcaccgacatcgtggacggcaaccacaagctgaccctgggcctgatctggaacatcatcctgcactggcaagtgaagaacgtgatgaagaacatcatggccggcctgcagcagaccaacagcgagaagatcctgctgagctgggtgcgccagagcaccagaaactacccccaagtgaacgtgatcaacttcaccacctcttggagcgacggcctggccctgaatgccctgatccacagccacagacccgacctgttcgactggaacagcgtcgtgtgtcagcagagcgccacccagaggctggaacacgccttcaatatcgccagataccagctgggcatcgagaagctgctggaccccgaggatgtggacaccacctaccccgacaagaaatccatcctgatgtatatcaccagcctgttccaggtgctgcctcagcaggtgtccatcgaggccatccaggaagtggaaatgctgcccagaccccccaaagtgaccaaagaggaacacttccagctgcaccaccagatgcactactctcagcagatcaccgtgtccctggcccagggctacgagagaaccagcagccccaagccccggttcaagagctacgcctatacccaggccgcctacgtgaccaccagcgaccctaccagaagcccattccccagccagcatctggaagcccccgaggacaagagcttcggcagcagcctgatggaaagcgaagtgaacctggatagataccagaccgccctggaagaggtgctgtcctggctgctgagcgccgaggatacactgcaggctcagggcgagatcagcaacgacgtggaagtcgtgaaggaccagttccacacccacgagggctacatgatggacctgacagcccaccagggcagagtgggcaacattctgcagctgggctccaagctgatcggcaccggcaagctgagcgaggacgaagagacagaggtgcaggaacagatgaacctgctgaacagcagatgggagtgcctgagagtggccagcatggaaaagcagagcaacctgcaccgggtgctgatggatctgcagaaccagaagctgaaagagctgaacgactggctgaccaagaccgaggaacggacccggaagatggaagaggaacccctgggaccagacctggaagatctgaaaagacaggtgcagcagcacaaagtgctgcaggaagatctggaacaggaacaggtgcgcgtgaacagcctgacccacatggtcgtggtggtggacgagagcagcggcgatcatgccacagccgctctggaagaacagctgaaggtgctgggcgacagatgggccaacatctgccggtggaccgaggatagatgggtgctgctgcaggacatcctgctgaagtggcagcggctgacagaggaacagtgcctgttctccgcctggctgtccgagaaagaggacgccgtgaacaaaatccacaccaccggcttcaaggaccagaacgagatgctgagcagcctgcagaaactggccgtgctgaaggccgacctggaaaagaaaaagcagtccatgggcaagctgtactccctgaagcaggacctgctgtccaccctgaagaacaagagcgtgacccagaaaaccgaggcctggctggacaacttcgcccggtgctgggacaacctggtgcagaagctggaaaagtccaccgcccagatctcccaggccattcacaccgtgcgggaagagacaatgatggtcatgactgaggacatgcccctggaaatcagctacgtgccctccacctacctgaccgagatcacccatgtgtcccaggccctgctggaagtggaacagctgctgaacgcccccgatctgtgcgccaaggacttcgaggatctgttcaagcaggaagagagcctgaagaatatcaaggactctctgcagcagtccagcggcagaatcgacatcatccacagcaagaaaacagccgccctgcagtccgccacccccgtggaaagagtgaaactgcaggaagccctgtcccagctggacttccagtgggagaaagtgaacaagatgtacaaggaccggcagggcagattcgaccgcagcgtggaaaagtggcggcggttccactacgacatcaagatcttcaaccagtggctgaccgaggccgaacagttcctgagaaagacccagatccccgagaactgggagcacgccaagtacaagtggtatctgaaagaactgcaggatggcatcggccagagacagaccgtcgtgcggacactgaatgccaccggcgaggaaatcatccagcagagcagcaagaccgacgccagcatcctgcaggaaaagctgggcagcctgaacctgagatggcaggaagtgtgcaagcagctgtccgaccggaagaagcggctggaagaacagctggaacggctgcaggaactgcaggaggccaccgacgagctggacctgaaactgagacaggccgaagtgatcaagggcagctggcagccagtgggcgacctgctgatcgattctctgcaggaccacctggaaaaagtgaaggccctgagaggcgagatcgcccccctgaaagaaaacgtgtcccacgtgaacgacctggcccggcagctgacaacactgggcatccagctgagcccctacaacctgagcacactggaagatctgaacacccggtggaagctgctgcaggtggccgtggaagatagagtgcggcagctgcacgaggcccacagagattttggccctgcctcccagcacttcctgagcacctcagtgcagggcccttgggagagagccatctcccctaacaaggtgccctactacatcaaccacgagacacagaccacctgttgggaccaccccaagatgaccgagctgtaccagagcctggccgacctgaacaatgtgcggttcagcgcctaccggaccgccatgaagctgcggagactgcagaaagctctgtgcctggatctgctgtccctgagcgccgcctgtgatgccctggaccagcacaatctgaagcagaacgaccagcccatggatatcctgcagatcattaactgcctgaccaccatctacgaccggctggaacaggaacacaacaacctcgtgaacgtgcccctgtgcgtggacatgtgcctgaattggctgctgaatgtgtacgacaccggccggacaggccggatcagagtgctgagcttcaagaccggcatcatcagcctgtgcaaagcccatctggaagataagtaccgctacctgttcaaacaggtggccagctctaccggcttctgcgatcagagaaggctgggcctgctgctgcatgactccatccagatccccagacagctgggcgaggtggcctctttcggcggcagcaatatcgagcctagcgtgcggagctgcttccagttcgccaacaacaagcccgagatcgaggccgccctgtttctggactggatgagactggaaccccagagcatggtgtggctgcccgtgctgcatagagtggccgctgccgagacagccaagcaccaggccaagtgcaatatctgcaaagagtgccccatcatcggcttccggtacagaagcctgaagcacttcaactacgatatctgccagagctgtttcttcagcggcagggtggccaagggccacaaaatgcactaccccatggtggaatactgcacccccaccacaagcggagaggatgtgcgggacttcgccaaggtgctgaaaaacaagttccggaccaagcggtatttcgccaaacacccccggatgggctacctgcctgtgcagacagtgctggaaggcgacaacatggaaaccgacaccatgtgatgatgatttgggcagagcgatggagtccttagtatcagtcatgacagatgaagaaggagcagaataaatgttttacaactcctgattcccgcatgcggccagcttatcgataccgtcgaaataaaagatccttattttcattggatctgtgtgttggttttttgtgtg

SEQ ID NO: 147 - DNA, 4323 bp, Homo sapiens
atgctgtggtgggaggaagtggaagattgctacgagcgcgaggacgtgcagaagaaaaccttcaccaaatgggtgaacgcccagttcagcaagttcggcaagcagcacatcgagaacctgttcagcgacctgcaggacggcagacggctgctggacctgctggaaggcctgaccggccagaagctgcccaaagagaagggcagcaccagagtgcacgccctgaacaacgtgaacaaggccctgcgggtgctgcagaacaacaacgtggacctggtgaacatcggcagcaccgacatcgtggacggcaaccacaagctgaccctgggcctgatctggaacatcatcctgcactggcaggtcaaaaacgtgatgaagaacatcatggccggcctgcagcagaccaacagcgagaagatcctgctgagctgggtgcgccagagcacccggaactacccccaggtcaacgtgatcaacttcaccacctcttggagcgacggcctggccctgaacgccctgatccacagccaccggcccgacctgttcgactggaacagcgtggtctgccagcagagcgccacccagcggctggaacacgccttcaatatcgccagataccagctgggcatcgagaagctgctggatcccgaggacgtggacaccacctaccccgacaagaaatccatcctgatgtatatcaccagcctgttccaggtgctgccccagcaggtgtccatcgaggccatccaggaagtggaaatgctgcccagaccccccaaagtgaccaaagaggaacacttccagctgcaccaccagatgcactacagccagcagatcaccgtgtccctggctcagggctacgagcggaccagcagccccaagccccggttcaagagctacgcctacacccaggccgcctacgtgaccaccagcgaccccaccagaagcccattccccagccagcatctggaagcccccgaggacaagagcttcggcagcagcctgatggaaagcgaagtgaacctggacagataccagaccgccctggaagaggtgctgtcctggctgctgagcgccgaggatacactgcaggcccagggcgagatcagcaacgacgtggaagtggtgaaagaccagttccacacccacgagggctacatgatggacctgaccgcccaccagggcagagtgggcaacatcctgcagctgggcagcaagctgatcggcaccggcaagctgagcgaggacgaagagacagaggtgcaggaacagatgaacctgctgaacagcagatgggagtgcctgcgggtggccagcatggaaaagcagagcaacctgcacatccacaccgtgcgggaagagacaatgatggtgatgaccgaggacatgcccctggaaatcagctacgtgcccagcacctacctgaccgagatcacccacgtgtcccaggctctgctggaagtggaacagctgctgaacgcccccgacctgtgcgccaaggacttcgaggatctgttcaagcaggaagagagcctgaagaatatcaaggactccctgcagcagtccagcggccggatcgacatcatccacagcaagaaaacagccgccctgcagtccgccacccccgtggaaagagtgaagctgcaggaagccctgagccagctggacttccagtgggagaaagtgaacaagatgtacaaggaccggcagggcagattcgaccgcagcgtggaaaagtggcggcggttccactacgacatcaagatcttcaaccagtggctgaccgaggccgagcagttcctgagaaagacccagatccccgagaactgggagcacgccaagtacaagtggtatctgaaagaactgcaggatggcatcggccagcggcagaccgtggtgcgcacactgaatgccaccggcgaggaaatcatccagcagagcagcaagaccgacgccagcatcctgcaggaaaagctgggctccctgaacctgcggtggcaggaagtgtgcaagcagctgagcgaccggaagaagaggctggaagaacaggcccctggcctgaccaccatcggcgccagccctacccagaccgtgaccctggtgacacagcccgtggtgacaaaagagacagccatctccaagctggaaatgcccagctccctgatgctggaatctgaccagtggaagcgtctgcacctttctctgcaggaacttctggtgtggctacagctgaaagatgatgaattaagccggcaggcacctattggaggcgactttccagcagttcagaagcagaacgatgtacatagggccttcaagagggaattgaaaactaaagaacctgtaatcatgagtactcttgagactgtacgaatatttctgacagagcagcctttggaaggactagagaaactctaccaggagcccagagagctgcctcctgaggagagagcccagaatgtcactcggcttctacgaaagcaggctgaggaggtcaatactgagtgggaaaaattgaacctgcactccgctgactggcagagaaaaatagatgagaccctggaaaggctgcaggaactgcaggaggccaccgacgagctggacctgaagctgcggcaggccgaagtgatcaagggcagctggcagcccgtgggcgacctgctgatcgacagcctgcaggaccacctggaaaaagtgaaggccctgagaggcgagatcgcccccctgaaagaaaacgtgtcccacgtgaacgacctggcccggcagctgaccaccctgggcatccagctgagcccctacaacctgagcaccctggaagatctgaacacccggtggaagctgctgcaggtggccgtggaagatagagtgcggcagctgcacgaggcccacagagactttggccctgccagccagcacttcctgagcacctctgtgcagggaccctgggagagagccatcagccccaacaaggtgccctactacatcaaccacgagacacagaccacctgttgggaccaccccaagatgaccgagctgtaccagagcctggccgacctgaacaatgtgcggttcagcgcctaccggaccgccatgaagctgaggcggctgcagaaagctctgtgcctggatctgctgagcctgagcgccgcctgcgacgccctggaccagcacaacctgaagcagaacgaccagcccatggatatcctgcagatcatcaactgcctgaccacaatctacgacaggctggaacaggaacacaacaatctggtcaacgtgcccctgtgcgtggacatgtgcctgaattggctgctgaatgtgtacgacaccggccggaccggcagaatccgggtgctgagcttcaagaccggcatcatcagcctgtgcaaggcccacctggaagataagtaccgctacctgttcaaacaggtggccagctccaccggcttttgcgaccagcggagactgggcctgctgctgcacgacagcatccagatccccagacagctgggcgaggtggcctccttcggcggcagcaacattgagcccagcgtgcggagctgcttccagttcgccaacaacaagcccgagatcgaggccgccctgttcctggactggatgagactggaaccccagagcatggtgtggctgcccgtgctgcatcgggtggccgctgccgagacagccaagcaccaggccaagtgcaacatctgcaaagagtgccccatcatcggcttccggtacagaagcctgaagcacttcaactacgatatctgccagagctgcttcttcagcggcagagtggccaagggccacaaaatgcactaccccatggtggaatactgcacccccaccaccagcggcgaggatgtgcgggacttcgccaaggtgctgaaaaacaagttccggaccaagcggtactttgccaagcacccccggatgggctacctgcccgtgcagacagtgctggaaggcgacaacatggaaacccctgcccagatcctgatcagcctggaaagcgaggaacggggcgagctggaacggatcctggccgatctggaagaggaaaaccggaacctgcaggccgagtacgaccggctgaagcagcagcacgagcacaagggcctgagccccctgcctagcccccctgacaccatgtgatgatgatttgggcagagcgatggagtccttagtatcagtcatgacagatgaagaaggagcagaataaatgttttacaactcctgattcccgcatgcggccagcttatcgataccgtcgaaataaaagatccttattttcattggatctgtgtgttggttttttgtgtg

SEQ ID NO: 148 - DNA, 4164 bp, Homo sapiens
atgctgtggtgggaggaagtggaagattgctacgagcgcgaggacgtgcagaagaaaaccttcaccaaatgggtgaacgcccagttcagcaagttcggcaagcagcacatcgagaacctgttcagcgacctgcaggacggcagacggctgctggacctgctggaaggcctgaccggccagaagctgcccaaagagaagggcagcaccagagtgcacgccctgaacaacgtgaacaaggccctgcgggtgctgcagaacaacaacgtggacctggtgaacatcggcagcaccgacatcgtggacggcaaccacaagctgaccctgggcctgatctggaacatcatcctgcactggcaggtcaaaaacgtgatgaagaacatcatggccggcctgcagcagaccaacagcgagaagatcctgctgagctgggtgcgccagagcacccggaactacccccaggtcaacgtgatcaacttcaccacctcttggagcgacggcctggccctgaacgccctgatccacagccaccggcccgacctgttcgactggaacagcgtggtctgccagcagagcgccacccagcggctggaacacgccttcaatatcgccagataccagctgggcatcgagaagctgctggatcccgaggacgtggacaccacctaccccgacaagaaatccatcctgatgtatatcaccagcctgttccaggtgctgccccagcaggtgtccatcgaggccatccaggaagtggaaatgctgcccagaccccccaaagtgaccaaagaggaacacttccagctgcaccaccagatgcactacagccagcagatcaccgtgtccctggctcagggctacgagcggaccagcagccccaagccccggttcaagagctacgcctacacccaggccgcctacgtgaccaccagcgaccccaccagaagcccattccccagccagcatctggaagcccccgaggacaagagcttcggcagcagcctgatggaaagcgaagtgaacctggacagataccagaccgccctggaagaggtgctgtcctggctgctgagcgccgaggatacactgcaggcccagggcgagatcagcaacgacgtggaagtggtgaaagaccagttccacacccacgagggctacatgatggacctgaccgcccaccagggcagagtgggcaacatcctgcagctgggcagcaagctgatcggcaccggcaagctgagcgaggacgaagagacagaggtgcaggaacagatgaacctgctgaacagcagatgggagtgcctgcgggtggccagcatggaaaagcagagcaacctgcacatccacaccgtgcgggaagagacaatgatggtgatgaccgaggacatgcccctggaaatcagctacgtgcccagcacctacctgaccgagatcacccacgtgtcccaggctctgctggaagtggaacagctgctgaacgcccccgacctgtgcgccaaggacttcgaggatctgttcaagcaggaagagagcctgaagaatatcaaggactccctgcagcagtccagcggccggatcgacatcatccacagcaagaaaacagccgccctgcagtccgccacccccgtggaaagagtgaagctgcaggaagccctgagccagctggacttccagtgggagaaagtgaacaagatgtacaaggaccggcagggcagattcgaccgcagcgtggaaaagtggcggcggttccactacgacatcaagatcttcaaccagtggctgaccgaggccgagcagttcctgagaaagacccagatccccgagaactgggagcacgccaagtacaagtggtatctgaaagagctgcaggacggcatcggccagcggcagacagtggtccgcaccctgaatgccaccggcgaggaaatcatccagcagagcagcaagaccgacgccagcatcctgcaggaaaagctgggcagcctgaacctgcggtggcaggaagtgtgcaagcagctgagcgaccggaagaagcggctggaagaacaggcccctggcctgaccacaatcggcgccagccctacccagaccgtgaccctggtgacacagcccgtggtgacaaaagagacagccatcagcaagctggaaatgcccagcagcctgatgctggaaagcgaccagtggaagcggctgcacctgagcctgcaggaactgctggtctggctgcagctgaaggacgacgagctgagcagacaggcccccatcggcggcgatttccccgccgtgcagaaacagaacgacgtgcaccgggccttcaagcgcgagctgaaaacaaaagaacccgtgatcatgagcaccctggaaaccgtgcggatcttcctgaccgagcagcccctggaaggcctggaaaagctgtaccaggaacccagagagctgccccccgaggaacgggcccagaacgtgaccagactgctgcggaagcaggccgaagaggtcaacaccgagtgggagaagctgaacctgcacagcgccgactggcagcggaagatcgacgagacactggaacggctgcaggaactgcaggaggccaccgacgagctggacctgaagctgagacaggccgaagtgatcaagggcagctggcagcccgtgggcgacctgctgatcgactccctgcaggaccacctggaaaaagtgaaggccctgcggggcgagatcgcccccctgaaagaaaacgtgtcccacgtgaacgacctggcccggcagctgaccaccctgggcatccagctgagcccctacaacctgtccaccctggaagatctgaacacccggtggaagctgctgcaggtggccgtggaagatagagtgcggcagctgcacgaggcccacagagactttggccctgccagccagcacttcctgagcacctctgtgcagggaccctgggagagagccatcagccccaacaaggtgccctactacatcaaccacgagacacagaccacctgttgggaccaccccaagatgaccgagctgtaccagagcctggccgacctgaacaatgtgcggttcagcgcctaccggaccgccatgaagctgaggcggctgcagaaagctctgtgcctggatctgctgagcctgagcgccgcctgcgacgccctggaccagcacaacctgaagcagaacgaccagcccatggatatcctgcagatcatcaactgcctgaccacaatctacgacaggctggaacaggaacacaacaatctggtcaacgtgcccctgtgcgtggacatgtgcctgaattggctgctgaatgtgtacgacaccggccggaccggcagaatccgggtgctgagcttcaagaccggcatcatcagcctgtgcaaggcccacctggaagataagtaccgctacctgttcaaacaggtggccagctccaccggcttttgcgaccagcggagactgggcctgctgctgcacgacagcatccagatccccagacagctgggcgaggtggcctccttcggcggcagcaacattgagcccagcgtgcggagctgcttccagttcgccaacaacaagcccgagatcgaggccgccctgttcctggactggatgagactggaaccccagagcatggtgtggctgcccgtgctgcatcgggtggccgctgccgagacagccaagcaccaggccaagtgcaacatctgcaaagagtgccccatcatcggcttccggtacagaagcctgaagcacttcaactacgatatctgccagagctgcttcttcagcggcagagtggccaagggccacaaaatgcactaccccatggtggaatactgcacccccaccaccagcggcgaggatgtgcgggacttcgccaaggtgctgaaaaacaagttccggaccaagcggtactttgccaagcacccccggatgggctacctgcccgtgcagacagtgctggaaggcgacaacatggaaaccgacaccatgtgatgatgatttgggcagagcgatggagtccttagtatcagtcatgacagatgaagaaggagcagaataaatgttttacaactcctgattcccgcatgcggccagcttatcgataccgtcgaaataaaagatccttattttcattggatctgtgtgttggttttttgtgtg

SEQ ID NO: 149 - DNA, 4076 bp, Homo sapiens
atgctgtggtgggaggaagtggaagattgctacgagcgcgaggacgtgcagaagaaaaccttcaccaaatgggtgaacgcccagttcagcaagttcggcaagcagcacatcgagaacctgttcagcgacctgcaggacggcagacggctgctggacctgctggaaggcctgaccggccagaagctgcccaaagagaagggcagcaccagagtgcacgccctgaacaacgtgaacaaggccctgcgggtgctgcagaacaacaacgtggacctggtgaacatcggcagcaccgacatcgtggacggcaaccacaagctgaccctgggcctgatctggaacatcatcctgcactggcaggtcaaaaacgtgatgaagaacatcatggccggcctgcagcagaccaacagcgagaagatcctgctgagctgggtgcgccagagcacccggaactacccccaggtcaacgtgatcaacttcaccacctcttggagcgacggcctggccctgaacgccctgatccacagccaccggcccgacctgttcgactggaacagcgtggtctgccagcagagcgccacccagcggctggaacacgccttcaatatcgccagataccagctgggcatcgagaagctgctggatcccgaggacgtggacaccacctaccccgacaagaaatccatcctgatgtatatcaccagcctgttccaggtgctgccccagcaggtgtccatcgaggccatccaggaagtggaaatgctgcccagaccccccaaagtgaccaaagaggaacacttccagctgcaccaccagatgcactacagccagcagatcaccgtgtccctggctcagggctacgagcggaccagcagccccaagccccggttcaagagctacgcctacacccaggccgcctacgtgaccaccagcgaccccaccagaagcccattccccagccagcatctggaagcccccgaggacaagagcttcggcagcagcctgatggaaagcgaagtgaacctggacagataccagaccgccctggaagaggtgctgtcctggctgctgagcgccgaggatacactgcaggcccagggcgagatcagcaacgacgtggaagtggtgaaagaccagttccacacccacgagggctacatgatggacctgaccgcccaccagggcagagtgggcaacatcctgcagctgggcagcaagctgatcggcaccggcaagctgagcgaggacgaagagacagaggtgcaggaacagatgaacctgctgaacagcagatgggagtgcctgcgggtggccagcatggaaaagcagagcaacctgcacatccacaccgtgcgggaagagacaatgatggtgatgaccgaggacatgcccctggaaatcagctacgtgcccagcacctacctgaccgagatcacccacgtgtcccaggctctgctggaagtggaacagctgctgaacgcccccgacctgtgcgccaaggacttcgaggatctgttcaagcaggaagagagcctgaagaatatcaaggactccctgcagcagtccagcggccggatcgacatcatccacagcaagaaaacagccgccctgcagtccgccacccccgtggaaagagtgaagctgcaggaagccctgagccagctggacttccagtgggagaaagtgaacaagatgtacaaggaccggcagggcagattcgaccgcagcgtggaaaagtggcggcggttccactacgacatcaagatcttcaaccagtggctgaccgaggccgagcagttcctgagaaagacccagatccccgagaactgggagcacgccaagtacaagtggtatctgaaagagctgcaggacggcatcggccagcggcagacagtggtccgcaccctgaatgccaccggcgaggaaatcatccagcagagcagcaagaccgacgccagcatcctgcaggaaaagctgggcagcctgaacctgcggtggcaggaagtgtgcaagcagctgagcgaccggaagaagcggctggaagaacaggcccctggcctgaccacaatcggcgccagccctacccagaccgtgaccctggtgacacagcccgtggtgacaaaagagacagccatcagcaagctggaaatgcccagcagcctgatgctggaaagcgaccagtggaagcggctgcacctgagcctgcaggaactgctggtctggctgcagctgaaggacgacgagctgagcagacaggcccccatcggcggcgatttccccgccgtgcagaaacagaacgacgtgcaccgggccttcaagcgcgagctgaaaacaaaagaacccgtgatcatgagcaccctggaaaccgtgcggatcttcctgaccgagcagcccctggaaggcctggaaaagctgtaccaggaacccagagagctgccccccgaggaacgggcccagaacgtgaccagactgctgcggaagcaggccgaagaggtcaacaccgagtgggagaagctgaacctgcacagcgccgactggcagcggaagatcgacgagacactggaacggctgcaggaactgcaggaggccaccgacgagctggacctgaagctgagacaggccgaagtgatcaagggcagctggcagcccgtgggcgacctgctgatcgactccctgcaggaccacctggaaaaagtgaaggccctgcggggcgagatcgcccccctgaaagaaaacgtgtcccacgtgaacgacctggcccggcagctgaccaccctgggcatccagctgagcccctacaacctgtccaccctggaagatctgaacacccggtggaagctgctgcaggtggccgtggaagatagagtgcggcagctgcacgaggcccacagagactttggccctgccagccagcacttcctgagcacctctgtgcagggaccctgggagagagccatcagccccaacaaggtgccctactacatcaaccacgagacacagaccacctgttgggaccaccccaagatgaccgagctgtaccagagcctggccgacctgaacaatgtgcggttcagcgcctaccggaccgccatgaagctgaggcggctgcagaaagctctgtgcctggatctgctgagcctgagcgccgcctgcgacgccctggaccagcacaacctgaagcagaacgaccagcccatggatatcctgcagatcatcaactgcctgaccacaatctacgacaggctggaacaggaacacaacaatctggtcaacgtgcccctgtgcgtggacatgtgcctgaattggctgctgaatgtgtacgacaccggccggaccggcagaatccgggtgctgagcttcaagaccggcatcatcagcctgtgcaaggcccacctggaagataagtaccgctacctgttcaaacaggtggccagctccaccggcttttgcgaccagcggagactgggcctgctgctgcacgacagcatccagatccccagacagctgggcgaggtggcctccttcggcggcagcaacattgagcccagcgtgcggagctgcttccagttcgccaacaacaagcccgagatcgaggccgccctgttcctggactggatgagactggaaccccagagcatggtgtggctgcccgtgctgcatcgggtggccgctgccgagacagccaagcaccaggccaagtgcaacatctgcaaagagtgccccatcatcggcttccggtacagaagcctgaagcacttcaactacgatatctgccagagctgcttcttcagcggcagagtggccaagggccacaaaatgcactaccccatggtggaatactgcacccccaccaccagcggcgaggatgtgcgggacttcgccaaggtgctgaaaaacaagttccggaccaagcggtactttgccaagcacccccggatgggctacctgcccgtgcagacagtgctggaaggcgacaacatggaaaccgacaccatgtgatgatgagaagtcttttccacatggcagatgaaataaaagatccttattttcattggatctgtgtgttggttttttgtgtg

SEQ ID NO: 150 - DNA, 10 bp, Homo sapiens
gccrccaugg

SEQ ID NO: 151 - DNA, 10 bp, Homo sapiens
gccaccatgg

SEQ ID NO: 152 - protein, 1332 aa, Homo sapiens
MLWWEEVEDCYEREDVQKKTFTKWVNAQFSKFGKQHIENLFSDLQDGRRLLDLLEGLTGQKLPKEKGSTRVHALNNVNKALRVLQNNNVDLVNIGSTDIVDGNHKLTLGLIWNIILHWQVKNVMKNIMAGLQQTNSEKILLSWVRQSTRNYPQVNVINFTTSWSDGLALNALIHSHRPDLFDWNSVVCQQSATQRLEHAFNIARYQLGIEKLLDPEDVDTTYPDKKSILMYITSLFQVLPQQVSIEAIQEVEMLPRPPKVTKEEHFQLHHQMHYSQQITVSLAQGYERTSSPKPRFKSYAYTQAAYVTTSDPTRSPFPSQHLEAPEDKSFGSSLMESEVNLDRYQTALEEVLSWLLSAEDTLQAQGEISNDVEVVKDQFHTHEGYMMDLTAHQGRVGNILQLGSKLIGTGKLSEDEETEVQEQMNLLNSRWECLRVASMEKQSNLHIHTVREETMMVMTEDMPLEISYVPSTYLTEITHVSQALLEVEQLLNAPDLCAKDFEDLFKQEESLKNIKDSLQQSSGRIDIIHSKKTAALQSATPVERVKLQEALSQLDFQWEKVNKMYKDRQGRFDRSVEKWRRFHYDIKIFNQWLTEAEQFLRKTQIPENWEHAKYKWYLKELQDGIGQRQTVVRTLNATGEEIIQQSSKTDASILQEKLGSLNLRWQEVCKQLSDRKKRLEEQKNDLAPGLTTIGASPTQTVTLVTQPVVTKETAISKLEMPSSLMLESDQWKRLHLSLQELLVWLQLKDDELSRQAPIGGDFPAVQKQNDVHRAFKRELKTKEPVIMSTLETVRIFLTEQPLEGLEKLYQEPRELPPEERAQNVTRLLRKQAEEVNTEWEKLNLHSADWQRKIDETLERLQELQEATDELDLKLRQAEVIKGSWQPVGDLLIDSLQDHLEKVKALRGEIAPLKENVSHVNDLARQLTTLGIQLSPYNLSTLEDLNTRWKLLQVAVEDRVRQLHEAHRDFGPASQHFLSTSVQGPWERAISPNKVPYYINHETQTTCWDHPKMTELYQSLADLNNVRFSAYRTAMKLRRLQKALCLDLLSLSAACDALDQHNLKQNDQPMDILQIINCLTTIYDRLEQEHNNLVNVPLCVDMCLNWLLNVYDTGRTGRIRVLSFKTGIISLCKAHLEDKYRYLFKQVASSTGFCDQRRLGLLLHDSIQIPRQLGEVASFGGSNIEPSVRSCFQFANNKPEIEAALFLDWMRLEPQSMVWLPVLHRVAAAETAKHQAKCNICKECPIIGFRYRSLKHFNYDICQSCFFSGRVAKGHKMHYPMVEYCTPTTSGEDVRDFAKVLKNKFRTKRYFAKHPRMGYLPVQTVLEGDNMET

SEQ ID NO: 153 - protein, 1322 aa, Homo sapiens
MLWWEEVEDCYEREDVQKKTFTKWVNAQFSKFGKQHIENLFSDLQDGRRLLDLLEGLTGQKLPKEKGSTRVHALNNVNKALRVLQNNNVDLVNIGSTDIVDGNHKLTLGLIWNIILHWQVKNVMKNIMAGLQQTNSEKILLSWVRQSTRNYPQVNVINFTTSWSDGLALNALIHSHRPDLFDWNSVVCQQSATQRLEHAFNIARYQLGIEKLLDPEDVDTTYPDKKSILMYITSLFQVLPQQVSIEAIQEVEMLPRPPKVTKEEHFQLHHQMHYSQQITVSLAQGYERTSSPKPRFKSYAYTQAAYVTTSDPTRSPFPSQHLEAPEDKSFGSSLMESEVNLDRYQTALEEVLSWLLSAEDTLQAQGEISNDVEVVKDQFHTHEGYMMDLTAHQGRVGNILQLGSKLIGTGKLSEDEETEVQEQMNLLNSRWECLRVASMEKQSNLHRVLLKWQRLTEEQCLFSAWLSEKEDAVNKIHTTGFKDQNEMLSSLQKLAVLKADLEKKKQSMGKLYSLKQDLLSTLKNKSVTQKTEAWLDNFARCWDNLVQKLEKSTAQISQAVTTTQPSLTQTTVMETVTTVTTREQILVKHAQEELPPPPPQKKRQITVDSEIHTVREETMMVMTEDMPLEISYVPSTYLTEITHVSQALLEVEQLLNAPDLCAKDFEDLFKQEESLKNIKDSLQQSSGRIDIIHSKKTAALQSATPVERVKLQEALSQLDFQWEKVNKMYKDRQGRFDRSVEKWRRFHYDIKIFNQWLTEAEQFLRKTQIPENWEHAKYKWYLKELQDGIGQRQTVVRTLNATGEEIIQQSSKTDASILQEKLGSLNLRWQEVCKQLSDRKKRLEEQLERLQELQEATDELDLKLRQAEVIKGSWQPVGDLLIDSLQDHLEKVKALRGEIAPLKENVSHVNDLARQLTTLGIQLSPYNLSTLEDLNTRWKLLQVAVEDRVRQLHEAHRDFGPASQHFLSTSVQGPWERAISPNKVPYYINHETQTTCWDHPKMTELYQSLADLNNVRFSAYRTAMKLRRLQKALCLDLLSLSAACDALDQHNLKQNDQPMDILQIINCLTTIYDRLEQEHNNLVNVPLCVDMCLNWLLNVYDTGRTGRIRVLSFKTGIISLCKAHLEDKYRYLFKQVASSTGFCDQRRLGLLLHDSIQIPRQLGEVASFGGSNIEPSVRSCFQFANNKPEIEAALFLDWMRLEPQSMVWLPVLHRVAAAETAKHQAKCNICKECPIIGFRYRSLKHFNYDICQSCFFSGRVAKGHKMHYPMVEYCTPTTSGEDVRDFAKVLKNKFRTKRYFAKHPRMGYLPVQTVLEGDNMET

SEQ ID NO: 154 - DNA, 4043 bp, Homo sapiens
atgctgtggtgggaggaagtggaagattgctacgagcgcgaggacgtgcagaagaaaaccttcaccaaatgggtgaacgcccagttcagcaagttcggcaagcagcacatcgagaacctgttcagcgacctgcaggacggcagacggctgctggacctgctggaaggcctgaccggccagaagctgcccaaagagaagggcagcaccagagtgcacgccctgaacaacgtgaacaaggccctgcgggtgctgcagaacaacaacgtggacctggtgaacatcggcagcaccgacatcgtggacggcaaccacaagctgaccctgggcctgatctggaacatcatcctgcactggcaggtcaaaaacgtgatgaagaacatcatggccggcctgcagcagaccaacagcgagaagatcctgctgagctgggtgcgccagagcacccggaactacccccaggtcaacgtgatcaacttcaccacctcttggagcgacggcctggccctgaacgccctgatccacagccaccggcccgacctgttcgactggaacagcgtggtctgccagcagagcgccacccagcggctggaacacgccttcaatatcgccagataccagctgggcatcgagaagctgctggatcccgaggacgtggacaccacctaccccgacaagaaatccatcctgatgtatatcaccagcctgttccaggtgctgccccagcaggtgtccatcgaggccatccaggaagtggaaatgctgcccagaccccccaaagtgaccaaagaggaacacttccagctgcaccaccagatgcactacagccagcagatcaccgtgtccctggcccagggctacgagagaaccagcagccccaagccccggttcaagagctacgcctatacccaggccgcctacgtgaccaccagcgaccctaccagaagcccattccccagccagcatctggaagcccccgaggacaagagcttcggcagcagcctgatggaaagcgaagtgaacctggacagataccagaccgccctggaagaggtgctgagctggctgctgagcgccgaggatacactgcaggctcagggcgagatcagcaacgacgtggaagtcgtgaaggaccagttccacacccacgagggctacatgatggacctgacagcccaccagggcagagtgggcaacatcctgcagctgggctccaagctgatcggcaccggcaagctgagcgaggacgaagagacagaggtgcaggaacagatgaacctgctgaacagcagatgggagtgcctgcgggtggccagcatggaaaagcagagcaacctgcatagggtcctgctgaagtggcagcggctgaccgaggaacagtgcctgtttagcgcctggctgtccgagaaagaggacgccgtgaacaagatccacaccaccggcttcaaggaccagaacgagatgctgagcagcctgcagaaactggccgtgctgaaggccgacctggaaaagaaaaagcagtccatgggcaagctgtactccctgaagcaggacctgctgtccaccctgaagaacaagagcgtgacccagaaaaccgaggcctggctggacaacttcgcccggtgctgggacaacctggtgcagaagctggaaaagtccaccgcccagatctcccaggccgtgaccacaacacagcccagcctgacccagaccaccgtgatggaaaccgtgacaacagtgaccacccgggaacagatcctcgtgaagcacgcccaggaagaactgccccctccacccccccagaagaaacggcagatcacagtggacagtgaaatccacaccgtgcgggaagagacaatgatggtcatgacagaggacatgcccctggaaatcagctacgtgcccagcacctacctgaccgagatcacccatgtgtcccaggccctgctggaagtggaacagctgctgaacgcccccgacctgtgcgccaaggatttcgaggacctgttcaagcaggaagagagcctgaagaatatcaaggatagcctgcagcagagcagcggccggatcgacatcatccacagcaagaaaacagccgccctgcagagcgccacccccgtggaaagagtgaaactgcaggaagccctgtcccagctggacttccagtgggagaaagtgaacaaaatgtacaaggaccggcagggcagattcgaccgcagcgtggaaaagtggcggcggttccactacgacatcaagatcttcaaccagtggctgacagaggccgagcagttcctgagaaagacccagatccccgagaactgggagcacgccaagtacaagtggtatctgaaagagctgcaggacggcatcggccagagacagacagtcgtgcggaccctgaatgccaccggcgaggaaatcatccagcagtccagcaagaccgacgccagcattctgcaggaaaagctgggcagcctgaacctgcggtggcaggaagtgtgcaagcagctgtccgaccggaagaagcggctggaagaacagctggaacggctgcaggaactgcaggaggccaccgacgagctggacctgaaactgagacaggccgaagtgatcaagggcagctggcagccagtgggcgacctgctgatcgactccctgcaggaccatctggaaaaagtgaaggccctgagaggcgagatcgcccccctgaaagaaaacgtgtcccacgtgaacgacctggcccggcagctgacaacactgggcattcagctgagcccctacaacctgagcacactggaagatctgaacacccggtggaagctgctgcaggtggccgtggaagatagagtgcggcagctgcacgaggcccacagagattttggccctgcctcccagcacttcctgagcaccagtgtgcagggcccttgggagagagccatctcccctaacaaggtgccctactacatcaaccacgagacacagaccacctgttgggaccaccccaagatgaccgagctgtaccagagcctggctgacctgaacaacgtgcggttcagcgcctaccggaccgccatgaagctgcggagactgcagaaagctctgtgcctggatctgctgtccctgtccgccgcctgtgatgccctggaccagcacaatctgaagcagaacgaccagcccatggatatcctgcagatcatcaactgcctgaccaccatctacgaccggctggaacaggaacacaacaatctcgtgaacgtgcccctgtgcgtggacatgtgcctgaattggctgctgaatgtgtacgacaccggccggacaggccggatcagagtgctgtccttcaagaccggcatcatcagcctgtgcaaagcccacctggaagataagtaccggtatctgttcaaacaggtggcctctagcaccggcttttgcgaccagagaaggctgggcctgctgctgcacgacagcatccagatccctagacagctgggcgaagtggccagctttggcggcagcaacatcgagcctagcgtgcggagctgcttccagttcgccaacaacaagcccgagatcgaggccgccctgttcctggactggatgagactggaaccccagagcatggtgtggctgcccgtgctgcatagagtggccgctgccgagacagccaagcaccaggccaagtgcaacatctgcaaagagtgccccatcatcggcttccggtacagaagcctgaagcacttcaactacgatatctgccagagctgtttcttcagcggcagggtggccaagggccacaaaatgcactaccccatggtggaatactgcacccccaccacaagcggcgaggatgtgcgggatttcgccaaggtgctgaaaaacaagttccggaccaagcggtacttcgccaaacacccccggatgggctacctgcctgtgcagacagtgctggaaggcgacaacatggaaacctgagaagtcttttccacatggcagatgaaataaaagatccttattttcattggatctgtgtgttggttttttgtgtg

SEQ ID NO: 155 - protein, 35 aa, Homo sapiens
LPPPPPQKKRQITVDIHTVREETMMVMTEDMPLEI

SEQ ID NO: 156 - protein, 36 aa, Homo sapiens
LPPPPPQKKRQITVDSIHTVREETMMVMTEDMPLEI

SEQ ID NO: 157 - protein, 37 aa, Homo sapiens
LPPPPPQKKRQITVDSEIHTVREETMMVMTEDMPLEI

SEQ ID NO: 158 - protein, 36 aa, Homo sapiens
LPPPPPQKKRQITVDQIHTVREETMMVMTEDMPLEI

SEQ ID NO: 159 - protein, 37 aa, Homo sapiens
LPPPPPQKKRQITVDAQIHTVREETMMVMTEDMPLEI

SEQ ID NO: 160 - protein, 34 aa, Homo sapiens
LPPPPPQKKRQITVIHTVREETMMVMTEDMPLEI

SEQ ID NO: 161 - protein, 34 aa, Homo sapiens
LPPPPPQKKRQITVDHTVREETMMVMTEDMPLEI

SEQ ID NO: 162 - protein, 33 aa, Homo sapiens
LPPPPPQKKRQITVHTVREETMMVMTEDMPLEI

SEQ ID NO: 163 - protein, 37 aa, Homo sapiens
LPPPPPQKKRQITVDSQIHTVREETMMVMTEDMPLEI

SEQ ID NO: 164 - protein, 35 aa, Homo sapiens
LPPPPPQKKRQITVDSHTVREETMMVMTEDMPLEI

SEQ ID NO: 165 - protein, 35 aa, Homo sapiens
LPPPPPQKKRQITVQIHTVREETMMVMTEDMPLEI

SEQ ID NO: 166 - protein, 24 aa, Homo sapiens
QKKRQITVDSEAQIHTVREETMMV